European Patent Application EP 4 289 949 A1, published December 13, 2023. Title: BacterioPhage lysine, chimera thereof and application thereof. Applicant: WUHAN LYSIGEN BIO-TECH COMPANY LIMITED. The sequence listing filed with the application follows.

SEQUENCE LISTING (406 sequences)

SEQ ID NO: 1 - protein, 502 aa, Artificial Sequence
MSLGSGRKERIHKMDVNTLREVMGNYRNVNYDAMVGPMNEAMIAAGCTNLRRAAMWCAQIGHESEGLTAMEEYASGAGYEGRLDLGNTQPGDGVRYKGRGPIQLTGRSNYRAFTTWARSKGYTTIDFEAEPHKVSEPKWGFLAASFYWTVRRPDINSLADQGDVTRVTHRINGGENGLSDRIARYNRAMALGDRILPSASETGTQTSKTTAAEKVLDYKRDWVKQDTYYNCGPASCQTVIGAATGNYPGEVELAAALKTTINGTDWIGVFPGVLNRYIPGGKYSSREIPNDPPRSDQRDQLWKDIINSINSGYGVVANIVAPPSNYPRASYKSTQSPAYAGGTVYHYVAVMGYAIDDSGRSHVWVADSGFAPYGYWMTLQQLSTLIPPKGYAYSTNIPQEGLDMDAVKQIIDFVKGWTGPMIQDIKDIRQQLTGGRDTVYREDGSVDLVASYPGWRQLGTDKNGNPLSMVDSIAWSHVKSDKIIEILTALQDRITELEKKVK

SEQ ID NO: 2 - protein, 343 aa, Artificial Sequence
MTKILTIEKAREFDAFARARDNLYYGYGEAFTRNPRQSTDCSGLVLQSGAILGGRTDWVGNRYGSTESFRLDYAIVYALGFKRMPRGGLPFVPVMKVGLQHGGGGIYSHTACTLMFLDKPGGPIKESARGVDWESQGAGVFYYEGARAWNDGLFHDFWYLDMRLGELAPPVNEINAEFERAKGWIGKRIDVAEKPCPDGEGKYIRCEGGHIYFHPKVNVGAKPGERAIAIPADVFEVWKRQGFEKGPLGYPTRRHATVNGVGTIQAFQNGAVYRKFGTDGGIVNGKILERWAREGHEKGRLGWPLGDEKFFDGGRVQAFENGDAYFHPTAVVEFLNDPAAPKQ

SEQ ID NO: 3 - protein, 270 aa, Artificial Sequence
MRPYRARHLATPPTPDSTPDTSSGASRRSVLRGGVLGAAALSTGAAAVATPAANAAGLYGQDVSGWQGEIDWSAQADLGSRFAYVKATEGRSYRSPAFNQQYRGAGNAGLVRGGYHFARPDSGGPEEQVDFFLNNGGGWSDDGITLPGMVDFEAYSGLPRDYGLSQQEMRNWIMAFSTRYRDSVGRRPVLYTNLHWWNDVVGDWTPVNSPLFLASYSSSAPTTLPGRWWAYEMWQYSDSGPFAGDSNLWHGSESQFESFVSDGDYHAIGI

SEQ ID NO: 4 - protein, 143 aa, Artificial Sequence
MRFIPAAHHSAGSNSPVNRVVIHATCPDVGFPSASRKGRAVSTANYFASPSSGGSAHYVCDVGETVQCLSEGTIGWHAPPNPHSLGIEICADGGSHASFRVPGHAYTREQWLDPRVWPAVEKAAILCRRLCDKYKCLHEGAVA

SEQ ID NO: 5 - protein, 473 aa, Artificial Sequence
MATMPVKKGFYVTSGFGPRWGTTHYGTDFGVDGGSGGHPIFAIKSGTVTASGPASGFGQWINVDHPASDGGGLSVYGHIIPEVRVGDQVVEGQRIGRINPDQNTNGGVAPHLHLEFHRSVWSPPGGDRLDPMKTVLAGADWPGDAPSNSSAKPETGKVKNIFGVDISNHQNGILAELIGAEGFEFCIIKATEGTWKDPILHSHLADVRKNSGMQVGAYVYVRGETSPEAHAIALHEHLNDTSVPVALDIEHNSGSNPDHWRAIKTAIEARGYRVILTYLPEWYWSQVGQPNLAGLPPLWASRYVGTTPGVASVLYSTAGRRGWQGYGGLEVAMWQFTDRAQVAGQKIDANVFEGTEKQLRALFHGDTPEIEEEFDMSAVQEIKDYIDTRLTGPVGTDVKDIRQQITGGRDSIPGDLKASYPGWDLGQLVRAAREKEFTGLTMMEILAVNIAGNDDDFRAARVAAGTEEAGNAE

SEQ ID NO: 6 - protein, 426 aa, Artificial Sequence
MADYFYPLSQGAHVTSPFGPRAGGYHWGTDYGRAGGSGGNAVYAPQAGTVIMAGPASGFGGPDPAGWIVIDHPTAAGGGVSVLGHIIREVAVGDTVRAGQRIGRVNPSSATNGGVAPHVHFEHHRYVWSPPGPDRLDPHAWLATRGARWPGAPATPTRKESMNALTADIDLLTPNDDGRATKPRNLLCIHTFEDDGTWSADRMAKYQQSPAAGGSYHLVIDLNGRIARENDDAFIPWAAMFTGNRVAFHFSLSGKASWTRQQWLARPKQMDALAKVLAAYSKAKGIPLIRRGPQDVRAGKWGVCGHDDISKAFGESTHWDPGPNFPFDVVIDKAKAILAEPKPTPAPPSDPAPRPIPPKETLVPTTLDTVLPSLVDGSTFEAPLATFIRTADKQAYEANQRIARLEAKFDRLLDAMGEKPDPKPGQ

SEQ ID NO: 7 - protein, 285 aa, Artificial Sequence
MRYIPAAHHSAGSNSPVNRVVIHATCPDVGFPSASRKGRAVSTANYFASPSAGGSAHYVCDVGETVQCLSESTIGWHAPPNPHSLGIEICADGGSHASFRVPGHAYTREQWLDPRVWPAVEKAAVLCRQLCDKYNVPKRKLSVSDLKAGRRGVCGHTDVTDAWHQSDHDDPGPWFPWDRFMAVVNGGSGESGELSMADVKALHDQIKQLSGQVAQSVNKLHHDVGVVQVQNGNLKKQVDSLSMVKNPVTGKLWRTRDAIWSIWYYVLECRSRIGKLEAEVARLKK

SEQ ID NO: 8 - protein, 245 aa, Artificial Sequence
MSTANYFASPSSGGSAHYVCDISETVQCLSESTIGWHAPPNPHSLGIEICADGGSHASFRVPGHAYTREQWLDPRVWPAVEKAAILCRRLCDKYNVPKRKLSVADLKAGRRGVCGHVDVTDAWHQSDHDDPGPWFPWDRFMAVVNGGSGDSGELTVADVKALHDQIKQLSAQLTGSVNKLHHDVGVVQVQNGDLGKRVDALSWVKNPVTGKLWRTKDALWSVWYYVLECRSRIDRLESAVNGLKK

SEQ ID NO: 9 - protein, 281 aa, Artificial Sequence
MTFIQARHHGGNSNTPITRLVIHATCPDVGYPSASKAGRAVSTAEYFASTSRSASAHYVCDVSATVQCLSEETIGYHAPPNSHSIGIEICADGGSRASFEKASHAYTREQWLSPQVWPAVERAAILARGICHRHHIPVRKLTTAQVKSGMSGICGHDNVSDAFHQSDHDDPGPYFPWNEFIAAIQGKNTNKGELSMSDVNTLTKLIKASNNQLHHDIGVVQTQNGTLKSKIDNLSWVKNPVTGKKWSTKDALWSVWYYVLECRNRIQAIENRLSDIEKKVK

SEQ ID NO: 10 - protein, 269 aa, Artificial Sequence
MTFIQAAHHSSGSNLPPTRVVIHATCPELGFPRASAKGRAVSTARYFQSAISGGSAHYVVDVGETVQCLAEDVIAWHAPPNSRSLGIEICADGGSATSFKNPNVRYSRAQWLSPQVWPAVLRAAALTRQMCQKYGIPVTKLSASDLKAGKKGICGHVDVSNAWHQSDHDDPGPDFPWAEFMAAVKGGATNPDELELTVSQFSDLTKRLQGMQEQTHHDLGVVQTKLATMDTVKNPRTGAKWSLKDAIWSIWYYVLENRDRIAALEKKVK

SEQ ID NO: 11 - protein, 284 aa, Artificial Sequence
MDWTNLNADVTKLMNVHFTPGREGHTIDKIVIHHNGGNLSIDQIWNVWQDREASAHYQVQSDGRIGQLVNDWDTAWHAGDWDANLTSIGIEHADDSTDPWHVSDAAVDAGAHLVAALCRGYNLGRPEWMRNVFPHSHFSATSCPASLAENQRADYMARAQAYFDGAPVTGRSSVPAPAPAPAGIHVDLPAWTLPAGNFYGSIDGGEDSHGGYYEGERPAIAAIQRWLIRHGYAGAVDDSWADGLYEQPTVDAVTRFQRAERPNSTDRWGEVWADDLATMAANNG

SEQ ID NO: 12 - protein, 298 aa, Artificial Sequence
MDRGIDVSSYQAPDGGLLEGMSFCIIKATEGTGYVNPNRTQWYKVATDRGVTTGAYHFMRGGDPVAQADYFLAHLPGDVDWLALDVEDPSDGLSWAGRVSFILAWTDRVKATGKPTLVYCSRSWANALLGAASSDERARLAQLPLWMADYTQRPGEYSGPWPGGWPIAIHQYTSAPIDKNVLLTDDLQGGDDMPLSTDDLRNIATAVWGGGGAASPMYADRLDGHQEYPETALFSLQQRLGARFGELSGKIDGLAEALKQVQGGNGVDADAIRAAAAEGAKAGVQAMIDTATVNLEAK

SEQ ID NO: 13 - protein, 297 aa, Artificial Sequence
MCGAFSFLKDLETFMDWTNLNADVTKLMGVHFTPGREGRTIDKIVIHHNGGNLSIDQIWNVWQTREASAHYQVEAGGRIGQLVNDLDTAWHAGDWDANLTSIGIEHADDSTDPWHVSDAAVDAGAHLVAALCRGYNLGRPEWMRNVFPHSQFTSTSCPASLARDQLGDYMGRAQAYFDGAPVAAVHQSVPAPAPAPSRHVDLPAWNLPEGNFYGLVSGGNDSHGGFYPAERPAVRAIQLWLIRHGYAGAVPDSWADGIYEQPTADAVTAFQHAERPNSTDRWGEVWADDLATMAANN

SEQ ID NO: 14 - protein, 354 aa, 人工序列(Artificial Sequence)
MKASRVIVVASVVALILAGLAMSSAAVIVVPLLSVGAGALDDNSGAGGVGGDPCIGTVTGGAVSVGGLTTRQKQLVTTIVTVVQRDKLPVQAAVIAIMTAKQESDLGANPAATKPNGDGDAGPFQQRVLPGWYGTLDQVNNDAYATETFLKGHTITYAGPTSAGGPGYHIPGLVDVPDWQSKSPAQAAQAVQASALPNAYAKWEAIAKQMVGATTTGRLSNDCVTGTANETGVSKNLTKAVEWAKSIAANNSYTYVWGGNGASDGGYDCSGLTSALYRRIGINLPRTAAEQQKVGTPVNRNQLKVGDLIFWGIPAHHVATYIGRGQMISADNQARGINVEKIYGNPSSYRRIVK

SEQ ID NO: 15 - protein, 280 aa, Artificial Sequence
MDWTNLNADVTKLMNVHFTPGREGRTIDKIVIHHNGGNLSIDQIWNVWQDREASAHYQVESSGRIGQLVNDWDTAWHAGDWDANLTSIGIEHADDSTDPWHVSDAAIDSGAHLVAALCRAYNLGRPEWMHNVFPHSHFSATSCPASLAENQRADYMSRAQAYYDGTSVAAAPAAPSAPAGIHVDLPSWTLPIGHYYGLVTGPNDSHGGFYESERPAVRAIQLWLIRHGYAGAVPDSWADGIYEQPTADAVTAFQHAERPNSTDRWGEVWADDLATMAANN

SEQ ID NO: 16 - protein, 283 aa, Artificial Sequence
MDWTNLIADTTKLMGVHFTPGREGRKIDKIVIHHNGGNLSIDQIWNVWQTREASAHYQVETGGRIGQLVNDWDTAWHAGDWDANLTSIGIEHADDSTDPWHVSDAAVDAGAHLVAALCKAYSLGRPEWMRNVFPHSHFSATSCPASLAENQRADYMSRAQAYYDGAPVAAVHQSAPAPAPASSRHVDLPAWNLPEGNFYGLASGGEDSHGGFYEGERPAIRQIQLWLIRHGYAGAVPDSWADGIYEQPTADAVAAFQHAERPNSTDRWGEVWADDLATMAANN

SEQ ID NO: 17 - protein, 290 aa, Artificial Sequence
MMRMLKAASPWLLRACVLLVALSFVIEVPVWLVFAPLGLAIAVPSPRADDESPQTMHAPVTGRWVAINSPATKVPSHGVRTLGQAFAVDILQASDSPRESAPGWQWRQAEPQEFPSFGEPVLAAGCGTVIAAHDGKRDHRARNTWPGLIYMMSLEAFGRELAGHRSIIGNHVILDHSDGTFSMYAHLKHGSAAVCVGQKVRAGDVLGAVGNTGNTSEPHLHFQLMDRPQAAMAAGLPFRWSPLTIEPDPDPHWAPKKPVAETVEGLPATGQIFRTPESGVMPQPKREASC

SEQ ID NO: 18 - protein, 252 aa, Artificial Sequence
MRRSVCISLLIITVGICLLAFPAPSHSIAAVPARSVANRPTPPVLGPVIKGFAPPAEKWLPGSRGVEFAASVGEPVTTVTAGVVVFAGQVAGAGVVSILLADGRRTTHMPVVPSVAVGQVVVPGQQIGVVGMGPPCTRTCLHWGLKKGDVYQNPMTLLQLQVRLLPLDSRPHSASGHGWPVRPLSLPGGSRRKAASSGALMPPWRGAGRDAALGIDTTVTEATRGGSGAGMSLAKRSAQSFGGNVGVDLRGG

SEQ ID NO: 19 - protein, 216 aa, Artificial Sequence
MAKTLSRIASVAAAAALAGGVSVTAAQSASADDVNWDAIANCESGGNWSTNTGNGYYGGLQFSQSTWAAYGGSGSASNASREEQIAVAERVLAGQGIGAWPVCGAYAYSGESYTGTNTEGSYGSSYDTSAQDASYDGSYSYDNSYSYDNSAGYDSSSAYSGGYQATREATGTYEIQPGDTLNAIAEAHGTTWQELAALNSSIVDANLIYAGETINV

SEQ ID NO: 20 - protein, 250 aa, Artificial Sequence
MAYPYIGALKHGGKQGKIQRIVIHATVSPCVRGGARNVAKYFQSSAAGGSAHYVVDPGEIIQCVKDDVVAYHAPPNTGTLGIELCDPQAGSPKRWSNEAHQAMLVLAAKLVRELAAKHDVPLVRVTAAQLRAGKRGICSHVAVSDAFGQSDHGDPEVAGPFPWAKFMQLIKEEDDMPSPKEIYEAVWEQDVMAAPDGSKSNPTWKPSSVLTDVDKKVRALQSQVTGLESELAATNAKLDQVLTLLRASVS

SEQ ID NO: 21 - protein, 282 aa, Artificial Sequence
MTFIQAAHRGGTSNTPITRLVIHATCPDVGFPSASRAGRAVSTAEYFASTSRSASAHYVCDISTTVQCLSEATIGYHAPPNAHSIGIEICADGGSRASFEKASHAYTREQWLSPQVWPAVERAAILARDICHRHHIPIRRLSVAQVRAGERGICGHNEVSEAFHQSDHDDPGPYFPWNEFIAAVQGKTTTPEGELSMSDVNTLTKLIKASNDQLHYDIGVVQTQNGNIKKKIDNLSWVKNPVTGKKWSTKDALWSVWYYVLECRNRIQAIENRIYDLEKKVK

SEQ ID NO: 22 - protein, 287 aa, Artificial Sequence
MRYIPAAHHSAGSNKPVNRVVIHATCPDVGFPSASRKGRAVSTANYFASPSSGGSAHYVCDIGETVQCLSESTIGWHAPPNPHSLGIEICADGGSHASFRVPGHAYTREQWLDPRVWPAVERAAILCRQLCDKHGVPKRKLSVADLKAGKRGVCGHVDVTDAWHQSDHDDPGPWFPWDKFMAVVNGHGGGSSSEELSMADVQALHNQIKQLSAQVAQSVNKLHHDVGVVQVQNGDLGKRVDALSWVKNPVTGKLWRSKDALWSVWYYVLECRSRLDRLESAVNDLKK

SEQ ID NO: 23 - protein, 281 aa, Artificial Sequence
MTFIQARHHGGNSNAPITRLVIHATCPDVGYPSASKAGRAVSTANYFATTDRPASAHYVCDIATTVQCLSEETIGYHAPPNSHSIGIEICADGGSHASFEKASHAYTRDQWLSDDVWPAVERAAILARDICQRHRIPVRKLSTAQVKAGLSGICGHDNVSGAFHQSDHDDPGPYFPWDQFMALVQGKPATPGDLTMADISKLTDAIKASNRQLHHDIGVVQTQNGKLREQIERITWVKNPVTGKKWRITDALWSIWHYVLECRTRIQRLDARLSEVEKKVK

SEQ ID NO: 24 - protein, 282 aa, Artificial Sequence
MTFIQAAHRGGTSNTPITRLVIHATCPDVGFPSASRAGRAVSTAEYFASTSRSASAHYVCDISTTVQCLSEATIGYHAPPNAHSIGIEICAAGGSRASFEKASHAYTREQWLSPQVWPAVERAAILARDICHRHHIPIRRLSVAQVRAGERGICGHNEVSEAFHQSDHDDPGPYFPWNEFIAAVQGKTTTPEGELSMSDVNTLTKLIKASNDQLHYDIGVVQTQNGNIKKKIDNLSWVKNPVTGKKWSTKDALWSVWYYVLECRNRIQAIENRIYDLEKKVK

SEQ ID NO: 25 - protein, 283 aa, Artificial Sequence
MTFIQAKHHGGHNNPPVTRLVIHATCPDVGYPSASRAGRAVSTAHYFQETTRPASAHYICDISTTVQCLSEETVGYHAPPNSHSIGIEICADGGSHASFSNPAHAYTREQWLSPQVWPAVERAAMLARGICQRHNIPIRRLSIADVKAGKRGICGHNEVSEAFHQSDHDDPGPYFPWDGFIALVNGHSAPSRQEELTVSDVNMLKGLIQQSNKQLHHDIGVVQTQAGNLRRQLESLSWVKNPVSGKLWRTKDALWSIWYYVLDCRSRLGKLEARLSTLEKKVK

SEQ ID NO: 26 - protein, 267 aa, Artificial Sequence
MTFIQAAHHSSGSNLPPTRVVIHATCPEMGFPKASAKGRAVSTARYFQSASSGGSAHYVVDIGETVQCLGENVIAWHAPPNAHSLGIEICADGGSATSFSNPKVRYTRAQWLSPQVWPAVLRAAALTRKMCSKYGIPVVKLSASDLKAGKKGICGHVDVSNAFHQSDHDDPGPDFPWAEFMAAVKGGTTTQEDEDEMKEADWQRMERLVDARLKYAGIAKNDDPVFKPDKSSSWPWRTALWSISYYATHSYNTICNIARKLGAEVSK

SEQ ID NO: 27 - protein, 284 aa, Artificial Sequence
MKYIPATHHGGHTNTPFTRIVIHATCPDLGFPHASAGGQAKATARYFQSEQSAGSAHYVCDIAETIQCLPDDVIAWHAPPNRRSIGIEICADGGSRSSFQHPEHAYTRSQWLSPQVWPAVARAAALTRDLCHRHNIPMQQLSVADVKAGKHGICGHNDVSEAFHKSDHDDPGPTFPWDQFIKEVRTPGQQDTKPSVPTPSLTEIGDQDMNGCYYNLNSKTRTYLIFDSRSGFYHEFSQGNGNGPMSPDYVNPIAKGWDTGSWPAISPGHAKVLKAALDKVRKGI

SEQ ID NO: 28 - protein, 489 aa, Artificial Sequence
MVAHSVWSGGQARGVHGNPTGGRQVFGWVAPASDEPKTVGQERLVVGLQVTIGAQLLPLMTQLVIWATTRLVPMLKRTGDWLKNHHRQIADLAPKILKVALALAGVFSAIKLVNIATSLTTSILGLVATPVGQVVLAVGAVAAAIAGLVAALIYAYHHCREFHDGGTRWSTASCRPGVGRSGSSRCGCRRRRWRGRRSASPPLHPSLHRTLNPHHVEENDMQFIQAAHHSADPNLPPTRVVIHATCPDVGFPSASRAGRAVGTAGYLASISASGSAHYVCDATETVQYLGEDVIGWLAPPHGHSIGIEICADGGSRASFNNPSHAYSPKQWLSPQVWLAVEKAAHLTRQICHRYAIPMRRLTVAGTPRRGCVRCRRRRSVSRVAGNRRCRWMFLTARRGGPARVQVRLRCPARSPERGPLLGWLPGGGAFVMPRHLPSPVGVIVPGTISSRSQQEIPSQRRTQLRSPDSPPDYPQNRPTPSPEGKKKTS

SEQ ID NO: 29 - DNA, 1509 bp, Artificial Sequence
atgtcacttgggtctggcaggaaggagagaatacataagatggatgttaacacactaagggaggtgatggggaattaccgaaacgttaactatgacgctatggtaggccccatgaatgaggcgatgatcgctgctggatgcactaacctccggcgagctgctatgtggtgtgctcagatcggccacgagtcagaaggcctcaccgcgatggaagagtacgccagcggagctggctacgaaggaaggcttgatctaggcaatactcagcctggagacggagtgcgctacaagggccgaggccctatccagctcacgggtaggtccaactatcgagcctttactacgtgggctagaagcaagggctatacaactatcgactttgaggcggaaccacacaaggtttccgagcctaagtggggattccttgcagcgtccttctattggacggtgaggaggcctgacattaactctctggccgaccagggagatgtaacgagagtaactcacaggattaacggaggagaaaacggactcagtgaccgtatagcgagatataatcgcgcgatggcactcggggaccgaatccttccttcagcctctgagacaggcacacagacatcgaaaacgacggctgcggagaaggtcctggattataagcgagactgggtgaagcaggacacctactataactgcggtcccgcttcttgtcagacagtaatcggcgcagctacagggaattaccctggagaggttgagctggcagcagctctcaagaccacgattaacggaactgactggatcggagtcttccctggagtcctaaacaggtacattcccggaggaaagtactcctccagggagatacctaacgatccgccaaggagcgaccagagagatcagctctggaaggacatcataaactccatcaactccggttatggagtcgtggcaaacattgttgctcctccaagcaactacccgagagcgagctacaagtccacacagtccccagcctatgcaggcggaacagtgtatcactacgttgcggtgatgggttacgccattgacgacagcggaagatctcatgtgtgggtcgcagattccggtttcgcaccctatggctactggatgactctccagcagctatccacgcttatcccaccaaagggatatgcgtactccaccaacattcctcaggaaggactagatatggacgcagtaaagcaaatcatcgactttgttaagggctggacaggcccgatgatccaggacatcaaggacatcagacagcagctgaccggaggcagggatactgtctaccgagaggatggctctgttgaccttgttgccagctacccaggctggaggcagctaggaaccgacaagaacggaaacccgctctctatggtcgatagtatcgcctggagccatgtgaagtcagataagatcatcgagatccttacggctctccaggatcgtatcaccgaactagaaaagaaggttaagtaa

SEQ ID NO: 30 - DNA, 1032 bp, Artificial Sequence
atgaccaagattctgaccatcgaaaaggcacgcgagttcgacgctttcgcgcgcgcccgcgacaacctgtactacgggtacggcgaggcattcacccgtaaccctcgccagtcgaccgactgctccgggctcgtcctgcagtcgggtgcgatcctcggtggccgcaccgactgggtgggaaaccgctacggatcgaccgagtcgttccgcctcgactacgcgatcgtgtacgcgctgggattcaagcgcatgcctcgaggtgggttgccgttcgtgccggtgatgaaggtcggtctgcagcacggtggcggcgggatctactcccacaccgcgtgcacgctgatgttcctcgacaagcccggtggcccgatcaaggagtctgcgcggggcgtcgactgggagtcccagggcgccggcgtcttttactacgagggcgcccgtgcctggaatgatggtctgttccacgatttctggtacctcgacatgcgcctcggtgagctcgcgccgccggtgaacgagatcaacgccgagttcgagcgggcgaagggctggatcggcaagcgcatcgacgtcgctgagaagccctgccccgacggcgaaggcaagtacatcaggtgcgagggcggccatatctacttccacccgaaggtcaacgtcggcgcgaagccgggcgagcgtgcgatcgcgatcccggctgacgtcttcgaggtgtggaagcgccagggattcgagaagggaccgctcggctacccgacgcgccgtcacgccacggtcaacggtgtcggcaccatccaggcatttcagaacggcgcggtctatcgcaagttcggcaccgacggcggcatcgtcaacggcaagatcctcgagcgctgggcgcgcgaaggtcacgagaagggccgcctcggttggcctctcggcgacgagaagttcttcgacggcggtcgcgtccaggcgttcgagaacggtgacgcctacttccaccccaccgcggtggtcgagttcctcaacgatcccgcagcccccaagcagtaa

SEQ ID NO: 31 - DNA, 813 bp, Artificial Sequence
atgcgtccctaccgtgcacgccatctcgccactcctcccacccccgactcgactcccgacacctcatccggtgcgtcgcgccgttccgtcctgcgcgggggtgtcctcggtgccgcggcactgagcaccggcgccgccgccgtcgcgaccccggcggcgaacgccgccggcctctacggacaggacgtctccggctggcagggagagatcgactggtccgcccaggcggacctcggctctcgcttcgcctatgtgaaggccaccgagggtcggtcctaccgcagccccgccttcaaccagcagtaccgcggcgccggcaatgccggcctggtccgcggcggctaccacttcgcccgccccgactccggcggccccgaggagcaggtcgacttcttcctcaacaacggcgggggatggtccgacgacggcatcacgctgccgggcatggtcgacttcgaggcctactccggactgcctcgcgactacgggctgagccagcaggagatgcggaactggatcatggcgttctccactcgctaccgggacagcgtcgggcgtcggcccgtcctctacacgaacctccactggtggaacgacgtggtgggggactggaccccggtcaactccccgctgttcctcgcgtcctacagcagcagcgcgccgaccaccctgccgggccgctggtgggcctacgagatgtggcagtactcggattcgggtcccttcgccggtgactcgaacctctggcacggctccgagtcccagttcgagagcttcgtctccgacggggactaccacgcgatcggcatctga

SEQ ID NO: 32 - DNA, 432 bp, Artificial Sequence
atgaggtttattcctgcggcgcatcattctgccggctcgaatagtccggtgaatagggttgtgatccatgcgacatgccctgatgtggggtttccgtctgcctcacgtaaggggcgggcggtgtctacagcaaactattttgcttccccatcgtcggggggttcggcgcattatgtgtgtgatgttggggagacggtgcagtgcctgtcagaggggactattggttggcatgccccgccgaatccgcattctttgggtatagagatttgcgcggatgggggttcgcacgcctcgttccgtgtgccggggcatgcttacacgagggagcagtggcttgatcctcgcgtgtggcctgcggtggagaaggctgccatcctgtgtagacgtttgtgtgacaaatataaatgcttacacgagggagcagtggcttga

SEQ ID NO: 33 - DNA, 1422 bp, Artificial Sequence
atggcaaccatgcctgtcaaaaaaggcttttatgtcacttcggggtttggcccgcgttggggcactacgcattacggcacggattttggtgttgatggtggctcaggtgggcaccctattttcgctatcaaatctggcactgtgaccgcttctggcccggcttctggttttgggcagtggatcaatgtggatcatcctgcaagtgatggcggtggcttgtcggtgtatgggcacatcatcccagaggtgcgcgtaggtgatcaggtggtggaggggcagcggatcggacgaatcaaccccgatcaaaacactaacggcggggttgcgcctcatcttcatttggagtttcaccgctccgtgtggtcaccacctggtggtgatcgcctcgaccccatgaaaactgtgctcgctggtgcagactggccgggtgatgcgccctcaaattcgagcgcgaaaccggaaacggggaaggtcaaaaacatctttggtgtggatatttccaatcatcaaaatggtattttggctgaattgatcggtgcggaaggttttgaattctgcatcatcaaagccaccgagggtacgtggaaagaccctattttgcattcgcatttggcggatgttcgcaaaaattccggcatgcaggttggcgcatatgtgtatgtgcgtggggaaacctcaccagaagcgcatgctatcgctctacatgagcatctgaatgacacgtcggtgccggttgctttggatattgagcataattccggctctaatcctgatcattggcgggcaattaaaacggcgatcgaggcccgtggctaccgcgtgatcctaacatacttgccggagtggtactggagccaagtcgggcagccaaacttggcggggctaccgccgttgtgggcttcccgttatgtcggcaccacaccaggggttgccagcgtcttatattccacggctggtcggcgtggctggcaaggatacggcggccttgaagttgcgatgtggcagttcaccgaccgggcgcaggtcgcaggccaaaagatcgacgccaatgtttttgagggcacggagaaacagcttcgtgcccttttccatggggacaccccagaaatagaggaggagttcgatatgagcgcagtccaggaaatcaaagactatattgacacccgactgacaggacctgtcggcaccgatgtcaaggacatcaggcagcagatcaccggagggcgcgactctatcccaggtgacctcaaagcgtcttaccctgggtgggatttaggtcagctggtgcgtgcggcacgtgaaaaagaatttactggcctgacgatgatggaaattcttgcagtcaatattgctggtaatgatgatgatttccgtgcagcacgtgttgctgcaggtaccgaggaggctggcaatgctgaataa

SEQ ID NO: 34 - DNA, 1281 bp, Artificial Sequence
atggccgactacttctacccactcagccagggcgctcacgtcaccagcccattcgggccccgagctggcggctatcactggggcaccgactacggccgcgccggaggctccggcggcaacgccgtctacgccccgcaagccggaaccgtcatcatggccggccccgccagcggcttcggcggccccgaccccgccggatggatcgtcatcgaccacccaaccgccgccggcggcggagtcagcgtcctcggccacatcatccgtgaagtcgccgtcggcgacaccgtccgcgccgggcagcgcatcgggcgggtcaatccttcctcggccaccaatggcggcgtggcgccgcacgtccacttcgagcatcaccgttacgtctggtccccgccgggaccggaccgtctggacccgcacgcttggctggccacccgcggcgcccgatggccgggagccccggccacacctacccgaaaggaatccatgaacgcgctcaccgctgacatcgacctgctgacccccaacgacgatggccgggcgacgaagccccgcaaccttttgtgcatccataccttcgaagacgacggcacgtggtcggccgacaggatggcgaagtaccagcagtcgcccgccgccggcggctcgtaccacctggtcattgacctcaacggccgcatcgctcgtgagaacgacgacgcgttcatcccatgggcggcgatgttcacgggcaaccgggtggcgttccacttctcgctgtcgggcaaggcgtcctggacgcgccagcagtggctggcccgtccgaagcagatggacgccctggcgaaggtgctggcggcgtactcgaaggccaagggcatcccgctcatccgccgcggaccgcaggacgtgcgagccgggaagtggggcgtgtgcggccacgacgacatttccaaggcattcggtgagtcgacgcactgggacccgggcccgaacttcccgttcgacgtcgtcatcgacaaggccaaggcgatcctcgccgagccgaagccgacgcccgccccgccgtcggatccggcgccccgtccgattcccccgaaggagactctggtgcccaccacgctcgacaccgtcctgccgtcgctcgtcgacggctccacgttcgaggctccgttggccacgttcatccgcaccgcggacaaacaggcctacgaagccaaccagcggatcgcccgcctggaggcgaagttcgatcggctgctcgatgccatgggcgaaaagcccgaccccaagcccggccagtag

SEQ ID NO: 35 - DNA, 858 bp, Artificial Sequence
atgagatacattcctgcggcgcatcactcggccggctctaatagtccggtgaacagggttgtgattcatgcaacatgcccggatgtggggtttccgtccgcttcccgtaaaggacgggcggtgtccacggcaaactatttcgcgtccccatcggcgggcggttctgcccattatgtgtgtgatgttggggagacggtgcagtgcttgtcggagtctacgattggttggcatgccccgccgaatccgcatagtttgggtatagagatttgcgcggatgggggttcgcacgcctcgttccgtgtgccggggcatgcttacactcgtgagcagtggcttgatccgagggtgtggcctgcggtggagaaggcggctgtgctgtgtagacagttgtgtgacaaatataatgttccgaagaggaaactgtctgtatccgatttgaaggctggcaggcggggtgtgtgcggccatacggatgtgacggatgcgtggcatcagtcggatcatgatgatccggggccgtggtttccgtgggacaggtttatggccgtcgtcaacggcggcagtggagagagtggagagttgagtatggctgatgtgaaagccttgcatgatcagattaaacagttgtcggggcaggtggcccagtcggtgaataagctgcatcacgatgtgggtgtggttcaggttcagaatgggaatcttaaaaagcaggttgattccctgtctatggtgaagaatcctgtgacggggaagctgtggcgtaccagggatgcgatctggtcgatctggtattacgtgttggagtgtcgtagccgtatcggcaagttggaggccgaggtggcccggttgaagaagtga

SEQ ID NO: 36 - DNA, 738 bp, Artificial Sequence
atgtccacggcaaactattttgcttccccatcgtcgggtggttcggcgcattatgtttgcgatattagtgagacggtgcaatgcctgtcggagtctacgatcgggtggcatgccccgccgaatccgcatagtttgggtatagagatttgcgcggatgggggttcgcacgcctcgtttagggtgccagggcacgcttacactcgtgagcagtggctggatcctagggtgtggcctgccgtggagaaggctgccatcctgtgtagacgtttgtgtgacaaatataatgttccgaagcggaaactgtctgtagccgatttgaaggctggcaggcggggtgtgtgcggccacgtggatgtgacggatgcgtggcatcagtcggatcatgacgatccggggccgtggtttccgtgggacaggtttatggccgtcgtcaacggcggtagtggagatagtggggagttaactgtggctgatgtgaaagccttgcatgatcagattaaacaattgtctgctcagcttactggttcggtgaataagctgcaccatgatgttggtgtggtacaggtacagaatggtgatttgggtaaacgtgttgatgccttgtcgtgggtgaagaatccggtgacggggaagctgtggcgcaccaaagacgctttgtggagtgtctggtattacgtgctggagtgtcgcagccgcatagacaggctcgagtctgctgttaacggtttgaaaaagtga

SEQ ID NO: 37 - DNA, 846 bp, Artificial Sequence
atgacattcatccaggcccgccatcacggcggcaactccaacacgccgatcacccggctggtcatccacgccacctgccccgacgtgggctacccgtcggcgtcgaaggccggtagggcagtctccacggcggagtatttcgcgtccacgtcgcggtctgcctcggctcactacgtctgtgacgtatcggcaacggtgcagtgcctctccgaggaaaccatcggctaccacgcgccgcccaacagtcattccatcggcattgagatttgcgccgacggcgggtcccgcgcctcatttgagaaggcttctcacgcatacacccgcgagcaatggctctcgcctcaagtgtggcccgccgtggagcgcgccgccattctcgcccgcggcatctgccaccgccaccacatcccggttcgcaaactcaccaccgcacaggtcaaatcggggatgtcgggtatttgcggacacgacaacgtatccgatgcattccaccaatccgaccacgacgaccctggcccctacttcccgtggaacgaatttatcgccgccatccaaggaaaaaacaccaacaagggagaactcagcatgtccgacgtcaacaccctgaccaagctcatcaaggccagcaacaatcagctccaccacgacattggcgtcgtccagacacagaacggcaccctcaaaagcaagatcgacaacttgtcgtgggtgaagaatcccgtcaccggcaagaagtggtccaccaaggatgcgctgtggtctgtctggtactacgtgctggaatgccgcaaccgcatccaggctatcgaaaaccgcctctctgacatcgaaaagaaggtgaagtga

SEQ ID NO: 38 - DNA, 810 bp, Artificial Sequence
atgacgttcattcaggccgcgcatcacagcagcggctccaatctgccgcccacgagggtggtgatccacgcgacatgccccgaactcggcttcccgagggccagtgcgaagggccgagctgtctcgacagcccgctacttccagtctgcgatctcgggcggctcggcgcactatgttgtcgatgtcggcgaaaccgtgcagtgtctggcagaggatgtgatcgcctggcacgccccgcccaacagccgcagcctggggatcgagatctgcgctgacggcggctcggcgaccagcttcaagaaccccaacgtgcgctacagccgcgcccagtggctcagcccgcaggtctggcccgccgtgctccgtgccgcagcactcacccggcagatgtgccagaagtacggcataccggtcaccaagctcagcgcgtcggacctcaaggccgggaagaagggcatctgcggacacgtcgatgtcagcaatgcgtggcatcagtccgaccacgacgaccccggcccggacttcccctgggccgaattcatggcagccgtcaaaggcggcgccaccaaccccgatgaactggagctcacagtgtctcaattcagtgacctgaccaagcgcctgcagggcatgcaggagcagacccaccacgacctcggcgtcgtccagaccaagctggccaccatggacaccgtcaagaacccccgcaccggcgccaagtggagcctcaaggacgccatctggtcgatctggtactacgtgctggagaacagggaccggatcgccgccctcgagaagaaggtgaagtga

SEQ ID NO: 39 - DNA, 855 bp, Artificial Sequence
atggactggaccaatctgaacgctgacgtgacgaagctgatgaacgtgcacttcacccccgggcgtgaaggccacacgatcgacaagatcgtgattcaccacaacggcggcaacctgagcatcgaccagatctggaatgtgtggcaggaccgtgaagcatcggcccactatcaggtgcaatctgatggccgtatcggccagctcgtcaacgactgggacaccgcctggcacgccggcgactgggacgccaacctgacctcgatcggcatcgagcacgccgacgactcgaccgacccgtggcatgtgtcggatgccgccgtcgatgccggcgcgcacctggtggctgcactgtgtcgcggctacaaccttggccggccggagtggatgcgcaacgtcttcccgcactcgcatttctcggcgacctcgtgcccggcctcgcttgccgagaatcagcgcgcggattacatggcgcgcgctcaggcctatttcgatggcgctcccgtcacaggccgttcttcggtccctgcaccggctccggcgcctgccgggatccatgtggacctgcctgcctggactctccccgcaggcaacttttacgggtcgatcgatggcggcgaggactcgcatggcggctactacgagggtgagcgtcctgcaatcgcagcgattcagcgctggcttatccgccacggctacgcgggtgcagtggacgactcatgggccgatggtctgtacgagcagcccaccgtcgacgccgtgacccgcttccagcgtgccgagcgaccaaactccacggaccggtggggcgaggtctgggccgacgatctggccaccatggccgccaacaacggctga

SEQ ID NO: 40 - DNA, 897 bp, Artificial Sequence
atggatcgtggtattgacgtgtcgtcctatcaggcccccgatggtggcctgctggagggcatgtcgttttgcatcatcaaggccaccgaaggcaccggctatgtgaacccgaaccgtacccagtggtacaaggtcgccacggatcgtggggtgaccaccggcgcctatcacttcatgcgtggcggcgatcccgtggcgcaggccgattacttcctcgcgcatctgcccggtgatgtcgattggctcgcccttgatgtcgaggatcccagcgacggcctgtcatgggccgggcgcgtcagcttcatcctcgcctggaccgatcgggtgaaggcgaccggcaagcccaccttggtctattgctcgcgctcctgggcgaatgccctgttgggtgcggccagcagcgacgagcgggcacggctcgcgcaattgccgctgtggatggctgattacacccaacgccccggcgaatattcggggccgtggccgggcggctggccgattgccatacaccagtacacctcggccccgatcgacaagaacgtcctgctcaccgacgatctccaaggaggagacgacatgcccctgtcaaccgacgaccttcgaaatatcgccactgccgtgtggggtggcggcggcgctgcaagcccaatgtatgccgaccggctcgatgggcatcaagaatatccggagacagcccttttcagcctgcaacagcggctgggtgcccgcttcggtgagctgtcgggcaagatcgacggtctggccgaggcgctcaagcaggtgcagggagggaacggcgtggacgcggacgccattagggctgctgctgccgaaggagccaaggctggcgtgcaggcgatgatcgacaccgccacggtgaatctggaggccaagtga

SEQ ID NO: 41 - DNA, 894 bp, Artificial Sequence
atgtgcggggctttctcattcctcaaagacttggagacattcatggactggaccaatctgaacgctgacgtgacgaagctgatgggcgtgcacttcacccccggacgtgaaggcaggacgatcgacaagatcgtgatccaccacaacggcggcaacctgagcatcgaccagatctggaatgtgtggcagacccgtgaagcctccgcgcattatcaggtggaggcgggtggccgtatcggccagctcgtcaacgatttggacaccgcgtggcatgccggcgactgggacgccaacctgacctcgatcggcatcgagcatgccgacgactcgaccgacccgtggcatgtgtctgatgctgccgtcgatgccggcgcgcacctggtggctgcactgtgtcgcggctacaaccttggccggccggagtggatgcgcaacgtcttcccgcactctcagttcacgtccacgtcgtgcccggcgtcgctggcccgggaccagctcggcgactacatggggcgcgcacaagcctacttcgatggcgcgccggtggctgcggtccatcagtcggtccctgcccccgccccagcgcccagccgtcatgtggacctgcccgcgtggaatctccccgagggcaacttctacggcctcgtcagcggcggaaacgactcccacggcggcttctatcccgccgagcgtcccgctgtgagggccatccagctgtggctcatccgtcacggctacgccggcgcggtgcctgacagttgggcggacggcatctacgagcagccgaccgccgacgccgtgaccgctttccagcacgccgagcgccccaacagcacggaccggtggggcgaggtctgggccgacgacctggccaccatggccgccaacaactga

SEQ ID NO: 42 - DNA, 1065 bp, Artificial Sequence
atgaaggcgtctcgcgtgatcgtcgtagcaagtgtcgtagcactgatccttgcgggcctggcaatgtcgtcagctgccgtgattgtggtgccactactgtcagtaggcgccggggccctcgacgacaactctggcgctggcggcgtcggtggggatccctgcataggaactgtcaccggtggcgctgttagtgtcggaggcctcacaaccaggcagaagcaactagtgaccaccatcgtcaccgtggtccaacgcgacaaactacctgtccaggctgcggtcatcgccatcatgaccgctaaacaggaatcagacctcggagccaaccccgccgcaacgaaacctaacggtgacggcgacgccggcccattccaacagcgcgttctaccgggctggtacggcaccttggaccaagtcaacaatgatgcctacgccacggagacattcctgaaaggccacaccatcacctatgctggccccacatcggccggcggccccggctaccacattcccggccttgtcgatgtccccgactggcagtcgaaatccccggcccaagcagcccaagcggttcaggcctcagccctgcctaacgcttacgctaaatgggaggccatcgccaaacagatggtgggagccaccaccacagggcgcctgtccaacgactgtgtcaccgggaccgctaacgaaaccggcgtctcaaagaacctgaccaaagccgtggaatgggccaaatcgatcgccgccaacaactcctacacctacgtgtggggcggtaatggtgcgagcgatggcggctacgactgctcaggcctgacctcggcactgtaccgacgtatcggcatcaaccttccccgcaccgctgccgaacagcaaaaagtcggcaccccagtcaaccgcaaccagctcaaagtcggcgaccttatcttctggggcatccctgcccaccacgtagccacctacatcggtagaggccagatgatcagcgccgacaaccaagcccgcggcatcaacgtggagaagatctacggcaacccctcgagctaccgaaggatcgtcaaatga

SEQ ID NO: 43 - DNA, 843 bp, Artificial Sequence
atggactggaccaatctgaacgctgacgtgaccaagctgatgaacgtgcacttcacccccggacgtgaaggcaggacgatcgacaagatcgtgatccaccacaacggcggcaacctgtcgatcgaccagatctggaatgtgtggcaggaccgtgaagccagcgcgcactaccaggtggaatcgagcggccgcatcggccagctcgtcaacgactgggacaccgcctggcatgccggcgactgggacgcgaatctcacgtcgatcggcatcgagcatgctgacgactcgacggatccgtggcatgtgtcggatgccgccatcgacagcggcgcccatctggtggcggccctgtgccgcgcctacaatcttggtcggccggagtggatgcacaacgtgttcccgcactcgcatttctcggcgacctcgtgcccggcctcgctggccgagaatcagcgcgcggattacatgtcacgggctcaggcctactacgacggcacttcagtggctgccgcacctgctgccccgtcggcacctgccgggatccacgtcgatcttccgagctggaccctcccgatcgggcattattacgggctggtcacagggccgaatgactcgcatggtggcttctacgagtccgagcgtcccgctgtgagggccatccagctgtggctcatccgccacggctacgccggcgcggtgcctgacagttgggcggacggcatctacgagcagccgaccgccgacgccgtgaccgctttccagcatgctgagcgacccaacagcacggaccggtggggcgaggtctgggccgacgatctggccaccatggccgccaacaactga

SEQ ID NO: 44 - DNA, 852 bp, Artificial Sequence
atggactggaccaacctcatcgccgacaccacgaagctcatgggcgtgcacttcacccccgggcgtgaaggccgcaagatcgacaagatcgtgatccaccacaacggcggcaacctgagcatcgaccagatctggaatgtgtggcagacccgcgaagccagcgcgcactaccaggttgagacgggtggccgcatcggccagctcgtcaacgactgggacaccgcctggcacgccggcgactgggatgcgaatctcacgtcgatcggcatcgagcacgccgacgactccacggacccgtggcatgtgtcggatgccgccgttgacgccggcgcgcaccttgtcgcggccctgtgcaaggcctacagtcttggtcgtcctgagtggatgcgcaacgtcttcccgcactcgcatttctcggcgacctcgtgcccggcctcgctggccgagaatcagcgcgcggattacatgtcacgggctcaggcctactacgacggcgcgccggtggctgcggtccatcagtcggcacctgcccccgccccagcgtccagccgtcacgtggacctgcccgcgtggaatctccccgagggcaacttctacggcctggcgagcggtggcgaggattcgcacggcggcttctacgagggtgagcgtcccgcgatccgccagatccagctgtggctcatccgtcacggctatgccggcgcggtgcctgacagttgggcggacgggatctacgaacaacccactgccgacgccgtggccgctttccagcatgctgagcgtcccaactccacggaccggtggggcgaggtctgggcagacgatctggccaccatggccgccaacaactga

SEQ ID NO: 45 - DNA, 873 bp, Artificial Sequence
atgatgcgcatgctcaaggcggcttccccctggctccttcgagcctgcgtcctgctcgtggcgctgagcttcgtcatcgaggtccccgtgtggctcgtgttcgcgccgctgggcctggcgatcgcagtcccttctccacgtgcagacgacgagtctccccagaccatgcatgctcccgtgacgggccgctgggtcgccatcaacagcccggcgacgaaggtccccagccacggcgttcgcacgctcggtcaggcattcgcagtcgacatcctgcaggcatcagactctccccgcgaaagcgcccccggctggcaatggagacaggccgagccccaggagttcccaagcttcggggagcctgtcctggcagcgggctgcggcaccgtgatcgctgcccatgacggcaagcgtgaccatcgcgcccggaacacctggcccggcctgatctacatgatgtcgctcgaggccttcggtcgagagttggccgggcaccgctccatcatcggcaatcacgtgatcctcgaccatagcgacggcacgttcagcatgtacgcccacctcaagcacggatctgcagccgtgtgcgtcgggcagaaagtccgggccggcgatgtcctgggagcggtcgggaacaccgggaataccagcgaaccccatctccacttccagctgatggaccggccccaagcggccatggccgccggcctgccgttccggtggtccccgctcacgatcgagccggatcccgatccccactgggctccgaagaaacctgtcgcagagacggtcgagggcctgcccgcgacagggcagatcttccgcaccccggagtccggcgtcatgccccaacccaagcgcgaggccagttgttga

SEQ ID NO: 46 - DNA, 759 bp, Artificial Sequence
atgaggagatctgtctgcatcagcctactaatcatcacggtggggatttgcttgctggccttcccagctcccagccacagcattgctgccgttcccgcgcgaagtgtggcgaatcgtccgactccgccggtgctaggccccgtcatcaaagggtttgcgccacctgccgaaaaatggctgccgggtagtaggggagtggaatttgcggcctccgtgggagaaccagtgacgaccgtgacggctggggtggtcgtttttgctggccaggtcgcgggggctggggtggtgagcatcctgcttgctgacggtcgtcggacaacccacatgccggttgtgcctagcgttgctgtcggccaggtagtggttcctggccagcagatcggagttgtcgggatggggccaccatgcacccgcacttgtttgcactgggggttgaagaagggagatgtttatcaaaaccccatgacattgttgcaacttcaggtgcggttgctgcccttggacagtcggcctcattcagcgtcggggcacggatggcctgtgcggcccctgagcctgccagggggcagcaggaggaaagctgcctcaagcggtgccctcatgcctccgtggcgtggagctgggcgggacgccgcgttaggcattgatacgacggtgaccgaagccacccgaggtggctcaggcgcggggatgagcctggcgaaacgcagtgcgcaatctttcggtggaaacgtgggtgtagatctgcgtggtggctag

SEQ ID NO: 47 - DNA, 651 bp, Artificial Sequence
atggcaaagacactctctcgaattgcttccgttgcggctgcggctgccctcgccggtggcgtctccgtgactgcggcgcagagcgcgtcggcagacgatgtcaactgggacgccatcgcaaactgcgagtccggcggtaactggagcacaaacaccggcaatggctactacggtggccttcagttctcccagagcacttgggccgcctacggtggctccggtagcgcctccaatgcctcccgtgaggagcagatcgccgtggccgagcgcgtgctcgcgggccagggcatcggtgcgtggccggtctgcggcgcgtacgcctactccggtgaaagctacaccggcaccaacaccgagggttcctacggctcttcgtacgacacgtcggcccaggacgcctcctacgacggctcgtactcgtatgacaactcgtactcgtacgacaacagcgccgggtacgactcgtcctccgcctactccggcggctaccaggccactcgtgaggccactggcacctacgagatccagccgggcgacaccctcaacgccatcgctgaggcccatggcaccacctggcaggagctcgcggccctcaacagctccatcgtcgacgcgaacctgatctacgccggcgaaaccatcaacgtctga

SEQ ID NO: 48 - DNA, 753 bp, Artificial Sequence
atggcctatccctatatcggggcattgaagcatggcggcaagcagggcaagatccagcggatcgtcatccatgccacggtttcgccctgtgtgcggggcggtgcccggaacgtcgcgaagtactttcagagttcagccgccggaggcagcgcccactacgtggtggatcccggtgagatcatccagtgtgtcaaggacgacgtggtggcctaccacgcgccgcccaacaccggaacgctcgggatcgagctgtgcgacccgcaggccggatcgccgaagcggtggagcaacgaggcccaccaggcgatgctcgtgctcgccgcgaagctcgtcagggaactcgcggcgaagcacgacgtgccgctcgtccgggtgaccgccgcgcagctcagggcgggcaagcgcggcatctgctcgcatgtcgcggtcagcgacgcgttcgggcagtccgaccacggcgatcccgaggtcgccgggccgttcccctgggcgaagttcatgcagctcatcaaggaggaggacgacatgccgtcgcccaaggagatctacgaagccgtctgggagcaggacgtcatggcggcccccgacggttccaagtcgaacccgacctggaagcccagcagcgtcctcaccgacgtcgacaagaaggtccgcgccctgcagagccaggtcaccggcctcgagagcgagctggccgccaccaacgccaagctcgaccaggttctcaccctgctccgcgcctcggtgtcctga

SEQ ID NO: 49 - DNA, 849 bp, Artificial Sequence
atgacattcatccaggccgcccaccgtggcggcacttccaacacgccgatcacccggctggtcatccacgccacctgccccgatgtcggcttcccgtcggcatcgcgggcaggacgagcagtatccacagcggaatatttcgcgtccacgtcgaggtcagcctcggcgcactacgtatgcgacatctctaccacggtgcagtgcctgtccgaggcaacgatcggctatcacgcgccaccaaacgcccactccatcggcattgaaatctgcgccgacggaggctcgcgcgcttcatttgagaaggcttctcacgcatacacccgcgagcaatggctcagcccgcaggtatggcccgccgtggagcgcgccgcgattctcgcccgcgacatctgccaccgacaccacatccccatccgccgcctctccgtcgcgcaggtgcgggcaggtgagcgcggaatctgcggccacaacgaggtgagcgaggcgttccaccaatccgaccacgacgaccccggcccctatttcccttggaatgaatttattgccgccgtccaaggaaaaaccaccacaccagagggagaactcagcatgtcagacgtaaacaccctgaccaagctcatcaaggccagcaacgaccagcttcactacgatattggcgtcgtccagacgcaaaacgggaacatcaagaagaagatcgacaatctgtcgtgggtgaagaaccccgtcaccggcaagaagtggtccactaaggatgccctgtggtccgtctggtattacgtgctggaatgccgcaaccgcatccaggctatcgagaaccgtatttacgaccttgagaagaaggtgaagtga

SEQ ID NO: 50 - DNA, 864 bp, Artificial Sequence
atgagatacattcctgcggcgcatcattctgccggatcaaataagccggtgaaccgggttgtgattcatgcaacatgcccggatgtggggtttccgtctgcttcgcgtaagggtcgggcggtgtctacagcaaactattttgcttccccatcgtctggtggttcggcgcattatgtgtgtgatattggggagacggtgcagtgcttgtcggagtctacgattggttggcatgccccgccgaatccgcatagtttgggtatagagatttgcgcggatgggggttcgcacgcctcattccgtgttccagggcatgcctatacgcgggagcagtggcttgaccctcgggtgtggcccgcggtggagagggccgccatcctgtgtcggcagttgtgtgataagcatggtgttccgaagaggaaactgtctgtggctgatttgaaggccggtaaacggggtgtttgcgggcatgtggatgttacggatgcgtggcatcagtcggatcatgacgatccggggccgtggtttccgtgggacaaatttatggctgtggtgaatggccacggcggcggttcaagtagtgaggagttgagtatggctgatgtacaagcgttacataatcagattaaacagttgtcggcacaggtggcccagtcggtgaataagctgcatcacgatgttggtgtggttcaggttcagaatggtgatttgggtaaacgtgttgatgccttgtcgtgggtgaagaatccggtgacggggaagctgtggcgcagcaaggatgctttgtggagtgtctggtattacgtgttggagtgtcgtagccgtcttgacaggctcgagtctgctgtcaacgatttgaaaaagtga

SEQ ID NO: 51 - DNA, 846 bp, Artificial Sequence
atgacattcatccaggcccgccaccacggcggcaactccaacgcgccgatcacccggctggtcatccacgccacctgccccgacgtgggctacccgtcggcatcgaaggccggtagggcagtctcgaccgcgaactacttcgccacgactgatcggcccgcctcggcacattacgtatgtgacatcgccactacagtgcagtgcctctccgaggaaaccatcggctaccacgcgccgccgaactcgcattccatcggcattgaaatttgcgccgatggcgggtcgcacgcctcatttgagaaggcttctcacgcatacacccgcgaccaatggttgagcgatgacgtgtggcccgccgtagagcgcgccgccattcttgcccgcgatatttgccaacgacaccgcatcccggttcgtaaactctccaccgcacaggtgaaagccggactgtcgggaatttgcggacacgacaatgtatccggcgcattccatcagtccgaccacgacgacccgggcccctacttcccgtgggaccagttcatggcactcgtccaaggaaaacccgccacaccaggagatctcaccatggcagacatcagcaaactcaccgacgcgatcaaggcatccaaccggcagctgcaccacgacatcggcgtagtacagacccaaaacggaaaattacgtgagcagatcgaaaggatcacctgggtcaaaaatccggtgacaggaaagaagtggcgcatcaccgacgcgctgtggtcgatctggcactacgtgctggaatgccgcacccgcatccagcggctcgacgcccgtctgtctgaggtcgagaagaaggtgaagtga

SEQ ID NO: 52 - DNA, 849 bp, Artificial Sequence
atgacattcatccaggccgcccaccgtggcggcacttccaacacgccgatcacccggctggtcatccacgccacctgccccgatgtcggcttcccgtcggcatcgcgggcaggacgagcagtatccacagcggaatatttcgcgtccacgtcgaggtcagcctcggcgcactacgtatgcgacatctctaccacggtgcagtgcctgtccgaggcaacgatcggctatcacgcgccaccaaacgcccactccatcggcattgaaatctgcgccgccggaggctcgcgcgcttcatttgagaaggcttctcacgcatacacccgcgagcaatggctcagcccgcaggtatggcccgccgtggagcgcgccgcgattctcgcccgcgacatctgccaccgacaccacatccccatccgccgcctctccgtcgcgcaggtgcgggcaggtgagcgcggaatctgcggccacaacgaggtgagcgaggcgttccaccaatccgaccacgacgaccccggcccctatttcccgtggaatgaatttattgccgccgtccaaggaaaaaccaccacaccagagggagaactcagcatgtcagacgtaaacaccctgaccaagctcatcaaggccagcaacgaccagcttcactacgacattggcgtcgtccagacgcaaaacgggaacatcaagaagaagatcgacaatctgtcgtgggtgaagaaccccgtcaccggcaagaagtggtccactaaggatgccctgtggtccgtctggtattacgtgctggaatgccgcaaccgcatccaggctatcgagaaccgtatttacgaccttgagaagaaggtgaagtga

SEQ ID NO: 53 - DNA, 852 bp, Artificial Sequence
atgacattcattcaggccaagcatcacggcggccacaacaaccctcccgtgactcgtcttgtcattcacgccacatgcccggatgtgggctatccgtctgcgtcgcgcgctggccgtgcggtgtcgacggcccactattttcaggaaacgacccggccagcatccgcccactacatttgtgacatatcgaccacggtgcagtgtctgtctgaggagacggtgggctatcacgccccgccgaactcacactccatcggtattgagatatgcgctgacggtgggtcgcatgcctcgttttcgaaccctgcccacgcctacacccgcgagcagtggttgagccctcaggtgtggcctgctgtggagcgtgccgcgatgctggcgcgcggtatctgtcaacgccacaacatcccgatccgccgcctctcgatcgctgacgtcaaggccgggaagcgcggcatctgcggccacaacgaggtgtccgaggccttccaccaatccgaccatgacgaccccggtccttatttcccgtgggacgggtttatcgcgcttgttaatggccattccgcaccatcacgccaggaggaactaactgtgtcagatgtcaatatgctcaaaggtcttattcagcaatcgaacaagcagctgcaccacgatatcggtgttgtgcagacgcaggcgggtaacctccgccgccagctggaatccctgtcatgggtgaagaacccggtcagcggcaagctgtggcgcaccaaggacgccttgtggtcgatctggtactacgtgctggactgccgatctcgtctcggcaaactcgaggcccgcctgtcgacgctggaaaagaaggtgaagtga

SEQ ID NO: 54 - DNA, 804 bp, Artificial Sequence
atgacgttcattcaggccgcgcatcacagcagcggctccaatctgccacccacgagggtggtgatccatgcgacatgccccgagatgggattcccgaaggccagtgcgaagggcagggctgtctcgacggcccgatacttccagtctgcgagctcgggcggtagcgcccactatgttgtcgacatcggcgagacggtgcagtgtctcggtgagaacgtgatcgcgtggcacgccccgcccaatgcccacagtctcggcatcgagatctgcgcggacgggggatcggccacctccttctccaatcccaaggtgcgctacacgcgggcgcagtggctgagcccgcaggtgtggcccgccgtgctccgtgccgcagcactcacccggaagatgtgcagcaagtacggcatccccgtcgtcaagctgtccgcgtcggacctcaaggccggaaagaagggcatctgcggccacgtggatgtcagcaatgctttccaccagtccgaccacgacgaccccggccccgacttcccgtgggccgaattcatggcagccgtcaaaggcggcaccaccacacaggaagatgaggatgaaatgaaggaagctgactggcagcgcatggagaggctcgttgacgcgaggctgaagtacgctggtatcgccaagaatgatgacccggtcttcaagcccgacaagtcctcgtcgtggccctggaggaccgcgctgtggagcatctcctactacgcgacccacagctacaacacgatctgcaatatcgcccgcaagctcggcgcagaggtgtccaagtga

SEQ ID NO: 55 - DNA, 855 bp, Artificial Sequence
atgaaatacattcccgcgacacatcacggaggccacacgaacacccccttcacccggatcgtgatccacgccacctgccccgaccttggcttcccccacgcatcagctggtggacaggcaaaagccaccgcacgctatttccaatcagagcagtctgccggatcagcacactatgtgtgcgacatcgccgagactatccaatgcctgcccgatgacgtgatcgcctggcacgccccaccaaacagaaggtcgatcggaatcgaaatatgtgccgacggcggctcccgctcctcattccagcaccccgagcacgcctacaccagatcccaatggctcagcccccaagtgtggcccgccgtcgcccgtgccgccgcgctcacccgcgacctctgccaccgccacaacattccgatgcaacaactctccgttgctgatgtgaaagccgggaagcacggaatctgcggccacaacgacgtatccgaggcattccacaagtccgaccatgacgaccccggccccacattcccgtgggaccaattcatcaaagaggttagaacaccaggacaacaagatacgaaaccttccgtaccaacaccatcactcacagaaataggagatcaggacatgaacgggtgctactacaacctcaattcgaaaacacggacgtaccttatcttcgatagccgttccggattttaccacgaattctcccaaggcaatgggaacggccccatgagcccagactatgtaaatccgatcgccaaaggatgggacaccggatcatggccggcaatctccccaggccacgcgaaagtgctcaaggccgccctcgataaagtccggaaaggaatctga

SEQ ID NO: 56 - DNA, 1470 bp, Artificial Sequence
atggtggcccactcggtgtggtcgggcgggcaggcccgtggcgtccacggcaacccgaccggcggccggcaggtgttcggctgggtggcgccggcctcggatgagccgaagacggtaggccaggagcggctggtggtgggcctgcaggtcacgatcggcgcccagctgcttccgctgatgacccagctggtgatatgggccaccacgcggctggttcccatgctcaagcgcaccggcgactggttgaagaatcaccacaggcagatcgccgacctggcgcccaagatcctcaaggtggccctagcgctggccggggtgttctcggcgatcaagctagtcaacatagcgacctcgctcaccacgtcgatcctcgggctggtggccaccccggtcggccaggtggtgctcgccgtcggcgcggtcgccgccgctatcgccggcctcgtggcggccctcatctacgcctaccaccactgtagggagttccacgacgggggaacaaggtggtccacggcatcatgcaggcctggcgtgggccgatccggctcttcacggtgtgggtgccgcaggcggcggtggcgggggcgacggtctgccagcccgcccctacaccccagcctgcaccgaaccctgaacccacaccacgttgaggagaacgacatgcaattcattcaggccgcgcaccattcggccgaccctaaccttccaccaacacgcgtcgtcatccacgccacctgccctgacgtcggattcccctccgcctcccgggcgggccgggcggtgggcaccgccggctacttagcctccatctcggcgagcggatccgcccactatgtgtgcgacgccaccgagacggtccagtacctgggcgaggacgtcatcggctggcttgccccgccccacggccactcgatcggcatcgaaatctgcgccgacgggggctcacgggcctccttcaacaaccccagccacgcctactcgcctaagcagtggctgtccccacaggtgtggctggcggtggagaaggccgcccacctcacccggcagatctgccacaggtatgccatccccatgcgcaggctcacggtcgccggcacacctcgtcgagggtgcgtgaggtgtcggaggcggcggtcagtgtcgagggtggcagggaaccgccggtgtcggtggatgttcctgacggcccgccgcggcgggccggcgagagtgcaggttcgactgcggtgccccgcacggtcgcctgagcgtggcccccttcttggctggctgccgggagggggcgctttcgtcatgcccaggcacttgccgagcccggttggggtaatcgtacccggtacgatctcatctagatctcaacaagaaatccctagtcagcgccgtacccagttacgatcaccggactctccacccgactacccccagaaccgccctactccatcgcccgagggtaagaaaaagaccagctga

SEQ ID NO: 57 - protein, 230 aa, Artificial Sequence
MSLGSGRKERIHKMDVNTLREVMGNYRNVNYDAMVGPMNEAMIAAGCTNLRRAAMWCAQIGHESEGLTAMEEYASGAGYEGRLDLGNTQPGDGVRYKGRGPIQLTGRSNYRAFTTWARSKGYTTIDFEAEPHKVSEPKWGFLAASFYWTVRRPDINSLADQGDVTRVTHRINGGENGLSDRIARYNRAMALGDRILPSASETGTQTSKTTAAEKVLDYKRDWVKQDTYYN

SEQ ID NO: 58 - protein, 210 aa, Artificial Sequence
DRILPSASETGTQTSKTTAAEKVLDYKRDWVKQDTYYNCGPASCQTVIGAATGNYPGEVELAAALKTTINGTDWIGVFPGVLNRYIPGGKYSSREIPNDPPRSDQRDQLWKDIINSINSGYGVVANIVAPPSNYPRASYKSTQSPAYAGGTVYHYVAVMGYAIDDSGRSHVWVADSGFAPYGYWMTLQQLSTLIPPKGYAYSTNIPQEGL

SEQ ID NO: 59 - protein, 402 aa, Artificial Sequence
MSLGSGRKERIHKMDVNTLREVMGNYRNVNYDAMVGPMNEAMIAAGCTNLRRAAMWCAQIGHESEGLTAMEEYASGAGYEGRLDLGNTQPGDGVRYKGRGPIQLTGRSNYRAFTTWARSKGYTTIDFEAEPHKVSEPKWGFLAASFYWTVRRPDINSLADQGDVTRVTHRINGGENGLSDRIARYNRAMALGDRILPSASETGTQTSKTTAAEKVLDYKRDWVKQDTYYNCGPASCQTVIGAATGNYPGEVELAAALKTTINGTDWIGVFPGVLNRYIPGGKYSSREIPNDPPRSDQRDQLWKDIINSINSGYGVVANIVAPPSNYPRASYKSTQSPAYAGGTVYHYVAVMGYAIDDSGRSHVWVADSGFAPYGYWMTLQQLSTLIPPKGYAYSTNIPQEGL

SEQ ID NO: 60 - protein, 106 aa, Artificial Sequence
IPQEGLDMDAVKQIIDFVKGWTGPMIQDIKDIRQQLTGGRDTVYREDGSVDLVASYPGWRQLGTDKNGNPLSMVDSIAWSHVKSDKIIEILTALQDRITELEKKVK

SEQ ID NO: 61 - protein, 262 aa, Artificial Sequence
MTKILTIEKAREFDAFARARDNLYYGYGEAFTRNPRQSTDCSGLVLQSGAILGGRTDWVGNRYGSTESFRLDYAIVYALGFKRMPRGGLPFVPVMKVGLQHGGGGIYSHTACTLMFLDKPGGPIKESARGVDWESQGAGVFYYEGARAWNDGLFHDFWYLDMRLGELAPPVNEINAEFERAKGWIGKRIDVAEKPCPDGEGKYIRCEGGHIYFHPKVNVGAKPGERAIAIPADVFEVWKRQGFEKGPLGYPTRRHATVNGVG

SEQ ID NO: 62 - protein, 102 aa, Artificial Sequence
GFEKGPLGYPTRRHATVNGVGTIQAFQNGAVYRKFGTDGGIVNGKILERWAREGHEKGRLGWPLGDEKFFDGGRVQAFENGDAYFHPTAVVEFLNDPAAPKQ

SEQ ID NO: 63 - protein, 270 aa, Artificial Sequence; identical to SEQ ID NO: 3

SEQ ID NO: 64 - protein, 143 aa, Artificial Sequence; identical to SEQ ID NO: 4

SEQ ID NO: 65 - protein, 161 aa, Artificial Sequence
MATMPVKKGFYVTSGFGPRWGTTHYGTDFGVDGGSGGHPIFAIKSGTVTASGPASGFGQWINVDHPASDGGGLSVYGHIIPEVRVGDQVVEGQRIGRINPDQNTNGGVAPHLHLEFHRSVWSPPGGDRLDPMKTVLAGADWPGDAPSNSSAKPETGKVKNI

SEQ ID NO: 66 - protein, 238 aa, Artificial Sequence
GADWPGDAPSNSSAKPETGKVKNIFGVDISNHQNGILAELIGAEGFEFCIIKATEGTWKDPILHSHLADVRKNSGMQVGAYVYVRGETSPEAHAIALHEHLNDTSVPVALDIEHNSGSNPDHWRAIKTAIEARGYRVILTYLPEWYWSQVGQPNLAGLPPLWASRYVGTTPGVASVLYSTAGRRGWQGYGGLEVAMWQFTDRAQVAGQKIDANVFEGTEKQLRALFHGDTPEIEEEFD

SEQ ID NO: 67 - protein, 375 aa, Artificial Sequence
MATMPVKKGFYVTSGFGPRWGTTHYGTDFGVDGGSGGHPIFAIKSGTVTASGPASGFGQWINVDHPASDGGGLSVYGHIIPEVRVGDQVVEGQRIGRINPDQNTNGGVAPHLHLEFHRSVWSPPGGDRLDPMKTVLAGADWPGDAPSNSSAKPETGKVKNIFGVDISNHQNGILAELIGAEGFEFCIIKATEGTWKDPILHSHLADVRKNSGMQVGAYVYVRGETSPEAHAIALHEHLNDTSVPVALDIEHNSGSNPDHWRAIKTAIEARGYRVILTYLPEWYWSQVGQPNLAGLPPLWASRYVGTTPGVASVLYSTAGRRGWQGYGGLEVAMWQFTDRAQVAGQKIDANVFEGTEKQLRALFHGDTPEIEEEFD

SEQ ID NO: 68 - protein, 110 aa, Artificial Sequence
HGDTPEIEEEFDMSAVQEIKDYIDTRLTGPVGTDVKDIRQQITGGRDSIPGDLKASYPGWDLGQLVRAAREKEFTGLTMMEILAVNIAGNDDDFRAARVAAGTEEAGNAE

SEQ ID NO: 69 - protein, 185 aa, Artificial Sequence
MADYFYPLSQGAHVTSPFGPRAGGYHWGTDYGRAGGSGGNAVYAPQAGTVIMAGPASGFGGPDPAGWIVIDHPTAAGGGVSVLGHIIREVAVGDTVRAGQRIGRVNPSSATNGGVAPHVHFEHHRYVWSPPGPDRLDPHAWLATRGARWPGAPATPTRKESMNALTADIDLLTPNDDGRATKPRN

SEQ ID NO: 70 - protein, 207 aa, Artificial Sequence
IDLLTPNDDGRATKPRNLLCIHTFEDDGTWSADRMAKYQQSPAAGGSYHLVIDLNGRIARENDDAFIPWAAMFTGNRVAFHFSLSGKASWTRQQWLARPKQMDALAKVLAAYSKAKGIPLIRRGPQDVRAGKWGVCGHDDISKAFGESTHWDPGPNFPFDVVIDKAKAILAEPKPTPAPPSDPAPRPIPPKETLVPTTLDTVLPSLV

SEQ ID NO: 71 - protein, 375 aa, Artificial Sequence
MADYFYPLSQGAHVTSPFGPRAGGYHWGTDYGRAGGSGGNAVYAPQAGTVIMAGPASGFGGPDPAGWIVIDHPTAAGGGVSVLGHIIREVAVGDTVRAGQRIGRVNPSSATNGGVAPHVHFEHHRYVWSPPGPDRLDPHAWLATRGARWPGAPATPTRKESMNALTADIDLLTPNDDGRATKPRNLLCIHTFEDDGTWSADRMAKYQQSPAAGGSYHLVIDLNGRIARENDDAFIPWAAMFTGNRVAFHFSLSGKASWTRQQWLARPKQMDALAKVLAAYSKAKGIPLIRRGPQDVRAGKWGVCGHDDISKAFGESTHWDPGPNFPFDVVIDKAKAILAEPKPTPAPPSDPAPRPIPPKETLVPTTLDTVLPSLV

SEQ ID NO: 72 - protein, 86 aa, Artificial Sequence
PKPTPAPPSDPAPRPIPPKETLVPTTLDTVLPSLVDGSTFEAPLATFIRTADKQAYEANQRIARLEAKFDRLLDAMGEKPDPKPGQ

SEQ ID NO: 73 - protein, 195 aa, Artificial Sequence
MRYIPAAHHSAGSNSPVNRVVIHATCPDVGFPSASRKGRAVSTANYFASPSAGGSAHYVCDVGETVQCLSESTIGWHAPPNPHSLGIEICADGGSHASFRVPGHAYTREQWLDPRVWPAVEKAAVLCRQLCDKYNVPKRKLSVSDLKAGRRGVCGHTDVTDAWHQSDHDDPGPWFPWDRFMAVVNGGSGESGELS

SEQ ID NO: 74 - protein, 186 aa, Artificial Sequence
MRYIPAAHHSAGSNSPVNRVVIHATCPDVGFPSASRKGRAVSTANYFASPSAGGSAHYVCDVGETVQCLSESTIGWHAPPNPHSLGIEICADGGSHASFRVPGHAYTREQWLDPRVWPAVEKAAVLCRQLCDKYNVPKRKLSVSDLKAGRRGVCGHTDVTDAWHQSDHDDPGPWFPWDRFMAVVNG

SEQ ID NO: 75 - protein, 99 aa, Artificial Sequence
GSGESGELSMADVKALHDQIKQLSGQVAQSVNKLHHDVGVVQVQNGNLKKQVDSLSMVKNPVTGKLWRTRDAIWSIWYYVLECRSRIGKLEAEVARLKK

SEQ ID NO: 76 - protein, 90 aa, Artificial Sequence
MADVKALHDQIKQLSGQVAQSVNKLHHDVGVVQVQNGNLKKQVDSLSMVKNPVTGKLWRTRDAIWSIWYYVLECRSRIGKLEAEVARLKK

SEQ ID NO: 77 - protein, 164 aa, Artificial Sequence
MSTANYFASPSSGGSAHYVCDISETVQCLSESTIGWHAPPNPHSLGIEICADGGSHASFRVPGHAYTREQWLDPRVWPAVEKAAILCRRLCDKYNVPKRKLSVADLKAGRRGVCGHVDVTDAWHQSDHDDPGPWFPWDRFMAVVNGGSGDSGELTVADVKALHD

SEQ ID NO: 78 - protein, 101 aa, Artificial Sequence
NGGSGDSGELTVADVKALHDQIKQLSAQLTGSVNKLHHDVGVVQVQNGDLGKRVDALSWVKNPVTGKLWRTKDALWSVWYYVLECRSRIDRLESAVNGLKK

SEQ ID NO: 79 - protein, 90 aa, Artificial Sequence
VADVKALHDQIKQLSAQLTGSVNKLHHDVGVVQVQNGDLGKRVDALSWVKNPVTGKLWRTKDALWSVWYYVLECRSRIDRLESAVNGLKK

SEQ ID NO: 80 - protein, 195 aa, Artificial Sequence
MTFIQARHHGGNSNTPITRLVIHATCPDVGYPSASKAGRAVSTAEYFASTSRSASAHYVCDVSATVQCLSEETIGYHAPPNSHSIGIEICADGGSRASFEKASHAYTREQWLSPQVWPAVERAAILARGICHRHHIPVRKLTTAQVKSGMSGICGHDNVSDAFHQSDHDDPGPYFPWNEFIAAIQGKNTNKGELS

SEQ ID NO: 81 - protein, 186 aa, Artificial Sequence
MTFIQARHHGGNSNTPITRLVIHATCPDVGYPSASKAGRAVSTAEYFASTSRSASAHYVCDVSATVQCLSEETIGYHAPPNSHSIGIEICADGGSRASFEKASHAYTREQWLSPQVWPAVERAAILARGICHRHHIPVRKLTTAQVKSGMSGICGHDNVSDAFHQSDHDDPGPYFPWNEFIAAIQG

SEQ ID NO: 82 - protein, 95 aa, Artificial Sequence
KNTNKGELSMSDVNTLTKLIKASNNQLHHDIGVVQTQNGTLKSKIDNLSWVKNPVTGKKWSTKDALWSVWYYVLECRNRIQAIENRLSDIEKKVK

SEQ ID NO: 83 - protein, 86 aa, Artificial Sequence
MSDVNTLTKLIKASNNQLHHDIGVVQTQNGTLKSKIDNLSWVKNPVTGKKWSTKDALWSVWYYVLECRNRIQAIENRLSDIEKKVK

SEQ ID NO: 84 - protein, 90 aa, Artificial Sequence
GELSMSDVNTLTKLIKASNNQLHHDIGVVQTQNGTLKSKIDNLSWVKNPVTGKKWSTKDALWSVWYYVLECRNRIQAIENRLSDIEKKVK

SEQ ID NO: 85 - protein, 197 aa, Artificial Sequence
MTFIQAAHHSSGSNLPPTRVVIHATCPELGFPRASAKGRAVSTARYFQSAISGGSAHYVVDVGETVQCLAEDVIAWHAPPNSRSLGIEICADGGSATSFKNPNVRYSRAQWLSPQVWPAVLRAAALTRQMCQKYGIPVTKLSASDLKAGKKGICGHVDVSNAWHQSDHDDPGPDFPWAEFMAAVKGGATNPDELELT

SEQ ID NO: 86 - protein, 185 aa, Artificial Sequence
MTFIQAAHHSSGSNLPPTRVVIHATCPELGFPRASAKGRAVSTARYFQSAISGGSAHYVVDVGETVQCLAEDVIAWHAPPNSRSLGIEICADGGSATSFKNPNVRYSRAQWLSPQVWPAVLRAAALTRQMCQKYGIPVTKLSASDLKAGKKGICGHVDVSNAWHQSDHDDPGPDFPWAEFMAAVK

SEQ ID NO: 87 - protein, 191 aa, Artificial Sequence
MTFIQAAHHSSGSNLPPTRVVIHATCPELGFPRASAKGRAVSTARYFQSAISGGSAHYVVDVGETVQCLAEDVIAWHAPPNSRSLGIEICADGGSATSFKNPNVRYSRAQWLSPQVWPAVLRAAALTRQMCQKYGIPVTKLSASDLKAGKKGICGHVDVSNAWHQSDHDDPGPDFPWAEFMAAVKGGATNP

SEQ ID NO: 88 - protein, 84 aa, Artificial Sequence
GGATNPDELELTVSQFSDLTKRLQGMQEQTHHDLGVVQTKLATMDTVKNPRTGAKWSLKDAIWSIWYYVLENRDRIAALEKKVK

SEQ ID NO: 89 - protein, 72 aa, Artificial Sequence
VSQFSDLTKRLQGMQEQTHHDLGVVQTKLATMDTVKNPRTGAKWSLKDAIWSIWYYVLENRDRIAALEKKVK

SEQ ID NO: 90 - protein, 78 aa, Artificial Sequence
DELELTVSQFSDLTKRLQGMQEQTHHDLGVVQTKLATMDTVKNPRTGAKWSLKDAIWSIWYYVLENRDRIAALEKKVK

SEQ ID NO: 91 - protein, 215 aa, Artificial Sequence
MDWTNLNADVTKLMNVHFTPGREGHTIDKIVIHHNGGNLSIDQIWNVWQDREASAHYQVQSDGRIGQLVNDWDTAWHAGDWDANLTSIGIEHADDSTDPWHVSDAAVDAGAHLVAALCRGYNLGRPEWMRNVFPHSHFSATSCPASLAENQRADYMARAQAYFDGAPVTGRSSVPAPAPAPAGIHVDLPAWTLPAGNFYGSIDGGEDSHGGYYEG

SEQ ID NO: 92 - protein, 140 aa, Artificial Sequence
ASLAENQRADYMARAQAYFDGAPVTGRSSVPAPAPAPAGIHVDLPAWTLPAGNFYGSIDGGEDSHGGYYEGERPAIAAIQRWLIRHGYAGAVDDSWADGLYEQPTVDAVTRFQRAERPNSTDRWGEVWADDLATMAANNG

SEQ ID NO: 93 - protein, 196 aa, Artificial Sequence
MDRGIDVSSYQAPDGGLLEGMSFCIIKATEGTGYVNPNRTQWYKVATDRGVTTGAYHFMRGGDPVAQADYFLAHLPGDVDWLALDVEDPSDGLSWAGRVSFILAWTDRVKATGKPTLVYCSRSWANALLGAASSDERARLAQLPLWMADYTQRPGEYSGPWPGGWPIAIHQYTSAPIDKNVLLTDDLQGGDDMPLS

SEQ ID NO: 94 - protein, 116 aa, Artificial Sequence
LTDDLQGGDDMPLSTDDLRNIATAVWGGGGAASPMYADRLDGHQEYPETALFSLQQRLGARFGELSGKIDGLAEALKQVQGGNGVDADAIRAAAAEGAKAGVQAMIDTATVNLEAK

SEQ ID NO: 95 - protein, 229 aa, Artificial Sequence
MCGAFSFLKDLETFMDWTNLNADVTKLMGVHFTPGREGRTIDKIVIHHNGGNLSIDQIWNVWQTREASAHYQVEAGGRIGQLVNDLDTAWHAGDWDANLTSIGIEHADDSTDPWHVSDAAVDAGAHLVAALCRGYNLGRPEWMRNVFPHSQFTSTSCPASLARDQLGDYMGRAQAYFDGAPVAAVHQSVPAPAPAPSRHVDLPAWNLPEGNFYGLVSGGNDSHGGFYPA

SEQ ID NO: 96 - protein, 139 aa, Artificial Sequence
ASLARDQLGDYMGRAQAYFDGAPVAAVHQSVPAPAPAPSRHVDLPAWNLPEGNFYGLVSGGNDSHGGFYPAERPAVRAIQLWLIRHGYAGAVPDSWADGIYEQPTADAVTAFQHAERPNSTDRWGEVWADDLATMAANN

SEQ ID NO: 97 - protein, 232 aa, Artificial Sequence
MKASRVIVVASVVALILAGLAMSSAAVIVVPLLSVGAGALDDNSGAGGVGGDPCIGTVTGGAVSVGGLTTRQKQLVTTIVTVVQRDKLPVQAAVIAIMTAKQESDLGANPAATKPNGDGDAGPFQQRVLPGWYGTLDQVNNDAYATETFLKGHTITYAGPTSAGGPGYHIPGLVDVPDWQSKSPAQAAQAVQASALPNAYAKWEAIAKQMVGATTTGRLSNDCVTGTANETG

SEQ ID NO: 98 - protein, 150 aa, Artificial Sequence
AIAKQMVGATTTGRLSNDCVTGTANETGVSKNLTKAVEWAKSIAANNSYTYVWGGNGASDGGYDCSGLTSALYRRIGINLPRTAAEQQKVGTPVNRNQLKVGDLIFWGIPAHHVATYIGRGQMISADNQARGINVEKIYGNPSSYRRIVK

SEQ ID NO: 99 - protein, 354 aa, Artificial Sequence; identical to SEQ ID NO: 14

SEQ ID NO: 100 - protein, 189 aa, Artificial Sequence
MDWTNLNADVTKLMNVHFTPGREGRTIDKIVIHHNGGNLSIDQIWNVWQDREASAHYQVESSGRIGQLVNDWDTAWHAGDWDANLTSIGIEHADDSTDPWHVSDAAIDSGAHLVAALCRAYNLGRPEWMHNVFPHSHFSATSCPASLAENQRADYMSRAQAYYDGTSVAAAPAAPSAPAGIHVDLPSWT

SEQ ID NO: 101 - protein, 123 aa, Artificial Sequence
RAQAYYDGTSVAAAPAAPSAPAGIHVDLPSWTLPIGHYYGLVTGPNDSHGGFYESERPAVRAIQLWLIRHGYAGAVPDSWADGIYEQPTADAVTAFQHAERPNSTDRWGEVWADDLATMAANN

SEQ ID NO: 102 - protein, 204 aa, Artificial Sequence
MDWTNLIADTTKLMGVHFTPGREGRKIDKIVIHHNGGNLSIDQIWNVWQTREASAHYQVETGGRIGQLVNDWDTAWHAGDWDANLTSIGIEHADDSTDPWHVSDAAVDAGAHLVAALCKAYSLGRPEWMRNVFPHSHFSATSCPASLAENQRADYMSRAQAYYDGAPVAAVHQSAPAPAPASSRHVDLPAWNLPEGNFYGLASG

SEQ ID NO: 103 - protein, 126 aa, Artificial Sequence
RAQAYYDGAPVAAVHQSAPAPAPASSRHVDLPAWNLPEGNFYGLASGGEDSHGGFYEGERPAIRQIQLWLIRHGYAGAVPDSWADGIYEQPTADAVAAFQHAERPNSTDRWGEVWADDLATMAANN

SEQ ID NO: 104 - protein, 145 aa, Artificial Sequence
AFAVDILQASDSPRESAPGWQWRQAEPQEFPSFGEPVLAAGCGTVIAAHDGKRDHRARNTWPGLIYMMSLEAFGRELAGHRSIIGNHVILDHSDGTFSMYAHLKHGSAAVCVGQKVRAGDVLGAVGNTGNTSEPHLHFQLMDRPQ

SEQ ID NO: 105 - protein, 290 aa, Artificial Sequence; identical to SEQ ID NO: 17

SEQ ID NO: 106 - protein, 93 aa, Artificial Sequence
GSRGVEFAASVGEPVTTVTAGVVVFAGQVAGAGVVSILLADGRRTTHMPVVPSVAVGQVVVPGQQIGVVGMGPPCTRTCLHWGLKKGDVYQNP

SEQ ID NO: 107 - protein, 252 aa, Artificial Sequence; identical to SEQ ID NO: 18

SEQ ID NO: 108 - protein, 171 aa, Artificial Sequence
MAKTLSRIASVAAAAALAGGVSVTAAQSASADDVNWDAIANCESGGNWSTNTGNGYYGGLQFSQSTWAAYGGSGSASNASREEQIAVAERVLAGQGIGAWPVCGAYAYSGESYTGTNTEGSYGSSYDTSAQDASYDGSYSYDNSYSYDNSAGYDSSSAYSGGYQATREATG

SEQ ID NO: 109 - protein, 113 aa, Artificial Sequence
GAYAYSGESYTGTNTEGSYGSSYDTSAQDASYDGSYSYDNSYSYDNSAGYDSSSAYSGGYQATREATGTYEIQPGDTLNAIAEAHGTTWQELAALNSSIVDANLIYAGETINV

SEQ ID NO: 110 - protein, 176 aa, Artificial Sequence
MAYPYIGALKHGGKQGKIQRIVIHATVSPCVRGGARNVAKYFQSSAAGGSAHYVVDPGEIIQCVKDDVVAYHAPPNTGTLGIELCDPQAGSPKRWSNEAHQAMLVLAAKLVRELAAKHDVPLVRVTAAQLRAGKRGICSHVAVSDAFGQSDHGDPEVAGPFPWAKFMQLIKEEDDM

SEQ ID NO: 111 - protein, 124 aa, Artificial Sequence
MAYPYIGALKHGGKQGKIQRIVIHATVSPCVRGGARNVAKYFQSSAAGGSAHYVVDPGEIIQCVKDDVVAYHAPPNTGTLGIELCDPQAGSPKRWSNEAHQAMLVLAAKLVRELAAKHDVPLVR

SEQ ID NO: 112 - protein, 126 aa, Artificial Sequence
VTAAQLRAGKRGICSHVAVSDAFGQSDHGDPEVAGPFPWAKFMQLIKEEDDMPSPKEIYEAVWEQDVMAAPDGSKSNPTWKPSSVLTDVDKKVRALQSQVTGLESELAATNAKLDQVLTLLRASVS

SEQ ID NO: 113 - protein, 193 aa, Artificial Sequence
MTFIQAAHRGGTSNTPITRLVIHATCPDVGFPSASRAGRAVSTAEYFASTSRSASAHYVCDISTTVQCLSEATIGYHAPPNAHSIGIEICADGGSRASFEKASHAYTREQWLSPQVWPAVERAAILARDICHRHHIPIRRLSVAQVRAGERGICGHNEVSEAFHQSDHDDPGPYFPWNEFIAAVQGKTTTPEG

SEQ ID NO: 114 - protein, 173 aa, Artificial Sequence
MTFIQAAHRGGTSNTPITRLVIHATCPDVGFPSASRAGRAVSTAEYFASTSRSASAHYVCDISTTVQCLSEATIGYHAPPNAHSIGIEICADGGSRASFEKASHAYTREQWLSPQVWPAVERAAILARDICHRHHIPIRRLSVAQVRAGERGICGHNEVSEAFHQSDHDDPGP

SEQ ID NO: 115 - protein, 109 aa, Artificial Sequence
YFPWNEFIAAVQGKTTTPEGELSMSDVNTLTKLIKASNDQLHYDIGVVQTQNGNIKKKIDNLSWVKNPVTGKKWSTKDALWSVWYYVLECRNRIQAIENRIYDLEKKVK

SEQ ID NO: 116 - protein, 90 aa, Artificial Sequence
GELSMSDVNTLTKLIKASNDQLHYDIGVVQTQNGNIKKKIDNLSWVKNPVTGKKWSTKDALWSVWYYVLECRNRIQAIENRIYDLEKKVK

SEQ ID NO: 117 - protein, 213 aa, Artificial Sequence
MRYIPAAHHSAGSNKPVNRVVIHATCPDVGFPSASRKGRAVSTANYFASPSSGGSAHYVCDIGETVQCLSESTIGWHAPPNPHSLGIEICADGGSHASFRVPGHAYTREQWLDPRVWPAVERAAILCRQLCDKHGVPKRKLSVADLKAGKRGVCGHVDVTDAWHQSDHDDPGPWFPWDKFMAVVNGHGGGSSSEELSMADVQALHNQIKQLSA

SEQ ID NO: 118 - protein, 173 aa, Artificial Sequence
MRYIPAAHHSAGSNKPVNRVVIHATCPDVGFPSASRKGRAVSTANYFASPSSGGSAHYVCDIGETVQCLSESTIGWHAPPNPHSLGIEICADGGSHASFRVPGHAYTREQWLDPRVWPAVERAAILCRQLCDKHGVPKRKLSVADLKAGKRGVCGHVDVTDAWHQSDHDDPGP

SEQ ID NO: 119 - protein, 114 aa, Artificial Sequence
WFPWDKFMAVVNGHGGGSSSEELSMADVQALHNQIKQLSAQVAQSVNKLHHDVGVVQVQNGDLGKRVDALSWVKNPVTGKLWRSKDALWSVWYYVLECRSRLDRLESAVNDLKK

SEQ ID NO: 120 - protein, 74 aa, Artificial Sequence
QVAQSVNKLHHDVGVVQVQNGDLGKRVDALSWVKNPVTGKLWRSKDALWSVWYYVLECRSRLDRLESAVNDLKK

SEQ ID NO: 121 - protein, 196 aa, Artificial Sequence
MTFIQARHHGGNSNAPITRLVIHATCPDVGYPSASKAGRAVSTANYFATTDRPASAHYVCDIATTVQCLSEETIGYHAPPNSHSIGIEICADGGSHASFEKASHAYTRDQWLSDDVWPAVERAAILARDICQRHRIPVRKLSTAQVKAGLSGICGHDNVSGAFHQSDHDDPGPYFPWDQFMALVQGKPATPGDLTM

SEQ ID NO: 122 - protein, 173 aa, Artificial Sequence
MTFIQARHHGGNSNAPITRLVIHATCPDVGYPSASKAGRAVSTANYFATTDRPASAHYVCDIATTVQCLSEETIGYHAPPNSHSIGIEICADGGSHASFEKASHAYTRDQWLSDDVWPAVERAAILARDICQRHRIPVRKLSTAQVKAGLSGICGHDNVSGAFHQSDHDDPGP

SEQ ID NO: 123 - protein, 108 aa, Artificial Sequence
YFPWDQFMALVQGKPATPGDLTMADISKLTDAIKASNRQLHHDIGVVQTQNGKLREQIERITWVKNPVTGKKWRITDALWSIWHYVLECRTRIQRLDARLSEVEKKVK

SEQ ID NO: 124 - protein, 86 aa, Artificial Sequence
MADISKLTDAIKASNRQLHHDIGVVQTQNGKLREQIERITWVKNPVTGKKWRITDALWSIWHYVLECRTRIQRLDARLSEVEKKVK

SEQ ID NO: 125 - protein, 193 aa, Artificial Sequence
MTFIQAAHRGGTSNTPITRLVIHATCPDVGFPSASRAGRAVSTAEYFASTSRSASAHYVCDISTTVQCLSEATIGYHAPPNAHSIGIEICAAGGSRASFEKASHAYTREQWLSPQVWPAVERAAILARDICHRHHIPIRRLSVAQVRAGERGICGHNEVSEAFHQSDHDDPGPYFPWNEFIAAVQGKTTTPEG

SEQ ID NO: 126 - protein, 109 aa, Artificial Sequence; identical to SEQ ID NO: 115

SEQ ID NO: 127 - protein, 200 aa, Artificial Sequence
MTFIQAKHHGGHNNPPVTRLVIHATCPDVGYPSASRAGRAVSTAHYFQETTRPASAHYICDISTTVQCLSEETVGYHAPPNSHSIGIEICADGGSHASFSNPAHAYTREQWLSPQVWPAVERAAMLARGICQRHNIPIRRLSIADVKAGKRGICGHNEVSEAFHQSDHDDPGPYFPWDGFIALVNGHSAPSRQEELTVSD

SEQ ID NO: 128 - protein, 173 aa, Artificial Sequence
MTFIQAKHHGGHNNPPVTRLVIHATCPDVGYPSASRAGRAVSTAHYFQETTRPASAHYICDISTTVQCLSEETVGYHAPPNSHSIGIEICADGGSHASFSNPAHAYTREQWLSPQVWPAVERAAMLARGICQRHNIPIRRLSIADVKAGKRGICGHNEVSEAFHQSDHDDPGP

SEQ ID NO: 129 - protein, 110 aa, Artificial Sequence
YFPWDGFIALVNGHSAPSRQEELTVSDVNMLKGLIQQSNKQLHHDIGVVQTQAGNLRRQLESLSWVKNPVSGKLWRTKDALWSIWYYVLDCRSRLGKLEARLSTLEKKVK

SEQ ID NO: 130 - protein, 93 aa, Artificial Sequence
SRQEELTVSDVNMLKGLIQQSNKQLHHDIGVVQTQAGNLRRQLESLSWVKNPVSGKLWRTKDALWSIWYYVLDCRSRLGKLEARLSTLEKKVK

SEQ ID NO: 131 - protein, 200 aa, Artificial Sequence
MTFIQAAHHSSGSNLPPTRVVIHATCPEMGFPKASAKGRAVSTARYFQSASSGGSAHYVVDIGETVQCLGENVIAWHAPPNAHSLGIEICADGGSATSFSNPKVRYTRAQWLSPQVWPAVLRAAALTRKMCSKYGIPVVKLSASDLKAGKKGICGHVDVSNAFHQSDHDDPGPDFPWAEFMAAVKGGTTTQEDEDEMKEA

SEQ ID NO: 132 - protein, 173 aa, Artificial Sequence
MTFIQAAHHSSGSNLPPTRVVIHATCPEMGFPKASAKGRAVSTARYFQSASSGGSAHYVVDIGETVQCLGENVIAWHAPPNAHSLGIEICADGGSATSFSNPKVRYTRAQWLSPQVWPAVLRAAALTRKMCSKYGIPVVKLSASDLKAGKKGICGHVDVSNAFHQSDHDDPGP

SEQ ID NO: 133 - protein, 185 aa, Artificial Sequence
MTFIQAAHHSSGSNLPPTRVVIHATCPEMGFPKASAKGRAVSTARYFQSASSGGSAHYVVDIGETVQCLGENVIAWHAPPNAHSLGIEICADGGSATSFSNPKVRYTRAQWLSPQVWPAVLRAAALTRKMCSKYGIPVVKLSASDLKAGKKGICGHVDVSNAFHQSDHDDPGPDFPWAEFMAAVK

SEQ ID NO: 134 - protein, 94 aa, Artificial Sequence
DFPWAEFMAAVKGGTTTQEDEDEMKEADWQRMERLVDARLKYAGIAKNDDPVFKPDKSSSWPWRTALWSISYYATHSYNTICNIARKLGAEVSK

SEQ ID NO: 135 - protein, 186 aa, Artificial Sequence
MKYIPATHHGGHTNTPFTRIVIHATCPDLGFPHASAGGQAKATARYFQSEQSAGSAHYVCDIAETIQCLPDDVIAWHAPPNRRSIGIEICADGGSRSSFQHPEHAYTRSQWLSPQVWPAVARAAALTRDLCHRHNIPMQQLSVADVKAGKHGICGHNDVSEAFHKSDHDDPGPTFPWDQFIKEVRT

SEQ ID NO: 136 - protein, 173 aa, Artificial Sequence
MKYIPATHHGGHTNTPFTRIVIHATCPDLGFPHASAGGQAKATARYFQSEQSAGSAHYVCDIAETIQCLPDDVIAWHAPPNRRSIGIEICADGGSRSSFQHPEHAYTRSQWLSPQVWPAVARAAALTRDLCHRHNIPMQQLSVADVKAGKHGICGHNDVSEAFHKSDHDDPGP

SEQ ID NO: 137 - protein, 111 aa, Artificial Sequence
TFPWDQFIKEVRTPGQQDTKPSVPTPSLTEIGDQDMNGCYYNLNSKTRTYLIFDSRSGFYHEFSQGNGNGPMSPDYVNPIAKGWDTGSWPAISPGHAKVLKAALDKVRKGI

SEQ ID NO: 138 - protein, 98 aa, Artificial Sequence
PGQQDTKPSVPTPSLTEIGDQDMNGCYYNLNSKTRTYLIFDSRSGFYHEFSQGNGNGPMSPDYVNPIAKGWDTGSWPAISPGHAKVLKAALDKVRKGI

SEQ ID NO: 139 - protein, 102 aa, Artificial Sequence
EVRTPGQQDTKPSVPTPSLTEIGDQDMNGCYYNLNSKTRTYLIFDSRSGFYHEFSQGNGNGPMSPDYVNPIAKGWDTGSWPAISPGHAKVLKAALDKVRKGI

SEQ ID NO: 140 - DNA, 690 bp, Artificial Sequence
atgtcacttgggtctggcaggaaggagagaatacataagatggatgttaacacactaagggaggtgatggggaattaccgaaacgttaactatgacgctatggtaggccccatgaatgaggcgatgatcgctgctggatgcactaacctccggcgagctgctatgtggtgtgctcagatcggccacgagtcagaaggcctcaccgcgatggaagagtacgccagcggagctggctacgaaggaaggcttgatctaggcaatactcagcctggagacggagtgcgctacaagggccgaggccctatccagctcacgggtaggtccaactatcgagcctttactacgtgggctagaagcaagggctatacaactatcgactttgaggcggaaccacacaaggtttccgagcctaagtggggattccttgcagcgtccttctattggacggtgaggaggcctgacattaactctctggccgaccagggagatgtaacgagagtaactcacaggattaacggaggagaaaacggactcagtgaccgtatagcgagatataatcgcgcgatggcactcggggaccgaatccttccttcagcctctgagacaggcacacagacatcgaaaacgacggctgcggagaaggtcctggattataagcgagactgggtgaagcaggacacctactataac

SEQ ID NO: 141 - DNA, 630 bp, Artificial Sequence
gaccgaatccttccttcagcctctgagacaggcacacagacatcgaaaacgacggctgcggagaaggtcctggattataagcgagactgggtgaagcaggacacctactataactgcggtcccgcttcttgtcagacagtaatcggcgcagctacagggaattaccctggagaggttgagctggcagcagctctcaagaccacgattaacggaactgactggatcggagtcttccctggagtcctaaacaggtacattcccggaggaaagtactcctccagggagatacctaacgatccgccaaggagcgaccagagagatcagctctggaaggacatcataaactccatcaactccggttatggagtcgtggcaaacattgttgctcctccaagcaactacccgagagcgagctacaagtccacacagtccccagcctatgcaggcggaacagtgtatcactacgttgcggtgatgggttacgccattgacgacagcggaagatctcatgtgtgggtcgcagattccggtttcgcaccctatggctactggatgactctccagcagctatccacgcttatcccaccaaagggatatgcgtactccaccaacattcctcaggaaggacta

SEQ ID NO: 142 - DNA, 1206 bp, Artificial Sequence
atgtcacttgggtctggcaggaaggagagaatacataagatggatgttaacacactaagggaggtgatggggaattaccgaaacgttaactatgacgctatggtaggccccatgaatgaggcgatgatcgctgctggatgcactaacctccggcgagctgctatgtggtgtgctcagatcggccacgagtcagaaggcctcaccgcgatggaagagtacgccagcggagctggctacgaaggaaggcttgatctaggcaatactcagcctggagacggagtgcgctacaagggccgaggccctatccagctcacgggtaggtccaactatcgagcctttactacgtgggctagaagcaagggctatacaactatcgactttgaggcggaaccacacaaggtttccgagcctaagtggggattccttgcagcgtccttctattggacggtgaggaggcctgacattaactctctggccgaccagggagatgtaacgagagtaactcacaggattaacggaggagaaaacggactcagtgaccgtatagcgagatataatcgcgcgatggcactcggggaccgaatccttccttcagcctctgagacaggcacacagacatcgaaaacgacggctgcggagaaggtcctggattataagcgagactgggtgaagcaggacacctactataactgcggtcccgcttcttgtcagacagtaatcggcgcagctacagggaattaccctggagaggttgagctggcagcagctctcaagaccacgattaacggaactgactggatcggagtcttccctggagtcctaaacaggtacattcccggaggaaagtactcctccagggagatacctaacgatccgccaaggagcgaccagagagatcagctctggaaggacatcataaactccatcaactccggttatggagtcgtggcaaacattgttgctcctccaagcaactacccgagagcgagctacaagtccacacagtccccagcctatgcaggcggaacagtgtatcactacgttgcggtgatgggttacgccattgacgacagcggaagatctcatgtgtgggtcgcagattccggtttcgcaccctatggctactggatgactctccagcagctatccacgcttatcccaccaaagggatatgcgtactccaccaacattcctcaggaaggacta

SEQ ID NO: 143 - DNA, 321 bp, Artificial Sequence
attcctcaggaaggactagatatggacgcagtaaagcaaatcatcgactttgttaagggctggacaggcccgatgatccaggacatcaaggacatcagacagcagctgaccggaggcagggatactgtctaccgagaggatggctctgttgaccttgttgccagctacccaggctggaggcagctaggaaccgacaagaacggaaacccgctctctatggtcgatagtatcgcctggagccatgtgaagtcagataagatcatcgagatccttacggctctccaggatcgtatcaccgaactagaaaagaaggttaagtaa

SEQ ID NO: 144 - DNA, 786 bp, Artificial Sequence
atgaccaagattctgaccatcgaaaaggcacgcgagttcgacgctttcgcgcgcgcccgcgacaacctgtactacgggtacggcgaggcattcacccgtaaccctcgccagtcgaccgactgctccgggctcgtcctgcagtcgggtgcgatcctcggtggccgcaccgactgggtgggaaaccgctacggatcgaccgagtcgttccgcctcgactacgcgatcgtgtacgcgctgggattcaagcgcatgcctcgaggtgggttgccgttcgtgccggtgatgaaggtcggtctgcagcacggtggcggcgggatctactcccacaccgcgtgcacgctgatgttcctcgacaagcccggtggcccgatcaaggagtctgcgcggggcgtcgactgggagtcccagggcgccggcgtcttttactacgagggcgcccgtgcctggaatgatggtctgttccacgatttctggtacctcgacatgcgcctcggtgagctcgcgccgccggtgaacgagatcaacgccgagttcgagcgggcgaagggctggatcggcaagcgcatcgacgtcgctgagaagccctgccccgacggcgaaggcaagtacatcaggtgcgagggcggccatatctacttccacccgaaggtcaacgtcggcgcgaagccgggcgagcgtgcgatcgcgatcccggctgacgtcttcgaggtgtggaagcgccagggattcgagaagggaccgctcggctacccgacgcgccgtcacgccacggtcaacggtgtcggc

SEQ ID NO: 145 - DNA, 309 bp, Artificial Sequence
ggattcgagaagggaccgctcggctacccgacgcgccgtcacgccacggtcaacggtgtcggcaccatccaggcatttcagaacggcgcggtctatcgcaagttcggcaccgacggcggcatcgtcaacggcaagatcctcgagcgctgggcgcgcgaaggtcacgagaagggccgcctcggttggcctctcggcgacgagaagttcttcgacggcggtcgcgtccaggcgttcgagaacggtgacgcctacttccaccccaccgcggtggtcgagttcctcaacgatcccgcagcccccaagcagtaa

SEQ ID NO: 146 - DNA, 810 bp, Artificial Sequence
atgcgtccctaccgtgcacgccatctcgccactcctcccacccccgactcgactcccgacacctcatccggtgcgtcgcgccgttccgtcctgcgcgggggtgtcctcggtgccgcggcactgagcaccggcgccgccgccgtcgcgaccccggcggcgaacgccgccggcctctacggacaggacgtctccggctggcagggagagatcgactggtccgcccaggcggacctcggctctcgcttcgcctatgtgaaggccaccgagggtcggtcctaccgcagccccgccttcaaccagcagtaccgcggcgccggcaatgccggcctggtccgcggcggctaccacttcgcccgccccgactccggcggccccgaggagcaggtcgacttcttcctcaacaacggcgggggatggtccgacgacggcatcacgctgccgggcatggtcgacttcgaggcctactccggactgcctcgcgactacgggctgagccagcaggagatgcggaactggatcatggcgttctccactcgctaccgggacagcgtcgggcgtcggcccgtcctctacacgaacctccactggtggaacgacgtggtgggggactggaccccggtcaactccccgctgttcctcgcgtcctacagcagcagcgcgccgaccaccctgccgggccgctggtgggcctacgagatgtggcagtactcggattcgggtcccttcgccggtgactcgaacctctggcacggctccgagtcccagttcgagagcttcgtctccgacggggactaccacgcgatcggcatc

SEQ ID NO: 147 - DNA, 429 bp, Artificial Sequence
atgaggtttattcctgcggcgcatcattctgccggctcgaatagtccggtgaatagggttgtgatccatgcgacatgccctgatgtggggtttccgtctgcctcacgtaaggggcgggcggtgtctacagcaaactattttgcttccccatcgtcggggggttcggcgcattatgtgtgtgatgttggggagacggtgcagtgcctgtcagaggggactattggttggcatgccccgccgaatccgcattctttgggtatagagatttgcgcggatgggggttcgcacgcctcgttccgtgtgccggggcatgcttacacgagggagcagtggcttgatcctcgcgtgtggcctgcggtggagaaggctgccatcctgtgtagacgtttgtgtgacaaatataaatgcttacacgagggagcagtggct

SEQ ID NO: 148 - DNA, 483 bp, Artificial Sequence
atggcaaccatgcctgtcaaaaaaggcttttatgtcacttcggggtttggcccgcgttggggcactacgcattacggcacggattttggtgttgatggtggctcaggtgggcaccctattttcgctatcaaatctggcactgtgaccgcttctggcccggcttctggttttgggcagtggatcaatgtggatcatcctgcaagtgatggcggtggcttgtcggtgtatgggcacatcatcccagaggtgcgcgtaggtgatcaggtggtggaggggcagcggatcggacgaatcaaccccgatcaaaacactaacggcggggttgcgcctcatcttcatttggagtttcaccgctccgtgtggtcaccacctggtggtgatcgcctcgaccccatgaaaactgtgctcgctggtgcagactggccgggtgatgcgccctcaaattcgagcgcgaaaccggaaacggggaaggtcaaaaacatc

SEQ ID NO: 149 - DNA, 714 bp, Artificial Sequence
ggtgcagactggccgggtgatgcgccctcaaattcgagcgcgaaaccggaaacggggaaggtcaaaaacatctttggtgtggatatttccaatcatcaaaatggtattttggctgaattgatcggtgcggaaggttttgaattctgcatcatcaaagccaccgagggtacgtggaaagaccctattttgcattcgcatttggcggatgttcgcaaaaattccggcatgcaggttggcgcatatgtgtatgtgcgtggggaaacctcaccagaagcgcatgctatcgctctacatgagcatctgaatgacacgtcggtgccggttgctttggatattgagcataattccggctctaatcctgatcattggcgggcaattaaaacggcgatcgaggcccgtggctaccgcgtgatcctaacatacttgccggagtggtactggagccaagtcgggcagccaaacttggcggggctaccgccgttgtgggcttcccgttatgtcggcaccacaccaggggttgccagcgtcttatattccacggctggtcggcgtggctggcaaggatacggcggccttgaagttgcgatgtggcagttcaccgaccgggcgcaggtcgcaggccaaaagatcgacgccaatgtttttgagggcacggagaaacagcttcgtgcccttttccatggggacaccccagaaatagaggaggagttcgat

SEQ ID NO: 150 - DNA, 1125 bp, Artificial Sequence
atggcaaccatgcctgtcaaaaaaggcttttatgtcacttcggggtttggcccgcgttggggcactacgcattacggcacggattttggtgttgatggtggctcaggtgggcaccctattttcgctatcaaatctggcactgtgaccgcttctggcccggcttctggttttgggcagtggatcaatgtggatcatcctgcaagtgatggcggtggcttgtcggtgtatgggcacatcatcccagaggtgcgcgtaggtgatcaggtggtggaggggcagcggatcggacgaatcaaccccgatcaaaacactaacggcggggttgcgcctcatcttcatttggagtttcaccgctccgtgtggtcaccacctggtggtgatcgcctcgaccccatgaaaactgtgctcgctggtgcagactggccgggtgatgcgccctcaaattcgagcgcgaaaccggaaacggggaaggtcaaaaacatctttggtgtggatatttccaatcatcaaaatggtattttggctgaattgatcggtgcggaaggttttgaattctgcatcatcaaagccaccgagggtacgtggaaagaccctattttgcattcgcatttggcggatgttcgcaaaaattccggcatgcaggttggcgcatatgtgtatgtgcgtggggaaacctcaccagaagcgcatgctatcgctctacatgagcatctgaatgacacgtcggtgccggttgctttggatattgagcataattccggctctaatcctgatcattggcgggcaattaaaacggcgatcgaggcccgtggctaccgcgtgatcctaacatacttgccggagtggtactggagccaagtcgggcagccaaacttggcggggctaccgccgttgtgggcttcccgttatgtcggcaccacaccaggggttgccagcgtcttatattccacggctggtcggcgtggctggcaaggatacggcggccttgaagttgcgatgtggcagttcaccgaccgggcgcaggtcgcaggccaaaagatcgacgccaatgtttttgagggcacggagaaacagcttcgtgcccttttccatggggacaccccagaaatagaggaggagttcgat

SEQ ID NO: 151 - DNA, 333 bp, Artificial Sequence
catggggacaccccagaaatagaggaggagttcgatatgagcgcagtccaggaaatcaaagactatattgacacccgactgacaggacctgtcggcaccgatgtcaaggacatcaggcagcagatcaccggagggcgcgactctatcccaggtgacctcaaagcgtcttaccctgggtgggatttaggtcagctggtgcgtgcggcacgtgaaaaagaatttactggcctgacgatgatggaaattcttgcagtcaatattgctggtaatgatgatgatttccgtgcagcacgtgttgctgcaggtaccgaggaggctggcaatgctgaataa

SEQ ID NO: 152 - DNA, 555 bp, Artificial Sequence
atggccgactacttctacccactcagccagggcgctcacgtcaccagcccattcgggccccgagctggcggctatcactggggcaccgactacggccgcgccggaggctccggcggcaacgccgtctacgccccgcaagccggaaccgtcatcatggccggccccgccagcggcttcggcggccccgaccccgccggatggatcgtcatcgaccacccaaccgccgccggcggcggagtcagcgtcctcggccacatcatccgtgaagtcgccgtcggcgacaccgtccgcgccgggcagcgcatcgggcgggtcaatccttcctcggccaccaatggcggcgtggcgccgcacgtccacttcgagcatcaccgttacgtctggtccccgccgggaccggaccgtctggacccgcacgcttggctggccacccgcggcgcccgatggccgggagccccggccacacctacccgaaaggaatccatgaacgcgctcaccgctgacatcgacctgctgacccccaacgacgatggccgggcgacgaagccccgcaac

SEQ ID NO: 153 - DNA, 621 bp, Artificial Sequence
atcgacctgctgacccccaacgacgatggccgggcgacgaagccccgcaaccttttgtgcatccataccttcgaagacgacggcacgtggtcggccgacaggatggcgaagtaccagcagtcgcccgccgccggcggctcgtaccacctggtcattgacctcaacggccgcatcgctcgtgagaacgacgacgcgttcatcccatgggcggcgatgttcacgggcaaccgggtggcgttccacttctcgctgtcgggcaaggcgtcctggacgcgccagcagtggctggcccgtccgaagcagatggacgccctggcgaaggtgctggcggcgtactcgaaggccaagggcatcccgctcatccgccgcggaccgcaggacgtgcgagccgggaagtggggcgtgtgcggccacgacgacatttccaaggcattcggtgagtcgacgcactgggacccgggcccgaacttcccgttcgacgtcgtcatcgacaaggccaaggcgatcctcgccgagccgaagccgacgcccgccccgccgtcggatccggcgccccgtccgattcccccgaaggagactctggtgcccaccacgctcgacaccgtcctgccgtcgctcgtc

SEQ ID NO: 154 - DNA, 1125 bp, Artificial Sequence
atggccgactacttctacccactcagccagggcgctcacgtcaccagcccattcgggccccgagctggcggctatcactggggcaccgactacggccgcgccggaggctccggcggcaacgccgtctacgccccgcaagccggaaccgtcatcatggccggccccgccagcggcttcggcggccccgaccccgccggatggatcgtcatcgaccacccaaccgccgccggcggcggagtcagcgtcctcggccacatcatccgtgaagtcgccgtcggcgacaccgtccgcgccgggcagcgcatcgggcgggtcaatccttcctcggccaccaatggcggcgtggcgccgcacgtccacttcgagcatcaccgttacgtctggtccccgccgggaccggaccgtctggacccgcacgcttggctggccacccgcggcgcccgatggccgggagccccggccacacctacccgaaaggaatccatgaacgcgctcaccgctgacatcgacctgctgacccccaacgacgatggccgggcgacgaagccccgcaaccttttgtgcatccataccttcgaagacgacggcacgtggtcggccgacaggatggcgaagtaccagcagtcgcccgccgccggcggctcgtaccacctggtcattgacctcaacggccgcatcgctcgtgagaacgacgacgcgttcatcccatgggcggcgatgttcacgggcaaccgggtggcgttccacttctcgctgtcgggcaaggcgtcctggacgcgccagcagtggctggcccgtccgaagcagatggacgccctggcgaaggtgctggcggcgtactcgaaggccaagggcatcccgctcatccgccgcggaccgcaggacgtgcgagccgggaagtggggcgtgtgcggccacgacgacatttccaaggcattcggtgagtcgacgcactgggacccgggcccgaacttcccgttcgacgtcgtcatcgacaaggccaaggcgatcctcgccgagccgaagccgacgcccgccccgccgtcggatccggcgccccgtccgattcccccgaaggagactctggtgcccaccacgctcgacaccgtcctgccgtcgctcgtc

SEQ ID NO: 155 - DNA, 261 bp, Artificial Sequence
ccgaagccgacgcccgccccgccgtcggatccggcgccccgtccgattcccccgaaggagactctggtgcccaccacgctcgacaccgtcctgccgtcgctcgtcgacggctccacgttcgaggctccgttggccacgttcatccgcaccgcggacaaacaggcctacgaagccaaccagcggatcgcccgcctggaggcgaagttcgatcggctgctcgatgccatgggcgaaaagcccgaccccaagcccggccagtag

SEQ ID NO: 156 - DNA, 585 bp, Artificial Sequence
atgagatacattcctgcggcgcatcactcggccggctctaatagtccggtgaacagggttgtgattcatgcaacatgcccggatgtggggtttccgtccgcttcccgtaaaggacgggcggtgtccacggcaaactatttcgcgtccccatcggcgggcggttctgcccattatgtgtgtgatgttggggagacggtgcagtgcttgtcggagtctacgattggttggcatgccccgccgaatccgcatagtttgggtatagagatttgcgcggatgggggttcgcacgcctcgttccgtgtgccggggcatgcttacactcgtgagcagtggcttgatccgagggtgtggcctgcggtggagaaggcggctgtgctgtgtagacagttgtgtgacaaatataatgttccgaagaggaaactgtctgtatccgatttgaaggctggcaggcggggtgtgtgcggccatacggatgtgacggatgcgtggcatcagtcggatcatgatgatccggggccgtggtttccgtgggacaggtttatggccgtcgtcaacggcggcagtggagagagtggagagttgagt

SEQ ID NO: 157 - DNA, 558 bp, Artificial Sequence
atgagatacattcctgcggcgcatcactcggccggctctaatagtccggtgaacagggttgtgattcatgcaacatgcccggatgtggggtttccgtccgcttcccgtaaaggacgggcggtgtccacggcaaactatttcgcgtccccatcggcgggcggttctgcccattatgtgtgtgatgttggggagacggtgcagtgcttgtcggagtctacgattggttggcatgccccgccgaatccgcatagtttgggtatagagatttgcgcggatgggggttcgcacgcctcgttccgtgtgccggggcatgcttacactcgtgagcagtggcttgatccgagggtgtggcctgcggtggagaaggcggctgtgctgtgtagacagttgtgtgacaaatataatgttccgaagaggaaactgtctgtatccgatttgaaggctggcaggcggggtgtgtgcggccatacggatgtgacggatgcgtggcatcagtcggatcatgatgatccggggccgtggtttccgtgggacaggtttatggccgtcgtcaacggc

SEQ ID NO: 158 - DNA, 300 bp, Artificial Sequence
ggcagtggagagagtggagagttgagtatggctgatgtgaaagccttgcatgatcagattaaacagttgtcggggcaggtggcccagtcggtgaataagctgcatcacgatgtgggtgtggttcaggttcagaatgggaatcttaaaaagcaggttgattccctgtctatggtgaagaatcctgtgacggggaagctgtggcgtaccagggatgcgatctggtcgatctggtattacgtgttggagtgtcgtagccgtatcggcaagttggaggccgaggtggcccggttgaagaagtga

SEQ ID NO: 159 - DNA, 273 bp, Artificial Sequence
atggctgatgtgaaagccttgcatgatcagattaaacagttgtcggggcaggtggcccagtcggtgaataagctgcatcacgatgtgggtgtggttcaggttcagaatgggaatcttaaaaagcaggttgattccctgtctatggtgaagaatcctgtgacggggaagctgtggcgtaccagggatgcgatctggtcgatctggtattacgtgttggagtgtcgtagccgtatcggcaagttggaggccgaggtggcccggttgaagaagtga

SEQ ID NO: 160 - DNA, 492 bp, Artificial Sequence
atgtccacggcaaactattttgcttccccatcgtcgggtggttcggcgcattatgtttgcgatattagtgagacggtgcaatgcctgtcggagtctacgatcgggtggcatgccccgccgaatccgcatagtttgggtatagagatttgcgcggatgggggttcgcacgcctcgtttagggtgccagggcacgcttacactcgtgagcagtggctggatcctagggtgtggcctgccgtggagaaggctgccatcctgtgtagacgtttgtgtgacaaatataatgttccgaagcggaaactgtctgtagccgatttgaaggctggcaggcggggtgtgtgcggccacgtggatgtgacggatgcgtggcatcagtcggatcatgacgatccggggccgtggtttccgtgggacaggtttatggccgtcgtcaacggcggtagtggagatagtggggagttaactgtggctgatgtgaaagccttgcatgat

SEQ ID NO: 161 - DNA, 306 bp, Artificial Sequence
aacggcggtagtggagatagtggggagttaactgtggctgatgtgaaagccttgcatgatcagattaaacaattgtctgctcagcttactggttcggtgaataagctgcaccatgatgttggtgtggtacaggtacagaatggtgatttgggtaaacgtgttgatgccttgtcgtgggtgaagaatccggtgacggggaagctgtggcgcaccaaagacgctttgtggagtgtctggtattacgtgctggagtgtcgcagccgcatagacaggctcgagtctgctgttaacggtttgaaaaagtga

SEQ ID NO: 162 - DNA, 273 bp, Artificial Sequence
gtggctgatgtgaaagccttgcatgatcagattaaacaattgtctgctcagcttactggttcggtgaataagctgcaccatgatgttggtgtggtacaggtacagaatggtgatttgggtaaacgtgttgatgccttgtcgtgggtgaagaatccggtgacggggaagctgtggcgcaccaaagacgctttgtggagtgtctggtattacgtgctggagtgtcgcagccgcatagacaggctcgagtctgctgttaacggtttgaaaaagtga

SEQ ID NO: 163 - DNA, 585 bp, Artificial Sequence
atgacattcatccaggcccgccatcacggcggcaactccaacacgccgatcacccggctggtcatccacgccacctgccccgacgtgggctacccgtcggcgtcgaaggccggtagggcagtctccacggcggagtatttcgcgtccacgtcgcggtctgcctcggctcactacgtctgtgacgtatcggcaacggtgcagtgcctctccgaggaaaccatcggctaccacgcgccgcccaacagtcattccatcggcattgagatttgcgccgacggcgggtcccgcgcctcatttgagaaggcttctcacgcatacacccgcgagcaatggctctcgcctcaagtgtggcccgccgtggagcgcgccgccattctcgcccgcggcatctgccaccgccaccacatcccggttcgcaaactcaccaccgcacaggtcaaatcggggatgtcgggtatttgcggacacgacaacgtatccgatgcattccaccaatccgaccacgacgaccctggcccctacttcccgtggaacgaatttatcgccgccatccaaggaaaaaacaccaacaagggagaactcagc

SEQ ID NO: 164 - DNA, 558 bp, Artificial Sequence
atgacattcatccaggcccgccatcacggcggcaactccaacacgccgatcacccggctggtcatccacgccacctgccccgacgtgggctacccgtcggcgtcgaaggccggtagggcagtctccacggcggagtatttcgcgtccacgtcgcggtctgcctcggctcactacgtctgtgacgtatcggcaacggtgcagtgcctctccgaggaaaccatcggctaccacgcgccgcccaacagtcattccatcggcattgagatttgcgccgacggcgggtcccgcgcctcatttgagaaggcttctcacgcatacacccgcgagcaatggctctcgcctcaagtgtggcccgccgtggagcgcgccgccattctcgcccgcggcatctgccaccgccaccacatcccggttcgcaaactcaccaccgcacaggtcaaatcggggatgtcgggtatttgcggacacgacaacgtatccgatgcattccaccaatccgaccacgacgaccctggcccctacttcccgtggaacgaatttatcgccgccatccaagga

SEQ ID NO: 165 - DNA, 288 bp, Artificial Sequence
aaaaacaccaacaagggagaactcagcatgtccgacgtcaacaccctgaccaagctcatcaaggccagcaacaatcagctccaccacgacattggcgtcgtccagacacagaacggcaccctcaaaagcaagatcgacaacttgtcgtgggtgaagaatcccgtcaccggcaagaagtggtccaccaaggatgcgctgtggtctgtctggtactacgtgctggaatgccgcaaccgcatccaggctatcgaaaaccgcctctctgacatcgaaaagaaggtgaagtga

SEQ ID NO: 166 - DNA, 261 bp, Artificial Sequence
atgtccgacgtcaacaccctgaccaagctcatcaaggccagcaacaatcagctccaccacgacattggcgtcgtccagacacagaacggcaccctcaaaagcaagatcgacaacttgtcgtgggtgaagaatcccgtcaccggcaagaagtggtccaccaaggatgcgctgtggtctgtctggtactacgtgctggaatgccgcaaccgcatccaggctatcgaaaaccgcctctctgacatcgaaaagaaggtgaagtga

SEQ ID NO: 167 - DNA, 273 bp, Artificial Sequence
ggagaactcagcatgtccgacgtcaacaccctgaccaagctcatcaaggccagcaacaatcagctccaccacgacattggcgtcgtccagacacagaacggcaccctcaaaagcaagatcgacaacttgtcgtgggtgaagaatcccgtcaccggcaagaagtggtccaccaaggatgcgctgtggtctgtctggtactacgtgctggaatgccgcaaccgcatccaggctatcgaaaaccgcctctctgacatcgaaaagaaggtgaagtga

SEQ ID NO: 168 - DNA, 591 bp, Artificial Sequence
atgacgttcattcaggccgcgcatcacagcagcggctccaatctgccgcccacgagggtggtgatccacgcgacatgccccgaactcggcttcccgagggccagtgcgaagggccgagctgtctcgacagcccgctacttccagtctgcgatctcgggcggctcggcgcactatgttgtcgatgtcggcgaaaccgtgcagtgtctggcagaggatgtgatcgcctggcacgccccgcccaacagccgcagcctggggatcgagatctgcgctgacggcggctcggcgaccagcttcaagaaccccaacgtgcgctacagccgcgcccagtggctcagcccgcaggtctggcccgccgtgctccgtgccgcagcactcacccggcagatgtgccagaagtacggcataccggtcaccaagctcagcgcgtcggacctcaaggccgggaagaagggcatctgcggacacgtcgatgtcagcaatgcgtggcatcagtccgaccacgacgaccccggcccggacttcccctgggccgaattcatggcagccgtcaaaggcggcgccaccaaccccgatgaactggagctcaca

SEQ ID NO: 169 - DNA, 555 bp, Artificial Sequence
atgacgttcattcaggccgcgcatcacagcagcggctccaatctgccgcccacgagggtggtgatccacgcgacatgccccgaactcggcttcccgagggccagtgcgaagggccgagctgtctcgacagcccgctacttccagtctgcgatctcgggcggctcggcgcactatgttgtcgatgtcggcgaaaccgtgcagtgtctggcagaggatgtgatcgcctggcacgccccgcccaacagccgcagcctggggatcgagatctgcgctgacggcggctcggcgaccagcttcaagaaccccaacgtgcgctacagccgcgcccagtggctcagcccgcaggtctggcccgccgtgctccgtgccgcagcactcacccggcagatgtgccagaagtacggcataccggtcaccaagctcagcgcgtcggacctcaaggccgggaagaagggcatctgcggacacgtcgatgtcagcaatgcgtggcatcagtccgaccacgacgaccccggcccggacttcccctgggccgaattcatggcagccgtcaaa

SEQ ID NO: 170 - DNA, 573 bp, Artificial Sequence
atgacgttcattcaggccgcgcatcacagcagcggctccaatctgccgcccacgagggtggtgatccacgcgacatgccccgaactcggcttcccgagggccagtgcgaagggccgagctgtctcgacagcccgctacttccagtctgcgatctcgggcggctcggcgcactatgttgtcgatgtcggcgaaaccgtgcagtgtctggcagaggatgtgatcgcctggcacgccccgcccaacagccgcagcctggggatcgagatctgcgctgacggcggctcggcgaccagcttcaagaaccccaacgtgcgctacagccgcgcccagtggctcagcccgcaggtctggcccgccgtgctccgtgccgcagcactcacccggcagatgtgccagaagtacggcataccggtcaccaagctcagcgcgtcggacctcaaggccgggaagaagggcatctgcggacacgtcgatgtcagcaatgcgtggcatcagtccgaccacgacgaccccggcccggacttcccctgggccgaattcatggcagccgtcaaaggcggcgccaccaacccc

SEQ ID NO: 171 - DNA, 255 bp, Artificial Sequence
ggcggcgccaccaaccccgatgaactggagctcacagtgtctcaattcagtgacctgaccaagcgcctgcagggcatgcaggagcagacccaccacgacctcggcgtcgtccagaccaagctggccaccatggacaccgtcaagaacccccgcaccggcgccaagtggagcctcaaggacgccatctggtcgatctggtactacgtgctggagaacagggaccggatcgccgccctcgagaagaaggtgaagtga

SEQ ID NO: 172 - DNA, 216 bp, Artificial Sequence
gtgtctcaattcagtgacctgaccaagcgcctgcagggcatgcaggagcagacccaccacgacctcggcgtcgtccagaccaagctggccaccatggacaccgtcaagaacccccgcaccggcgccaagtggagcctcaaggacgccatctggtcgatctggtactacgtgctggagaacagggaccggatcgccgccctcgagaagaaggtgaag

SEQ ID NO: 173 - DNA, 237 bp, Artificial Sequence
gatgaactggagctcacagtgtctcaattcagtgacctgaccaagcgcctgcagggcatgcaggagcagacccaccacgacctcggcgtcgtccagaccaagctggccaccatggacaccgtcaagaacccccgcaccggcgccaagtggagcctcaaggacgccatctggtcgatctggtactacgtgctggagaacagggaccggatcgccgccctcgagaagaaggtgaagtga

SEQ ID NO: 174 - DNA, 645 bp, Artificial Sequence
atggactggaccaatctgaacgctgacgtgacgaagctgatgaacgtgcacttcacccccgggcgtgaaggccacacgatcgacaagatcgtgattcaccacaacggcggcaacctgagcatcgaccagatctggaatgtgtggcaggaccgtgaagcatcggcccactatcaggtgcaatctgatggccgtatcggccagctcgtcaacgactgggacaccgcctggcacgccggcgactgggacgccaacctgacctcgatcggcatcgagcacgccgacgactcgaccgacccgtggcatgtgtcggatgccgccgtcgatgccggcgcgcacctggtggctgcactgtgtcgcggctacaaccttggccggccggagtggatgcgcaacgtcttcccgcactcgcatttctcggcgacctcgtgcccggcctcgcttgccgagaatcagcgcgcggattacatggcgcgcgctcaggcctatttcgatggcgctcccgtcacaggccgttcttcggtccctgcaccggctccggcgcctgccgggatccatgtggacctgcctgcctggactctccccgcaggcaacttttacgggtcgatcgatggcggcgaggactcgcatggcggctactacgagggt

SEQ ID NO: 175 - DNA, 423 bp, Artificial Sequence
gcctcgcttgccgagaatcagcgcgcggattacatggcgcgcgctcaggcctatttcgatggcgctcccgtcacaggccgttcttcggtccctgcaccggctccggcgcctgccgggatccatgtggacctgcctgcctggactctccccgcaggcaacttttacgggtcgatcgatggcggcgaggactcgcatggcggctactacgagggtgagcgtcctgcaatcgcagcgattcagcgctggcttatccgccacggctacgcgggtgcagtggacgactcatgggccgatggtctgtacgagcagcccaccgtcgacgccgtgacccgcttccagcgtgccgagcgaccaaactccacggaccggtggggcgaggtctgggccgacgatctggccaccatggccgccaacaacggctga

SEQ ID NO: 176 - DNA, 588 bp, Artificial Sequence
atggatcgtggtattgacgtgtcgtcctatcaggcccccgatggtggcctgctggagggcatgtcgttttgcatcatcaaggccaccgaaggcaccggctatgtgaacccgaaccgtacccagtggtacaaggtcgccacggatcgtggggtgaccaccggcgcctatcacttcatgcgtggcggcgatcccgtggcgcaggccgattacttcctcgcgcatctgcccggtgatgtcgattggctcgcccttgatgtcgaggatcccagcgacggcctgtcatgggccgggcgcgtcagcttcatcctcgcctggaccgatcgggtgaaggcgaccggcaagcccaccttggtctattgctcgcgctcctgggcgaatgccctgttgggtgcggccagcagcgacgagcgggcacggctcgcgcaattgccgctgtggatggctgattacacccaacgccccggcgaatattcggggccgtggccgggcggctggccgattgccatacaccagtacacctcggccccgatcgacaagaacgtcctgctcaccgacgatctccaaggaggagacgacatgcccctgtca

SEQ ID NO: 177 - DNA, 351 bp, Artificial Sequence
ctcaccgacgatctccaaggaggagacgacatgcccctgtcaaccgacgaccttcgaaatatcgccactgccgtgtggggtggcggcggcgctgcaagcccaatgtatgccgaccggctcgatgggcatcaagaatatccggagacagcccttttcagcctgcaacagcggctgggtgcccgcttcggtgagctgtcgggcaagatcgacggtctggccgaggcgctcaagcaggtgcagggagggaacggcgtggacgcggacgccattagggctgctgctgccgaaggagccaaggctggcgtgcaggcgatgatcgacaccgccacggtgaatctggaggccaagtga

SEQ ID NO: 178 - DNA, 687 bp, Artificial Sequence
atgtgcggggctttctcattcctcaaagacttggagacattcatggactggaccaatctgaacgctgacgtgacgaagctgatgggcgtgcacttcacccccggacgtgaaggcaggacgatcgacaagatcgtgatccaccacaacggcggcaacctgagcatcgaccagatctggaatgtgtggcagacccgtgaagcctccgcgcattatcaggtggaggcgggtggccgtatcggccagctcgtcaacgatttggacaccgcgtggcatgccggcgactgggacgccaacctgacctcgatcggcatcgagcatgccgacgactcgaccgacccgtggcatgtgtctgatgctgccgtcgatgccggcgcgcacctggtggctgcactgtgtcgcggctacaaccttggccggccggagtggatgcgcaacgtcttcccgcactctcagttcacgtccacgtcgtgcccggcgtcgctggcccgggaccagctcggcgactacatggggcgcgcacaagcctacttcgatggcgcgccggtggctgcggtccatcagtcggtccctgcccccgccccagcgcccagccgtcatgtggacctgcccgcgtggaatctccccgagggcaacttctacggcctcgtcagcggcggaaacgactcccacggcggcttctatcccgcc

SEQ ID NO: 179 - DNA, 420 bp, Artificial Sequence
gcgtcgctggcccgggaccagctcggcgactacatggggcgcgcacaagcctacttcgatggcgcgccggtggctgcggtccatcagtcggtccctgcccccgccccagcgcccagccgtcatgtggacctgcccgcgtggaatctccccgagggcaacttctacggcctcgtcagcggcggaaacgactcccacggcggcttctatcccgccgagcgtcccgctgtgagggccatccagctgtggctcatccgtcacggctacgccggcgcggtgcctgacagttgggcggacggcatctacgagcagccgaccgccgacgccgtgaccgctttccagcacgccgagcgccccaacagcacggaccggtggggcgaggtctgggccgacgacctggccaccatggccgccaacaactga

SEQ ID NO: 180 - DNA, 696 bp, Artificial Sequence
atgaaggcgtctcgcgtgatcgtcgtagcaagtgtcgtagcactgatccttgcgggcctggcaatgtcgtcagctgccgtgattgtggtgccactactgtcagtaggcgccggggccctcgacgacaactctggcgctggcggcgtcggtggggatccctgcataggaactgtcaccggtggcgctgttagtgtcggaggcctcacaaccaggcagaagcaactagtgaccaccatcgtcaccgtggtccaacgcgacaaactacctgtccaggctgcggtcatcgccatcatgaccgctaaacaggaatcagacctcggagccaaccccgccgcaacgaaacctaacggtgacggcgacgccggcccattccaacagcgcgttctaccgggctggtacggcaccttggaccaagtcaacaatgatgcctacgccacggagacattcctgaaaggccacaccatcacctatgctggccccacatcggccggcggccccggctaccacattcccggccttgtcgatgtccccgactggcagtcgaaatccccggcccaagcagcccaagcggttcaggcctcagccctgcctaacgcttacgctaaatgggaggccatcgccaaacagatggtgggagccaccaccacagggcgcctgtccaacgactgtgtcaccgggaccgctaacgaaaccggc

SEQ ID NO: 181 - DNA, 450 bp, Artificial Sequence
gccatcgccaaacagatggtgggagccaccaccacagggcgcctgtccaacgactgtgtcaccgggaccgctaacgaaaccggcgtctcaaagaacctgaccaaagccgtggaatgggccaaatcgatcgccgccaacaactcctacacctacgtgtggggcggtaatggtgcgagcgatggcggctacgactgctcaggcctgacctcggcactgtaccgacgtatcggcatcaaccttccccgcaccgctgccgaacagcaaaaagtcggcaccccagtcaaccgcaaccagctcaaagtcggcgaccttatcttctggggcatccctgcccaccacgtagccacctacatcggtagaggccagatgatcagcgccgacaaccaagcccgcggcatcaacgtggagaagatctacggcaacccctcgagctaccgaaggatcgtcaaa

SEQ ID NO: 182 - DNA, 1062 bp, Artificial Sequence
atgaaggcgtctcgcgtgatcgtcgtagcaagtgtcgtagcactgatccttgcgggcctggcaatgtcgtcagctgccgtgattgtggtgccactactgtcagtaggcgccggggccctcgacgacaactctggcgctggcggcgtcggtggggatccctgcataggaactgtcaccggtggcgctgttagtgtcggaggcctcacaaccaggcagaagcaactagtgaccaccatcgtcaccgtggtccaacgcgacaaactacctgtccaggctgcggtcatcgccatcatgaccgctaaacaggaatcagacctcggagccaaccccgccgcaacgaaacctaacggtgacggcgacgccggcccattccaacagcgcgttctaccgggctggtacggcaccttggaccaagtcaacaatgatgcctacgccacggagacattcctgaaaggccacaccatcacctatgctggccccacatcggccggcggccccggctaccacattcccggccttgtcgatgtccccgactggcagtcgaaatccccggcccaagcagcccaagcggttcaggcctcagccctgcctaacgcttacgctaaatgggaggccatcgccaaacagatggtgggagccaccaccacagggcgcctgtccaacgactgtgtcaccgggaccgctaacgaaaccggcgtctcaaagaacctgaccaaagccgtggaatgggccaaatcgatcgccgccaacaactcctacacctacgtgtggggcggtaatggtgcgagcgatggcggctacgactgctcaggcctgacctcggcactgtaccgacgtatcggcatcaaccttccccgcaccgctgccgaacagcaaaaagtcggcaccccagtcaaccgcaaccagctcaaagtcggcgaccttatcttctggggcatccctgcccaccacgtagccacctacatcggtagaggccagatgatcagcgccgacaaccaagcccgcggcatcaacgtggagaagatctacggcaacccctcgagctaccgaaggatcgtcaaa

SEQ ID NO: 183 - DNA, 567 bp, Artificial Sequence
atggactggaccaatctgaacgctgacgtgaccaagctgatgaacgtgcacttcacccccggacgtgaaggcaggacgatcgacaagatcgtgatccaccacaacggcggcaacctgtcgatcgaccagatctggaatgtgtggcaggaccgtgaagccagcgcgcactaccaggtggaatcgagcggccgcatcggccagctcgtcaacgactgggacaccgcctggcatgccggcgactgggacgcgaatctcacgtcgatcggcatcgagcatgctgacgactcgacggatccgtggcatgtgtcggatgccgccatcgacagcggcgcccatctggtggcggccctgtgccgcgcctacaatcttggtcggccggagtggatgcacaacgtgttcccgcactcgcatttctcggcgacctcgtgcccggcctcgctggccgagaatcagcgcgcggattacatgtcacgggctcaggcctactacgacggcacttcagtggctgccgcacctgctgccccgtcggcacctgccgggatccacgtcgatcttccgagctggacc

SEQ ID NO: 184 - DNA, 372 bp, Artificial Sequence
cgggctcaggcctactacgacggcacttcagtggctgccgcacctgctgccccgtcggcacctgccgggatccacgtcgatcttccgagctggaccctcccgatcgggcattattacgggctggtcacagggccgaatgactcgcatggtggcttctacgagtccgagcgtcccgctgtgagggccatccagctgtggctcatccgccacggctacgccggcgcggtgcctgacagttgggcggacggcatctacgagcagccgaccgccgacgccgtgaccgctttccagcatgctgagcgacccaacagcacggaccggtggggcgaggtctgggccgacgatctggccaccatggccgccaacaactga

SEQ ID NO: 185 - DNA, 612 bp, Artificial Sequence
atggactggaccaacctcatcgccgacaccacgaagctcatgggcgtgcacttcacccccgggcgtgaaggccgcaagatcgacaagatcgtgatccaccacaacggcggcaacctgagcatcgaccagatctggaatgtgtggcagacccgcgaagccagcgcgcactaccaggttgagacgggtggccgcatcggccagctcgtcaacgactgggacaccgcctggcacgccggcgactgggatgcgaatctcacgtcgatcggcatcgagcacgccgacgactccacggacccgtggcatgtgtcggatgccgccgttgacgccggcgcgcaccttgtcgcggccctgtgcaaggcctacagtcttggtcgtcctgagtggatgcgcaacgtcttcccgcactcgcatttctcggcgacctcgtgcccggcctcgctggccgagaatcagcgcgcggattacatgtcacgggctcaggcctactacgacggcgcgccggtggctgcggtccatcagtcggcacctgcccccgccccagcgtccagccgtcacgtggacctgcccgcgtggaatctccccgagggcaacttctacggcctggcgagcggt

SEQ ID NO: 186 - DNA, 381 bp, Artificial Sequence
cgggctcaggcctactacgacggcgcgccggtggctgcggtccatcagtcggcacctgcccccgccccagcgtccagccgtcacgtggacctgcccgcgtggaatctccccgagggcaacttctacggcctggcgagcggtggcgaggattcgcacggcggcttctacgagggtgagcgtcccgcgatccgccagatccagctgtggctcatccgtcacggctatgccggcgcggtgcctgacagttgggcggacgggatctacgaacaacccactgccgacgccgtggccgctttccagcatgctgagcgtcccaactccacggaccggtggggcgaggtctgggcagacgatctggccaccatggccgccaacaactga

SEQ ID NO: 187 - DNA, 435 bp, Artificial Sequence
gcattcgcagtcgacatcctgcaggcatcagactctccccgcgaaagcgcccccggctggcaatggagacaggccgagccccaggagttcccaagcttcggggagcctgtcctggcagcgggctgcggcaccgtgatcgctgcccatgacggcaagcgtgaccatcgcgcccggaacacctggcccggcctgatctacatgatgtcgctcgaggccttcggtcgagagttggccgggcaccgctccatcatcggcaatcacgtgatcctcgaccatagcgacggcacgttcagcatgtacgcccacctcaagcacggatctgcagccgtgtgcgtcgggcagaaagtccgggccggcgatgtcctgggagcggtcgggaacaccgggaataccagcgaaccccatctccacttccagctgatggaccggccccaa

SEQ ID NO: 188 - DNA, 870 bp, Artificial Sequence
atgatgcgcatgctcaaggcggcttccccctggctccttcgagcctgcgtcctgctcgtggcgctgagcttcgtcatcgaggtccccgtgtggctcgtgttcgcgccgctgggcctggcgatcgcagtcccttctccacgtgcagacgacgagtctccccagaccatgcatgctcccgtgacgggccgctgggtcgccatcaacagcccggcgacgaaggtccccagccacggcgttcgcacgctcggtcaggcattcgcagtcgacatcctgcaggcatcagactctccccgcgaaagcgcccccggctggcaatggagacaggccgagccccaggagttcccaagcttcggggagcctgtcctggcagcgggctgcggcaccgtgatcgctgcccatgacggcaagcgtgaccatcgcgcccggaacacctggcccggcctgatctacatgatgtcgctcgaggccttcggtcgagagttggccgggcaccgctccatcatcggcaatcacgtgatcctcgaccatagcgacggcacgttcagcatgtacgcccacctcaagcacggatctgcagccgtgtgcgtcgggcagaaagtccgggccggcgatgtcctgggagcggtcgggaacaccgggaataccagcgaaccccatctccacttccagctgatggaccggccccaagcggccatggccgccggcctgccgttccggtggtccccgctcacgatcgagccggatcccgatccccactgggctccgaagaaacctgtcgcagagacggtcgagggcctgcccgcgacagggcagatcttccgcaccccggagtccggcgtcatgccccaacccaagcgcgaggccagttgt

SEQ ID NO: 189 - DNA, 279 bp, Artificial Sequence
ggtagtaggggagtggaatttgcggcctccgtgggagaaccagtgacgaccgtgacggctggggtggtcgtttttgctggccaggtcgcgggggctggggtggtgagcatcctgcttgctgacggtcgtcggacaacccacatgccggttgtgcctagcgttgctgtcggccaggtagtggttcctggccagcagatcggagttgtcgggatggggccaccatgcacccgcacttgtttgcactgggggttgaagaagggagatgtttatcaaaacccc

SEQ ID NO: 190 - DNA, 756 bp, Artificial Sequence
atgaggagatctgtctgcatcagcctactaatcatcacggtggggatttgcttgctggccttcccagctcccagccacagcattgctgccgttcccgcgcgaagtgtggcgaatcgtccgactccgccggtgctaggccccgtcatcaaagggtttgcgccacctgccgaaaaatggctgccgggtagtaggggagtggaatttgcggcctccgtgggagaaccagtgacgaccgtgacggctggggtggtcgtttttgctggccaggtcgcgggggctggggtggtgagcatcctgcttgctgacggtcgtcggacaacccacatgccggttgtgcctagcgttgctgtcggccaggtagtggttcctggccagcagatcggagttgtcgggatggggccaccatgcacccgcacttgtttgcactgggggttgaagaagggagatgtttatcaaaaccccatgacattgttgcaacttcaggtgcggttgctgcccttggacagtcggcctcattcagcgtcggggcacggatggcctgtgcggcccctgagcctgccagggggcagcaggaggaaagctgcctcaagcggtgccctcatgcctccgtggcgtggagctgggcgggacgccgcgttaggcattgatacgacggtgaccgaagccacccgaggtggctcaggcgcggggatgagcctggcgaaacgcagtgcgcaatctttcggtggaaacgtgggtgtagatctgcgtggtggc

SEQ ID NO: 191 - DNA, 513 bp, Artificial Sequence
atggcaaagacactctctcgaattgcttccgttgcggctgcggctgccctcgccggtggcgtctccgtgactgcggcgcagagcgcgtcggcagacgatgtcaactgggacgccatcgcaaactgcgagtccggcggtaactggagcacaaacaccggcaatggctactacggtggccttcagttctcccagagcacttgggccgcctacggtggctccggtagcgcctccaatgcctcccgtgaggagcagatcgccgtggccgagcgcgtgctcgcgggccagggcatcggtgcgtggccggtctgcggcgcgtacgcctactccggtgaaagctacaccggcaccaacaccgagggttcctacggctcttcgtacgacacgtcggcccaggacgcctcctacgacggctcgtactcgtatgacaactcgtactcgtacgacaacagcgccgggtacgactcgtcctccgcctactccggcggctaccaggccactcgtgaggccactggc

SEQ ID NO: 192 - DNA, 342 bp, Artificial Sequence
ggcgcgtacgcctactccggtgaaagctacaccggcaccaacaccgagggttcctacggctcttcgtacgacacgtcggcccaggacgcctcctacgacggctcgtactcgtatgacaactcgtactcgtacgacaacagcgccgggtacgactcgtcctccgcctactccggcggctaccaggccactcgtgaggccactggcacctacgagatccagccgggcgacaccctcaacgccatcgctgaggcccatggcaccacctggcaggagctcgcggccctcaacagctccatcgtcgacgcgaacctgatctacgccggcgaaaccatcaacgtctga

SEQ ID NO: 193 - DNA, 528 bp, Artificial Sequence
atggcctatccctatatcggggcattgaagcatggcggcaagcagggcaagatccagcggatcgtcatccatgccacggtttcgccctgtgtgcggggcggtgcccggaacgtcgcgaagtactttcagagttcagccgccggaggcagcgcccactacgtggtggatcccggtgagatcatccagtgtgtcaaggacgacgtggtggcctaccacgcgccgcccaacaccggaacgctcgggatcgagctgtgcgacccgcaggccggatcgccgaagcggtggagcaacgaggcccaccaggcgatgctcgtgctcgccgcgaagctcgtcagggaactcgcggcgaagcacgacgtgccgctcgtccgggtgaccgccgcgcagctcagggcgggcaagcgcggcatctgctcgcatgtcgcggtcagcgacgcgttcgggcagtccgaccacggcgatcccgaggtcgccgggccgttcccctgggcgaagttcatgcagctcatcaaggaggaggacgacatg

SEQ ID NO: 194 - DNA, 372 bp, Artificial Sequence
atggcctatccctatatcggggcattgaagcatggcggcaagcagggcaagatccagcggatcgtcatccatgccacggtttcgccctgtgtgcggggcggtgcccggaacgtcgcgaagtactttcagagttcagccgccggaggcagcgcccactacgtggtggatcccggtgagatcatccagtgtgtcaaggacgacgtggtggcctaccacgcgccgcccaacaccggaacgctcgggatcgagctgtgcgacccgcaggccggatcgccgaagcggtggagcaacgaggcccaccaggcgatgctcgtgctcgccgcgaagctcgtcagggaactcgcggcgaagcacgacgtgccgctcgtccgg

SEQ ID NO: 195 - DNA, 381 bp, Artificial Sequence
gtgaccgccgcgcagctcagggcgggcaagcgcggcatctgctcgcatgtcgcggtcagcgacgcgttcgggcagtccgaccacggcgatcccgaggtcgccgggccgttcccctgggcgaagttcatgcagctcatcaaggaggaggacgacatgccgtcgcccaaggagatctacgaagccgtctgggagcaggacgtcatggcggcccccgacggttccaagtcgaacccgacctggaagcccagcagcgtcctcaccgacgtcgacaagaaggtccgcgccctgcagagccaggtcaccggcctcgagagcgagctggccgccaccaacgccaagctcgaccaggttctcaccctgctccgcgcctcggtgtcctga

SEQ ID NO: 196 - DNA, 579 bp, Artificial Sequence
atgacattcatccaggccgcccaccgtggcggcacttccaacacgccgatcacccggctggtcatccacgccacctgccccgatgtcggcttcccgtcggcatcgcgggcaggacgagcagtatccacagcggaatatttcgcgtccacgtcgaggtcagcctcggcgcactacgtatgcgacatctctaccacggtgcagtgcctgtccgaggcaacgatcggctatcacgcgccaccaaacgcccactccatcggcattgaaatctgcgccgacggaggctcgcgcgcttcatttgagaaggcttctcacgcatacacccgcgagcaatggctcagcccgcaggtatggcccgccgtggagcgcgccgcgattctcgcccgcgacatctgccaccgacaccacatccccatccgccgcctctccgtcgcgcaggtgcgggcaggtgagcgcggaatctgcggccacaacgaggtgagcgaggcgttccaccaatccgaccacgacgaccccggcccctatttcccttggaatgaatttattgccgccgtccaaggaaaaaccaccacaccagaggga

SEQ ID NO: 197 - DNA, 519 bp, Artificial Sequence
atgacattcatccaggccgcccaccgtggcggcacttccaacacgccgatcacccggctggtcatccacgccacctgccccgatgtcggcttcccgtcggcatcgcgggcaggacgagcagtatccacagcggaatatttcgcgtccacgtcgaggtcagcctcggcgcactacgtatgcgacatctctaccacggtgcagtgcctgtccgaggcaacgatcggctatcacgcgccaccaaacgcccactccatcggcattgaaatctgcgccgacggaggctcgcgcgcttcatttgagaaggcttctcacgcatacacccgcgagcaatggctcagcccgcaggtatggcccgccgtggagcgcgccgcgattctcgcccgcgacatctgccaccgacaccacatccccatccgccgcctctccgtcgcgcaggtgcgggcaggtgagcgcggaatctgcggccacaacgaggtgagcgaggcgttccaccaatccgaccacgacgaccccggcccc

SEQ ID NO: 198 - DNA, 330 bp, Artificial Sequence
tatttcccttggaatgaatttattgccgccgtccaaggaaaaaccaccacaccagagggagaactcagcatgtcagacgtaaacaccctgaccaagctcatcaaggccagcaacgaccagcttcactacgatattggcgtcgtccagacgcaaaacgggaacatcaagaagaagatcgacaatctgtcgtgggtgaagaaccccgtcaccggcaagaagtggtccactaaggatgccctgtggtccgtctggtattacgtgctggaatgccgcaaccgcatccaggctatcgagaaccgtatttacgaccttgagaagaaggtgaagtga

SEQ ID NO: 199 - DNA, 273 bp, Artificial Sequence
ggagaactcagcatgtcagacgtaaacaccctgaccaagctcatcaaggccagcaacgaccagcttcactacgatattggcgtcgtccagacgcaaaacgggaacatcaagaagaagatcgacaatctgtcgtgggtgaagaaccccgtcaccggcaagaagtggtccactaaggatgccctgtggtccgtctggtattacgtgctggaatgccgcaaccgcatccaggctatcgagaaccgtatttacgaccttgagaagaaggtgaagtga

SEQ ID NO: 200 - DNA, 639 bp, Artificial Sequence
atgagatacattcctgcggcgcatcattctgccggatcaaataagccggtgaaccgggttgtgattcatgcaacatgcccggatgtggggtttccgtctgcttcgcgtaagggtcgggcggtgtctacagcaaactattttgcttccccatcgtctggtggttcggcgcattatgtgtgtgatattggggagacggtgcagtgcttgtcggagtctacgattggttggcatgccccgccgaatccgcatagtttgggtatagagatttgcgcggatgggggttcgcacgcctcattccgtgttccagggcatgcctatacgcgggagcagtggcttgaccctcgggtgtggcccgcggtggagagggccgccatcctgtgtcggcagttgtgtgataagcatggtgttccgaagaggaaactgtctgtggctgatttgaaggccggtaaacggggtgtttgcgggcatgtggatgttacggatgcgtggcatcagtcggatcatgacgatccggggccgtggtttccgtgggacaaatttatggctgtggtgaatggccacggcggcggttcaagtagtgaggagttgagtatggctgatgtacaagcgttacataatcagattaaacagttgtcggca

SEQ ID NO: 201 - DNA, 519 bp, Artificial Sequence
atgagatacattcctgcggcgcatcattctgccggatcaaataagccggtgaaccgggttgtgattcatgcaacatgcccggatgtggggtttccgtctgcttcgcgtaagggtcgggcggtgtctacagcaaactattttgcttccccatcgtctggtggttcggcgcattatgtgtgtgatattggggagacggtgcagtgcttgtcggagtctacgattggttggcatgccccgccgaatccgcatagtttgggtatagagatttgcgcggatgggggttcgcacgcctcattccgtgttccagggcatgcctatacgcgggagcagtggcttgaccctcgggtgtggcccgcggtggagagggccgccatcctgtgtcggcagttgtgtgataagcatggtgttccgaagaggaaactgtctgtggctgatttgaaggccggtaaacggggtgtttgcgggcatgtggatgttacggatgcgtggcatcagtcggatcatgacgatccggggccg

SEQ ID NO: 202 - DNA, 345 bp, Artificial Sequence
tggtttccgtgggacaaatttatggctgtggtgaatggccacggcggcggttcaagtagtgaggagttgagtatggctgatgtacaagcgttacataatcagattaaacagttgtcggcacaggtggcccagtcggtgaataagctgcatcacgatgttggtgtggttcaggttcagaatggtgatttgggtaaacgtgttgatgccttgtcgtgggtgaagaatccggtgacggggaagctgtggcgcagcaaggatgctttgtggagtgtctggtattacgtgttggagtgtcgtagccgtcttgacaggctcgagtctgctgtcaacgatttgaaaaagtga

SEQ ID NO: 203 - DNA, 225 bp, Artificial Sequence
caggtggcccagtcggtgaataagctgcatcacgatgttggtgtggttcaggttcagaatggtgatttgggtaaacgtgttgatgccttgtcgtgggtgaagaatccggtgacggggaagctgtggcgcagcaaggatgctttgtggagtgtctggtattacgtgttggagtgtcgtagccgtcttgacaggctcgagtctgctgtcaacgatttgaaaaagtga

SEQ ID NO: 204 - DNA, 588 bp, Artificial Sequence
atgacattcatccaggcccgccaccacggcggcaactccaacgcgccgatcacccggctggtcatccacgccacctgccccgacgtgggctacccgtcggcatcgaaggccggtagggcagtctcgaccgcgaactacttcgccacgactgatcggcccgcctcggcacattacgtatgtgacatcgccactacagtgcagtgcctctccgaggaaaccatcggctaccacgcgccgccgaactcgcattccatcggcattgaaatttgcgccgatggcgggtcgcacgcctcatttgagaaggcttctcacgcatacacccgcgaccaatggttgagcgatgacgtgtggcccgccgtagagcgcgccgccattcttgcccgcgatatttgccaacgacaccgcatcccggttcgtaaactctccaccgcacaggtgaaagccggactgtcgggaatttgcggacacgacaatgtatccggcgcattccatcagtccgaccacgacgacccgggcccctacttcccgtgggaccagttcatggcactcgtccaaggaaaacccgccacaccaggagatctcaccatg

SEQ ID NO: 205 - DNA, 519 bp, Artificial Sequence
atgacattcatccaggcccgccaccacggcggcaactccaacgcgccgatcacccggctggtcatccacgccacctgccccgacgtgggctacccgtcggcatcgaaggccggtagggcagtctcgaccgcgaactacttcgccacgactgatcggcccgcctcggcacattacgtatgtgacatcgccactacagtgcagtgcctctccgaggaaaccatcggctaccacgcgccgccgaactcgcattccatcggcattgaaatttgcgccgatggcgggtcgcacgcctcatttgagaaggcttctcacgcatacacccgcgaccaatggttgagcgatgacgtgtggcccgccgtagagcgcgccgccattcttgcccgcgatatttgccaacgacaccgcatcccggttcgtaaactctccaccgcacaggtgaaagccggactgtcgggaatttgcggacacgacaatgtatccggcgcattccatcagtccgaccacgacgacccgggcccc

SEQ ID NO: 206 - DNA, 327 bp, Artificial Sequence
tacttcccgtgggaccagttcatggcactcgtccaaggaaaacccgccacaccaggagatctcaccatggcagacatcagcaaactcaccgacgcgatcaaggcatccaaccggcagctgcaccacgacatcggcgtagtacagacccaaaacggaaaattacgtgagcagatcgaaaggatcacctgggtcaaaaatccggtgacaggaaagaagtggcgcatcaccgacgcgctgtggtcgatctggcactacgtgctggaatgccgcacccgcatccagcggctcgacgcccgtctgtctgaggtcgagaagaaggtgaagtga

SEQ ID NO: 207 - DNA, 261 bp, Artificial Sequence
atggcagacatcagcaaactcaccgacgcgatcaaggcatccaaccggcagctgcaccacgacatcggcgtagtacagacccaaaacggaaaattacgtgagcagatcgaaaggatcacctgggtcaaaaatccggtgacaggaaagaagtggcgcatcaccgacgcgctgtggtcgatctggcactacgtgctggaatgccgcacccgcatccagcggctcgacgcccgtctgtctgaggtcgagaagaaggtgaagtga

SEQ ID NO: 208 - DNA, 579 bp, Artificial Sequence
atgacattcatccaggccgcccaccgtggcggcacttccaacacgccgatcacccggctggtcatccacgccacctgccccgatgtcggcttcccgtcggcatcgcgggcaggacgagcagtatccacagcggaatatttcgcgtccacgtcgaggtcagcctcggcgcactacgtatgcgacatctctaccacggtgcagtgcctgtccgaggcaacgatcggctatcacgcgccaccaaacgcccactccatcggcattgaaatctgcgccgccggaggctcgcgcgcttcatttgagaaggcttctcacgcatacacccgcgagcaatggctcagcccgcaggtatggcccgccgtggagcgcgccgcgattctcgcccgcgacatctgccaccgacaccacatccccatccgccgcctctccgtcgcgcaggtgcgggcaggtgagcgcggaatctgcggccacaacgaggtgagcgaggcgttccaccaatccgaccacgacgaccccggcccctatttcccgtggaatgaatttattgccgccgtccaaggaaaaaccaccacaccagaggga

SEQ ID NO: 209 - DNA, 330 bp, Artificial Sequence
tatttcccgtggaatgaatttattgccgccgtccaaggaaaaaccaccacaccagagggagaactcagcatgtcagacgtaaacaccctgaccaagctcatcaaggccagcaacgaccagcttcactacgacattggcgtcgtccagacgcaaaacgggaacatcaagaagaagatcgacaatctgtcgtgggtgaagaaccccgtcaccggcaagaagtggtccactaaggatgccctgtggtccgtctggtattacgtgctggaatgccgcaaccgcatccaggctatcgagaaccgtatttacgaccttgagaagaaggtgaagtga

SEQ ID NO: 210 - DNA, 600 bp, Artificial Sequence
atgacattcattcaggccaagcatcacggcggccacaacaaccctcccgtgactcgtcttgtcattcacgccacatgcccggatgtgggctatccgtctgcgtcgcgcgctggccgtgcggtgtcgacggcccactattttcaggaaacgacccggccagcatccgcccactacatttgtgacatatcgaccacggtgcagtgtctgtctgaggagacggtgggctatcacgccccgccgaactcacactccatcggtattgagatatgcgctgacggtgggtcgcatgcctcgttttcgaaccctgcccacgcctacacccgcgagcagtggttgagccctcaggtgtggcctgctgtggagcgtgccgcgatgctggcgcgcggtatctgtcaacgccacaacatcccgatccgccgcctctcgatcgctgacgtcaaggccgggaagcgcggcatctgcggccacaacgaggtgtccgaggccttccaccaatccgaccatgacgaccccggtccttatttcccgtgggacgggtttatcgcgcttgttaatggccattccgcaccatcacgccaggaggaactaactgtgtcagat

SEQ ID NO: 211 - DNA, 519 bp, Artificial Sequence
atgacattcattcaggccaagcatcacggcggccacaacaaccctcccgtgactcgtcttgtcattcacgccacatgcccggatgtgggctatccgtctgcgtcgcgcgctggccgtgcggtgtcgacggcccactattttcaggaaacgacccggccagcatccgcccactacatttgtgacatatcgaccacggtgcagtgtctgtctgaggagacggtgggctatcacgccccgccgaactcacactccatcggtattgagatatgcgctgacggtgggtcgcatgcctcgttttcgaaccctgcccacgcctacacccgcgagcagtggttgagccctcaggtgtggcctgctgtggagcgtgccgcgatgctggcgcgcggtatctgtcaacgccacaacatcccgatccgccgcctctcgatcgctgacgtcaaggccgggaagcgcggcatctgcggccacaacgaggtgtccgaggccttccaccaatccgaccatgacgaccccggtcct

SEQ ID NO: 212 - DNA, 333 bp, Artificial Sequence
tatttcccgtgggacgggtttatcgcgcttgttaatggccattccgcaccatcacgccaggaggaactaactgtgtcagatgtcaatatgctcaaaggtcttattcagcaatcgaacaagcagctgcaccacgatatcggtgttgtgcagacgcaggcgggtaacctccgccgccagctggaatccctgtcatgggtgaagaacccggtcagcggcaagctgtggcgcaccaaggacgccttgtggtcgatctggtactacgtgctggactgccgatctcgtctcggcaaactcgaggcccgcctgtcgacgctggaaaagaaggtgaagtga

SEQ ID NO: 213 - DNA, 282 bp, Artificial Sequence
tcacgccaggaggaactaactgtgtcagatgtcaatatgctcaaaggtcttattcagcaatcgaacaagcagctgcaccacgatatcggtgttgtgcagacgcaggcgggtaacctccgccgccagctggaatccctgtcatgggtgaagaacccggtcagcggcaagctgtggcgcaccaaggacgccttgtggtcgatctggtactacgtgctggactgccgatctcgtctcggcaaactcgaggcccgcctgtcgacgctggaaaagaaggtgaagtga

SEQ ID NO: 214 - DNA, 600 bp, Artificial Sequence
atgacgttcattcaggccgcgcatcacagcagcggctccaatctgccacccacgagggtggtgatccatgcgacatgccccgagatgggattcccgaaggccagtgcgaagggcagggctgtctcgacggcccgatacttccagtctgcgagctcgggcggtagcgcccactatgttgtcgacatcggcgagacggtgcagtgtctcggtgagaacgtgatcgcgtggcacgccccgcccaatgcccacagtctcggcatcgagatctgcgcggacgggggatcggccacctccttctccaatcccaaggtgcgctacacgcgggcgcagtggctgagcccgcaggtgtggcccgccgtgctccgtgccgcagcactcacccggaagatgtgcagcaagtacggcatccccgtcgtcaagctgtccgcgtcggacctcaaggccggaaagaagggcatctgcggccacgtggatgtcagcaatgctttccaccagtccgaccacgacgaccccggccccgacttcccgtgggccgaattcatggcagccgtcaaaggcggcaccaccacacaggaagatgaggatgaaatgaaggaagct

SEQ ID NO: 215 - DNA, 519 bp, Artificial Sequence
atgacgttcattcaggccgcgcatcacagcagcggctccaatctgccacccacgagggtggtgatccatgcgacatgccccgagatgggattcccgaaggccagtgcgaagggcagggctgtctcgacggcccgatacttccagtctgcgagctcgggcggtagcgcccactatgttgtcgacatcggcgagacggtgcagtgtctcggtgagaacgtgatcgcgtggcacgccccgcccaatgcccacagtctcggcatcgagatctgcgcggacgggggatcggccacctccttctccaatcccaaggtgcgctacacgcgggcgcagtggctgagcccgcaggtgtggcccgccgtgctccgtgccgcagcactcacccggaagatgtgcagcaagtacggcatccccgtcgtcaagctgtccgcgtcggacctcaaggccggaaagaagggcatctgcggccacgtggatgtcagcaatgctttccaccagtccgaccacgacgaccccggcccc

SEQ ID NO: 216 - DNA, 555 bp, Artificial Sequence
atgacgttcattcaggccgcgcatcacagcagcggctccaatctgccacccacgagggtggtgatccatgcgacatgccccgagatgggattcccgaaggccagtgcgaagggcagggctgtctcgacggcccgatacttccagtctgcgagctcgggcggtagcgcccactatgttgtcgacatcggcgagacggtgcagtgtctcggtgagaacgtgatcgcgtggcacgccccgcccaatgcccacagtctcggcatcgagatctgcgcggacgggggatcggccacctccttctccaatcccaaggtgcgctacacgcgggcgcagtggctgagcccgcaggtgtggcccgccgtgctccgtgccgcagcactcacccggaagatgtgcagcaagtacggcatccccgtcgtcaagctgtccgcgtcggacctcaaggccggaaagaagggcatctgcggccacgtggatgtcagcaatgctttccaccagtccgaccacgacgaccccggccccgacttcccgtgggccgaattcatggcagccgtcaaa

SEQ ID NO: 217 - DNA, 285 bp, Artificial Sequence
gacttcccgtgggccgaattcatggcagccgtcaaaggcggcaccaccacacaggaagatgaggatgaaatgaaggaagctgactggcagcgcatggagaggctcgttgacgcgaggctgaagtacgctggtatcgccaagaatgatgacccggtcttcaagcccgacaagtcctcgtcgtggccctggaggaccgcgctgtggagcatctcctactacgcgacccacagctacaacacgatctgcaatatcgcccgcaagctcggcgcagaggtgtccaagtga

SEQ ID NO: 218 - DNA, 558 bp, Artificial Sequence
atgaaatacattcccgcgacacatcacggaggccacacgaacacccccttcacccggatcgtgatccacgccacctgccccgaccttggcttcccccacgcatcagctggtggacaggcaaaagccaccgcacgctatttccaatcagagcagtctgccggatcagcacactatgtgtgcgacatcgccgagactatccaatgcctgcccgatgacgtgatcgcctggcacgccccaccaaacagaaggtcgatcggaatcgaaatatgtgccgacggcggctcccgctcctcattccagcaccccgagcacgcctacaccagatcccaatggctcagcccccaagtgtggcccgccgtcgcccgtgccgccgcgctcacccgcgacctctgccaccgccacaacattccgatgcaacaactctccgttgctgatgtgaaagccgggaagcacggaatctgcggccacaacgacgtatccgaggcattccacaagtccgaccatgacgaccccggccccacattcccgtgggaccaattcatcaaagaggttagaaca

SEQ ID NO: 219 - DNA, 519 bp, Artificial Sequence
atgaaatacattcccgcgacacatcacggaggccacacgaacacccccttcacccggatcgtgatccacgccacctgccccgaccttggcttcccccacgcatcagctggtggacaggcaaaagccaccgcacgctatttccaatcagagcagtctgccggatcagcacactatgtgtgcgacatcgccgagactatccaatgcctgcccgatgacgtgatcgcctggcacgccccaccaaacagaaggtcgatcggaatcgaaatatgtgccgacggcggctcccgctcctcattccagcaccccgagcacgcctacaccagatcccaatggctcagcccccaagtgtggcccgccgtcgcccgtgccgccgcgctcacccgcgacctctgccaccgccacaacattccgatgcaacaactctccgttgctgatgtgaaagccgggaagcacggaatctgcggccacaacgacgtatccgaggcattccacaagtccgaccatgacgaccccggcccc

SEQ ID NO: 220 - DNA, 336 bp, Artificial Sequence
acattcccgtgggaccaattcatcaaagaggttagaacaccaggacaacaagatacgaaaccttccgtaccaacaccatcactcacagaaataggagatcaggacatgaacgggtgctactacaacctcaattcgaaaacacggacgtaccttatcttcgatagccgttccggattttaccacgaattctcccaaggcaatgggaacggccccatgagcccagactatgtaaatccgatcgccaaaggatgggacaccggatcatggccggcaatctccccaggccacgcgaaagtgctcaaggccgccctcgataaagtccggaaaggaatctga

SEQ ID NO: 221 - DNA, 297 bp, Artificial Sequence
ccaggacaacaagatacgaaaccttccgtaccaacaccatcactcacagaaataggagatcaggacatgaacgggtgctactacaacctcaattcgaaaacacggacgtaccttatcttcgatagccgttccggattttaccacgaattctcccaaggcaatgggaacggccccatgagcccagactatgtaaatccgatcgccaaaggatgggacaccggatcatggccggcaatctccccaggccacgcgaaagtgctcaaggccgccctcgataaagtccggaaaggaatctga

SEQ ID NO: 222 - DNA, 309 bp, Artificial Sequence
gaggttagaacaccaggacaacaagatacgaaaccttccgtaccaacaccatcactcacagaaataggagatcaggacatgaacgggtgctactacaacctcaattcgaaaacacggacgtaccttatcttcgatagccgttccggattttaccacgaattctcccaaggcaatgggaacggccccatgagcccagactatgtaaatccgatcgccaaaggatgggacaccggatcatggccggcaatctccccaggccacgcgaaagtgctcaaggccgccctcgataaagtccggaaaggaatctga

SEQ ID NO: 223 - protein, 310 aa, Artificial Sequence
MTFIQAAHHSSGSNLPPTRVVIHATCPELGFPRASAKGRAVSTARYFQSAISGGSAHYVVDVGETVQCLAEDVIAWHAPPNSRSLGIEICADGGSATSFKNPNVRYSRAQWLSPQVWPAVLRAAALTRQMCQKYGIPVTKLSASDLKAGKKGICGHVDVSNAWHQSDHDDPGPDFPWAEFMAAVKGGATNPDELELTGGTFPWDQFIKEVRTPGQQDTKPSVPTPSLTEIGDQDMNGCYYNLNSKTRTYLIFDSRSGFYHEFSQGNGNGPMSPDYVNPIAKGWDTGSWPAISPGHAKVLKAALDKVRKGI

SEQ ID NO: 224 - protein, 309 aa, Artificial Sequence
MTFIQAAHHSSGSNLPPTRVVIHATCPELGFPRASAKGRAVSTARYFQSAISGGSAHYVVDVGETVQCLAEDVIAWHAPPNSRSLGIEICADGGSATSFKNPNVRYSRAQWLSPQVWPAVLRAAALTRQMCQKYGIPVTKLSASDLKAGKKGICGHVDVSNAWHQSDHDDPGPDFPWAEFMAAVKGGATNPDELELTGGYFPWDGFIALVNGHSAPSRQEELTVSDVNMLKGLIQQSNKQLHHDIGVVQTQAGNLRRQLESLSWVKNPVSGKLWRTKDALWSIWYYVLDCRSRLGKLEARLSTLEKKVK

SEQ ID NO: 225 - protein, 313 aa, Artificial Sequence
MTFIQAAHHSSGSNLPPTRVVIHATCPEMGFPKASAKGRAVSTARYFQSASSGGSAHYVVDIGETVQCLGENVIAWHAPPNAHSLGIEICADGGSATSFSNPKVRYTRAQWLSPQVWPAVLRAAALTRKMCSKYGIPVVKLSASDLKAGKKGICGHVDVSNAFHQSDHDDPGPDFPWAEFMAAVKGGTTTQEDEDEMKEAGGTFPWDQFIKEVRTPGQQDTKPSVPTPSLTEIGDQDMNGCYYNLNSKTRTYLIFDSRSGFYHEFSQGNGNGPMSPDYVNPIAKGWDTGSWPAISPGHAKVLKAALDKVRKGI

SEQ ID NO: 226 - protein, 298 aa, Artificial Sequence
MTFIQAAHHSSGSNLPPTRVVIHATCPELGFPRASAKGRAVSTARYFQSAISGGSAHYVVDVGETVQCLAEDVIAWHAPPNSRSLGIEICADGGSATSFKNPNVRYSRAQWLSPQVWPAVLRAAALTRQMCQKYGIPVTKLSASDLKAGKKGICGHVDVSNAWHQSDHDDPGPDFPWAEFMAAVKGGATNPDELELTGGGSGESGELSMADVKALHDQIKQLSGQVAQSVNKLHHDVGVVQVQNGNLKKQVDSLSMVKNPVTGKLWRTRDAIWSIWYYVLECRSRIGKLEAEVARLKK

SEQ ID NO: 227 - protein, 294 aa, Artificial Sequence
MTFIQAAHHSSGSNLPPTRVVIHATCPELGFPRASAKGRAVSTARYFQSAISGGSAHYVVDVGETVQCLAEDVIAWHAPPNSRSLGIEICADGGSATSFKNPNVRYSRAQWLSPQVWPAVLRAAALTRQMCQKYGIPVTKLSASDLKAGKKGICGHVDVSNAWHQSDHDDPGPDFPWAEFMAAVKGGATNPDELELTGGKNTNKGELSMSDVNTLTKLIKASNNQLHHDIGVVQTQNGTLKSKIDNLSWVKNPVTGKKWSTKDALWSVWYYVLECRNRIQAIENRLSDIEKKVK

SEQ ID NO: 228 - protein, 308 aa, Artificial Sequence
MTFIQARHHGGNSNTPITRLVIHATCPDVGYPSASKAGRAVSTAEYFASTSRSASAHYVCDVSATVQCLSEETIGYHAPPNSHSIGIEICADGGSRASFEKASHAYTREQWLSPQVWPAVERAAILARGICHRHHIPVRKLTTAQVKSGMSGICGHDNVSDAFHQSDHDDPGPYFPWNEFIAAIQGKNTNKGELSGGTFPWDQFIKEVRTPGQQDTKPSVPTPSLTEIGDQDMNGCYYNLNSKTRTYLIFDSRSGFYHEFSQGNGNGPMSPDYVNPIAKGWDTGSWPAISPGHAKVLKAALDKVRKGI

SEQ ID NO: 229 - protein, 309 aa, Artificial Sequence
MTFIQARHHGGNSNAPITRLVIHATCPDVGYPSASKAGRAVSTANYFATTDRPASAHYVCDIATTVQCLSEETIGYHAPPNSHSIGIEICADGGSHASFEKASHAYTRDQWLSDDVWPAVERAAILARDICQRHRIPVRKLSTAQVKAGLSGICGHDNVSGAFHQSDHDDPGPYFPWDQFMALVQGKPATPGDLTMGGTFPWDQFIKEVRTPGQQDTKPSVPTPSLTEIGDQDMNGCYYNLNSKTRTYLIFDSRSGFYHEFSQGNGNGPMSPDYVNPIAKGWDTGSWPAISPGHAKVLKAALDKVRKGI

SEQ ID NO: 230 - protein, 313 aa, Artificial Sequence
MTFIQAKHHGGHNNPPVTRLVIHATCPDVGYPSASRAGRAVSTAHYFQETTRPASAHYICDISTTVQCLSEETVGYHAPPNSHSIGIEICADGGSHASFSNPAHAYTREQWLSPQVWPAVERAAMLARGICQRHNIPIRRLSIADVKAGKRGICGHNEVSEAFHQSDHDDPGPYFPWDGFIALVNGHSAPSRQEELTVSDGGTFPWDQFIKEVRTPGQQDTKPSVPTPSLTEIGDQDMNGCYYNLNSKTRTYLIFDSRSGFYHEFSQGNGNGPMSPDYVNPIAKGWDTGSWPAISPGHAKVLKAALDKVRKGI

SEQ ID NO: 231 - protein, 288 aa, Artificial Sequence
MGFPKASAKGRAVSTARYFQSASSGGSAHYVVDIGETVQCLGENVIAWHAPPNAHSLGIEICADGGSATSFSNPKVRYTRAQWLSPQVWPAVLRAAALTRKMCSKYGIPVVKLSASDLKAGKKGICGHVDVSNAFHQSDHDDPGPDFPWAEFMAAVKGGTTTQEDEDEMKEAGGWFPWDKFMAVVNGHGGGSSSEELSMADVQALHNQIKQLSAQVAQSVNKLHHDVGVVQVQNGDLGKRVDALSWVKNPVTGKLWRSKDALWSVWYYVLECRSRLDRLESAVNDLKK

SEQ ID NO: 232 - protein, 312 aa, Artificial Sequence
MTFIQAAHHSSGSNLPPTRVVIHATCPEMGFPKASAKGRAVSTARYFQSASSGGSAHYVVDIGETVQCLGENVIAWHAPPNAHSLGIEICADGGSATSFSNPKVRYTRAQWLSPQVWPAVLRAAALTRKMCSKYGIPVVKLSASDLKAGKKGICGHVDVSNAFHQSDHDDPGPDFPWAEFMAAVKGGTTTQEDEDEMKEAGGYFPWDGFIALVNGHSAPSRQEELTVSDVNMLKGLIQQSNKQLHHDIGVVQTQAGNLRRQLESLSWVKNPVSGKLWRTKDALWSIWYYVLDCRSRLGKLEARLSTLEKKVK

SEQ ID NO: 233 - protein, 292 aa, Artificial Sequence
MTFIQARHHGGNSNTPITRLVIHATCPDVGYPSASKAGRAVSTAEYFASTSRSASAHYVCDVSATVQCLSEETIGYHAPPNSHSIGIEICADGGSRASFEKASHAYTREQWLSPQVWPAVERAAILARGICHRHHIPVRKLTTAQVKSGMSGICGHDNVSDAFHQSDHDDPGPYFPWNEFIAAIQGKNTNKGELSGGKNTNKGELSMSDVNTLTKLIKASNNQLHHDIGVVQTQNGTLKSKIDNLSWVKNPVTGKKWSTKDALWSVWYYVLECRNRIQAIENRLSDIEKKVK

SEQ ID NO: 234 - protein, 313 aa, Artificial Sequence
MTFIQAAHHSSGSNLPPTRVVIHATCPELGFPRASAKGRAVSTARYFQSAISGGSAHYVVDVGETVQCLAEDVIAWHAPPNSRSLGIEICADGGSATSFKNPNVRYSRAQWLSPQVWPAVLRAAALTRQMCQKYGIPVTKLSASDLKAGKKGICGHVDVSNAWHQSDHDDPGPDFPWAEFMAAVKGGATNPDELELTGGWFPWDKFMAVVNGHGGGSSSEELSMADVQALHNQIKQLSAQVAQSVNKLHHDVGVVQVQNGDLGKRVDALSWVKNPVTGKLWRSKDALWSVWYYVLECRSRLDRLESAVNDLKK

SEQ ID NO: 235 - protein, 308 aa, Artificial Sequence
MRYIPAAHHSAGSNSPVNRVVIHATCPDVGFPSASRKGRAVSTANYFASPSAGGSAHYVCDVGETVQCLSESTIGWHAPPNPHSLGIEICADGGSHASFRVPGHAYTREQWLDPRVWPAVEKAAVLCRQLCDKYNVPKRKLSVSDLKAGRRGVCGHTDVTDAWHQSDHDDPGPWFPWDRFMAVVNGGSGESGELSGGTFPWDQFIKEVRTPGQQDTKPSVPTPSLTEIGDQDMNGCYYNLNSKTRTYLIFDSRSGFYHEFSQGNGNGPMSPDYVNPIAKGWDTGSWPAISPGHAKVLKAALDKVRKGI

SEQ ID NO: 236 - protein, 306 aa, Artificial Sequence
MTFIQAAHRGGTSNTPITRLVIHATCPDVGFPSASRAGRAVSTAEYFASTSRSASAHYVCDISTTVQCLSEATIGYHAPPNAHSIGIEICADGGSRASFEKASHAYTREQWLSPQVWPAVERAAILARDICHRHHIPIRRLSVAQVRAGERGICGHNEVSEAFHQSDHDDPGPYFPWNEFIAAVQGKTTTPEGGGTFPWDQFIKEVRTPGQQDTKPSVPTPSLTEIGDQDMNGCYYNLNSKTRTYLIFDSRSGFYHEFSQGNGNGPMSPDYVNPIAKGWDTGSWPAISPGHAKVLKAALDKVRKGI

SEQ ID NO: 237 - protein, 290 aa, Artificial Sequence
MTFIQAAHRGGTSNTPITRLVIHATCPDVGFPSASRAGRAVSTAEYFASTSRSASAHYVCDISTTVQCLSEATIGYHAPPNAHSIGIEICADGGSRASFEKASHAYTREQWLSPQVWPAVERAAILARDICHRHHIPIRRLSVAQVRAGERGICGHNEVSEAFHQSDHDDPGPYFPWNEFIAAVQGKTTTPEGGGKNTNKGELSMSDVNTLTKLIKASNNQLHHDIGVVQTQNGTLKSKIDNLSWVKNPVTGKKWSTKDALWSVWYYVLECRNRIQAIENRLSDIEKKVK

SEQ ID NO: 238 - protein, 310 aa, Artificial Sequence
MRYIPAAHHSAGSNKPVNRVVIHATCPDVGFPSASRKGRAVSTANYFASPSSGGSAHYVCDIGETVQCLSESTIGWHAPPNPHSLGIEICADGGSHASFRVPGHAYTREQWLDPRVWPAVERAAILCRQLCDKHGVPKRKLSVADLKAGKRGVCGHVDVTDAWHQSDHDDPGPWFPWDKFMAVVNGHGGGSSSEELSMADVQALHNQIKQLSAGGKNTNKGELSMSDVNTLTKLIKASNNQLHHDIGVVQTQNGTLKSKIDNLSWVKNPVTGKKWSTKDALWSVWYYVLECRNRIQAIENRLSDIEKKVK

SEQ ID NO: 239 - protein, 299 aa, Artificial Sequence
MKYIPATHHGGHTNTPFTRIVIHATCPDLGFPHASAGGQAKATARYFQSEQSAGSAHYVCDIAETIQCLPDDVIAWHAPPNRRSIGIEICADGGSRSSFQHPEHAYTRSQWLSPQVWPAVARAAALTRDLCHRHNIPMQQLSVADVKAGKHGICGHNDVSEAFHKSDHDDPGPTFPWDQFIKEVRTGGTFPWDQFIKEVRTPGQQDTKPSVPTPSLTEIGDQDMNGCYYNLNSKTRTYLIFDSRSGFYHEFSQGNGNGPMSPDYVNPIAKGWDTGSWPAISPGHAKVLKAALDKVRKGI

SEQ ID NO: 240 - protein, 293 aa, Artificial Sequence
MTFIQARHHGGNSNAPITRLVIHATCPDVGYPSASKAGRAVSTANYFATTDRPASAHYVCDIATTVQCLSEETIGYHAPPNSHSIGIEICADGGSHASFEKASHAYTRDQWLSDDVWPAVERAAILARDICQRHRIPVRKLSTAQVKAGLSGICGHDNVSGAFHQSDHDDPGPYFPWDQFMALVQGKPATPGDLTMGGKNTNKGELSMSDVNTLTKLIKASNNQLHHDIGVVQTQNGTLKSKIDNLSWVKNPVTGKKWSTKDALWSVWYYVLECRNRIQAIENRLSDIEKKVK

SEQ ID NO: 241 - protein, 289 aa, Artificial Sequence
MAYPYIGALKHGGKQGKIQRIVIHATVSPCVRGGARNVAKYFQSSAAGGSAHYVVDPGEIIQCVKDDVVAYHAPPNTGTLGIELCDPQAGSPKRWSNEAHQAMLVLAAKLVRELAAKHDVPLVRVTAAQLRAGKRGICSHVAVSDAFGQSDHGDPEVAGPFPWAKFMQLIKEEDDMGGTFPWDQFIKEVRTPGQQDTKPSVPTPSLTEIGDQDMNGCYYNLNSKTRTYLIFDSRSGFYHEFSQGNGNGPMSPDYVNPIAKGWDTGSWPAISPGHAKVLKAALDKVRKGI

SEQ ID NO: 242 - protein, 311 aa, Artificial Sequence
MTFIQAAHHSSGSNLPPTRVVIHATCPEMGFPKASAKGRAVSTARYFQSASSGGSAHYVVDIGETVQCLGENVIAWHAPPNAHSLGIEICADGGSATSFSNPKVRYTRAQWLSPQVWPAVLRAAALTRKMCSKYGIPVVKLSASDLKAGKKGICGHVDVSNAFHQSDHDDPGPDFPWAEFMAAVKGGTTTQEDEDEMKEAGGYFPWNEFIAAVQGKTTTPEGELSMSDVNTLTKLIKASNDQLHYDIGVVQTQNGNIKKKIDNLSWVKNPVTGKKWSTKDALWSVWYYVLECRNRIQAIENRIYDLEKKVK

SEQ ID NO: 243 - protein, 310 aa, Artificial Sequence
MTFIQAAHHSSGSNLPPTRVVIHATCPEMGFPKASAKGRAVSTARYFQSASSGGSAHYVVDIGETVQCLGENVIAWHAPPNAHSLGIEICADGGSATSFSNPKVRYTRAQWLSPQVWPAVLRAAALTRKMCSKYGIPVVKLSASDLKAGKKGICGHVDVSNAFHQSDHDDPGPDFPWAEFMAAVKGGTTTQEDEDEMKEAGGYFPWDQFMALVQGKPATPGDLTMADISKLTDAIKASNRQLHHDIGVVQTQNGKLREQIERITWVKNPVTGKKWRITDALWSIWHYVLECRTRIQRLDARLSEVEKKVK

SEQ ID NO: 244 - protein, 326 aa, Artificial Sequence
MRYIPAAHHSAGSNKPVNRVVIHATCPDVGFPSASRKGRAVSTANYFASPSSGGSAHYVCDIGETVQCLSESTIGWHAPPNPHSLGIEICADGGSHASFRVPGHAYTREQWLDPRVWPAVERAAILCRQLCDKHGVPKRKLSVADLKAGKRGVCGHVDVTDAWHQSDHDDPGPWFPWDKFMAVVNGHGGGSSSEELSMADVQALHNQIKQLSAGGTFPWDQFIKEVRTPGQQDTKPSVPTPSLTEIGDQDMNGCYYNLNSKTRTYLIFDSRSGFYHEFSQGNGNGPMSPDYVNPIAKGWDTGSWPAISPGHAKVLKAALDKVRKGI

SEQ ID NO: 245 - protein, 302 aa, Artificial Sequence
MKYIPATHHGGHTNTPFTRIVIHATCPDLGFPHASAGGQAKATARYFQSEQSAGSAHYVCDIAETIQCLPDDVIAWHAPPNRRSIGIEICADGGSRSSFQHPEHAYTRSQWLSPQVWPAVARAAALTRDLCHRHNIPMQQLSVADVKAGKHGICGHNDVSEAFHKSDHDDPGPTFPWDQFIKEVRTGGWFPWDKFMAVVNGHGGGSSSEELSMADVQALHNQIKQLSAQVAQSVNKLHHDVGVVQVQNGDLGKRVDALSWVKNPVTGKLWRSKDALWSVWYYVLECRSRLDRLESAVNDLKK

SEQ ID NO: 246 - protein, 303 aa, Artificial Sequence
MTFIQAAHHSSGSNLPPTRVVIHATCPEMGFPKASAKGRAVSTARYFQSASSGGSAHYVVDIGETVQCLGENVIAWHAPPNAHSLGIEICADGGSATSFSNPKVRYTRAQWLSPQVWPAVLRAAALTRKMCSKYGIPVVKLSASDLKAGKKGICGHVDVSNAFHQSDHDDPGPDFPWAEFMAAVKGGTTTQEDEDEMKEAGGNGGSGDSGELTVADVKALHDQIKQLSAQLTGSVNKLHHDVGVVQVQNGDLGKRVDALSWVKNPVTGKLWRTKDALWSVWYYVLECRSRIDRLESAVNGLKK

SEQ ID NO: 247 - protein, 308 aa, Artificial Sequence
MTFIQAAHHSSGSNLPPTRVVIHATCPELGFPRASAKGRAVSTARYFQSAISGGSAHYVVDVGETVQCLAEDVIAWHAPPNSRSLGIEICADGGSATSFKNPNVRYSRAQWLSPQVWPAVLRAAALTRQMCQKYGIPVTKLSASDLKAGKKGICGHVDVSNAWHQSDHDDPGPDFPWAEFMAAVKGGATNPDELELTGGYFPWNEFIAAVQGKTTTPEGELSMSDVNTLTKLIKASNDQLHYDIGVVQTQNGNIKKKIDNLSWVKNPVTGKKWSTKDALWSVWYYVLECRNRIQAIENRIYDLEKKVK

SEQ ID NO: 248 - protein, 306 aa, Artificial Sequence
MTFIQARHHGGNSNTPITRLVIHATCPDVGYPSASKAGRAVSTAEYFASTSRSASAHYVCDVSATVQCLSEETIGYHAPPNSHSIGIEICADGGSRASFEKASHAYTREQWLSPQVWPAVERAAILARGICHRHHIPVRKLTTAQVKSGMSGICGHDNVSDAFHQSDHDDPGPYFPWNEFIAAIQGKNTNKGELSGGYFPWNEFIAAVQGKTTTPEGELSMSDVNTLTKLIKASNDQLHYDIGVVQTQNGNIKKKIDNLSWVKNPVTGKKWSTKDALWSVWYYVLECRNRIQAIENRIYDLEKKVK

SEQ ID NO: 249 - protein, 297 aa, Artificial Sequence
MTFIQAKHHGGHNNPPVTRLVIHATCPDVGYPSASRAGRAVSTAHYFQETTRPASAHYICDISTTVQCLSEETVGYHAPPNSHSIGIEICADGGSHASFSNPAHAYTREQWLSPQVWPAVERAAMLARGICQRHNIPIRRLSIADVKAGKRGICGHNEVSEAFHQSDHDDPGPYFPWDGFIALVNGHSAPSRQEELTVSDGGKNTNKGELSMSDVNTLTKLIKASNNQLHHDIGVVQTQNGTLKSKIDNLSWVKNPVTGKKWSTKDALWSVWYYVLECRNRIQAIENRLSDIEKKVK

SEQ ID NO: 250 - protein, 297 aa, Artificial Sequence
MTFIQAAHHSSGSNLPPTRVVIHATCPEMGFPKASAKGRAVSTARYFQSASSGGSAHYVVDIGETVQCLGENVIAWHAPPNAHSLGIEICADGGSATSFSNPKVRYTRAQWLSPQVWPAVLRAAALTRKMCSKYGIPVVKLSASDLKAGKKGICGHVDVSNAFHQSDHDDPGPDFPWAEFMAAVKGGTTTQEDEDEMKEAGGKNTNKGELSMSDVNTLTKLIKASNNQLHHDIGVVQTQNGTLKSKIDNLSWVKNPVTGKKWSTKDALWSVWYYVLECRNRIQAIENRLSDIEKKVK

SEQ ID NO: 251 - protein, 290 aa, Artificial Sequence
MTFIQARHHGGNSNTPITRLVIHATCPDVGYPSASKAGRAVSTAEYFASTSRSASAHYVCDVSATVQCLSEETIGYHAPPNSHSIGIEICADGGSRASFEKASHAYTREQWLSPQVWPAVERAAILARGICHRHHIPVRKLTTAQVKSGMSGICGHDNVSDAFHQSDHDDPGPYFPWNEFIAAIQGGGEVRTPGQQDTKPSVPTPSLTEIGDQDMNGCYYNLNSKTRTYLIFDSRSGFYHEFSQGNGNGPMSPDYVNPIAKGWDTGSWPAISPGHAKVLKAALDKVRKGI

SEQ ID NO: 252 - protein, 286 aa, Artificial Sequence
MTFIQARHHGGNSNTPITRLVIHATCPDVGYPSASKAGRAVSTAEYFASTSRSASAHYVCDVSATVQCLSEETIGYHAPPNSHSIGIEICADGGSRASFEKASHAYTREQWLSPQVWPAVERAAILARGICHRHHIPVRKLTTAQVKSGMSGICGHDNVSDAFHQSDHDDPGPYFPWNEFIAAIQGGGPGQQDTKPSVPTPSLTEIGDQDMNGCYYNLNSKTRTYLIFDSRSGFYHEFSQGNGNGPMSPDYVNPIAKGWDTGSWPAISPGHAKVLKAALDKVRKGI

SEQ ID NO: 253 - protein, 289 aa, Artificial Sequence
MTFIQAAHHSSGSNLPPTRVVIHATCPELGFPRASAKGRAVSTARYFQSAISGGSAHYVVDVGETVQCLAEDVIAWHAPPNSRSLGIEICADGGSATSFKNPNVRYSRAQWLSPQVWPAVLRAAALTRQMCQKYGIPVTKLSASDLKAGKKGICGHVDVSNAWHQSDHDDPGPDFPWAEFMAAVKGGEVRTPGQQDTKPSVPTPSLTEIGDQDMNGCYYNLNSKTRTYLIFDSRSGFYHEFSQGNGNGPMSPDYVNPIAKGWDTGSWPAISPGHAKVLKAALDKVRKGI

SEQ ID NO: 254 - protein, 283 aa, Artificial Sequence
MTFIQARHHGGNSNTPITRLVIHATCPDVGYPSASKAGRAVSTAEYFASTSRSASAHYVCDVSATVQCLSEETIGYHAPPNSHSIGIEICADGGSRASFEKASHAYTREQWLSPQVWPAVERAAILARGICHRHHIPVRKLTTAQVKSGMSGICGHDNVSDAFHQSDHDDPGPYFPWNEFIAAIQGGGKNTNKGELSMSDVNTLTKLIKASNNQLHHDIGVVQTQNGTLKSKIDNLSWVKNPVTGKKWSTKDALWSVWYYVLECRNRIQAIENRLSDIEKKVK

SEQ ID NO: 255 - protein, 298 aa, Artificial Sequence
MTFIQAAHHSSGSNLPPTRVVIHATCPELGFPRASAKGRAVSTARYFQSAISGGSAHYVVDVGETVQCLAEDVIAWHAPPNSRSLGIEICADGGSATSFKNPNVRYSRAQWLSPQVWPAVLRAAALTRQMCQKYGIPVTKLSASDLKAGKKGICGHVDVSNAWHQSDHDDPGPDFPWAEFMAAVKGGTFPWDQFIKEVRTPGQQDTKPSVPTPSLTEIGDQDMNGCYYNLNSKTRTYLIFDSRSGFYHEFSQGNGNGPMSPDYVNPIAKGWDTGSWPAISPGHAKVLKAALDKVRKGI

SEQ ID NO: 256 - protein, 299 aa, Artificial Sequence
MTFIQARHHGGNSNTPITRLVIHATCPDVGYPSASKAGRAVSTAEYFASTSRSASAHYVCDVSATVQCLSEETIGYHAPPNSHSIGIEICADGGSRASFEKASHAYTREQWLSPQVWPAVERAAILARGICHRHHIPVRKLTTAQVKSGMSGICGHDNVSDAFHQSDHDDPGPYFPWNEFIAAIQGGGTFPWDQFIKEVRTPGQQDTKPSVPTPSLTEIGDQDMNGCYYNLNSKTRTYLIFDSRSGFYHEFSQGNGNGPMSPDYVNPIAKGWDTGSWPAISPGHAKVLKAALDKVRKGI

SEQ ID NO: 257 - protein, 289 aa, Artificial Sequence
MTFIQAAHHSSGSNLPPTRVVIHATCPEMGFPKASAKGRAVSTARYFQSASSGGSAHYVVDIGETVQCLGENVIAWHAPPNAHSLGIEICADGGSATSFSNPKVRYTRAQWLSPQVWPAVLRAAALTRKMCSKYGIPVVKLSASDLKAGKKGICGHVDVSNAFHQSDHDDPGPDFPWAEFMAAVKGGEVRTPGQQDTKPSVPTPSLTEIGDQDMNGCYYNLNSKTRTYLIFDSRSGFYHEFSQGNGNGPMSPDYVNPIAKGWDTGSWPAISPGHAKVLKAALDKVRKGI

SEQ ID NO: 258 - protein, 285 aa, Artificial Sequence
MTFIQAAHHSSGSNLPPTRVVIHATCPEMGFPKASAKGRAVSTARYFQSASSGGSAHYVVDIGETVQCLGENVIAWHAPPNAHSLGIEICADGGSATSFSNPKVRYTRAQWLSPQVWPAVLRAAALTRKMCSKYGIPVVKLSASDLKAGKKGICGHVDVSNAFHQSDHDDPGPDFPWAEFMAAVKGGPGQQDTKPSVPTPSLTEIGDQDMNGCYYNLNSKTRTYLIFDSRSGFYHEFSQGNGNGPMSPDYVNPIAKGWDTGSWPAISPGHAKVLKAALDKVRKGI

SEQ ID NO: 259 - protein, 295 aa, Artificial Sequence
MTFIQAAHHSSGSNLPPTRVVIHATCPELGFPRASAKGRAVSTARYFQSAISGGSAHYVVDVGETVQCLAEDVIAWHAPPNSRSLGIEICADGGSATSFKNPNVRYSRAQWLSPQVWPAVLRAAALTRQMCQKYGIPVTKLSASDLKAGKKGICGHVDVSNAWHQSDHDDPGPDFPWAEFMAAVKGGATNPGGEVRTPGQQDTKPSVPTPSLTEIGDQDMNGCYYNLNSKTRTYLIFDSRSGFYHEFSQGNGNGPMSPDYVNPIAKGWDTGSWPAISPGHAKVLKAALDKVRKGI

SEQ ID NO: 260 - protein, 291 aa, Artificial Sequence
MTFIQAAHHSSGSNLPPTRVVIHATCPELGFPRASAKGRAVSTARYFQSAISGGSAHYVVDVGETVQCLAEDVIAWHAPPNSRSLGIEICADGGSATSFKNPNVRYSRAQWLSPQVWPAVLRAAALTRQMCQKYGIPVTKLSASDLKAGKKGICGHVDVSNAWHQSDHDDPGPDFPWAEFMAAVKGGATNPGGPGQQDTKPSVPTPSLTEIGDQDMNGCYYNLNSKTRTYLIFDSRSGFYHEFSQGNGNGPMSPDYVNPIAKGWDTGSWPAISPGHAKVLKAALDKVRKGI

SEQ ID NO: 261 - protein, 288 aa, Artificial Sequence
MTFIQAAHHSSGSNLPPTRVVIHATCPEMGFPKASAKGRAVSTARYFQSASSGGSAHYVVDIGETVQCLGENVIAWHAPPNAHSLGIEICADGGSATSFSNPKVRYTRAQWLSPQVWPAVLRAAALTRKMCSKYGIPVVKLSASDLKAGKKGICGHVDVSNAFHQSDHDDPGPDFPWAEFMAAVKGGNGGSGDSGELTVADVKALHDQIKQLSAQLTGSVNKLHHDVGVVQVQNGDLGKRVDALSWVKNPVTGKLWRTKDALWSVWYYVLECRSRIDRLESAVNGLKK

SEQ ID NO: 262 - protein, 298 aa, Artificial Sequence
MTFIQAAHHSSGSNLPPTRVVIHATCPEMGFPKASAKGRAVSTARYFQSASSGGSAHYVVDIGETVQCLGENVIAWHAPPNAHSLGIEICADGGSATSFSNPKVRYTRAQWLSPQVWPAVLRAAALTRKMCSKYGIPVVKLSASDLKAGKKGICGHVDVSNAFHQSDHDDPGPDFPWAEFMAAVKGGTFPWDQFIKEVRTPGQQDTKPSVPTPSLTEIGDQDMNGCYYNLNSKTRTYLIFDSRSGFYHEFSQGNGNGPMSPDYVNPIAKGWDTGSWPAISPGHAKVLKAALDKVRKGI

SEQ ID NO: 263 - protein, 301 aa, Artificial Sequence
MTFIQAAHHSSGSNLPPTRVVIHATCPELGFPRASAKGRAVSTARYFQSAISGGSAHYVVDVGETVQCLAEDVIAWHAPPNSRSLGIEICADGGSATSFKNPNVRYSRAQWLSPQVWPAVLRAAALTRQMCQKYGIPVTKLSASDLKAGKKGICGHVDVSNAWHQSDHDDPGPDFPWAEFMAAVKGGATNPDELELTGGEVRTPGQQDTKPSVPTPSLTEIGDQDMNGCYYNLNSKTRTYLIFDSRSGFYHEFSQGNGNGPMSPDYVNPIAKGWDTGSWPAISPGHAKVLKAALDKVRKGI

SEQ ID NO: 264 - protein, 299 aa, Artificial Sequence
MTFIQARHHGGNSNTPITRLVIHATCPDVGYPSASKAGRAVSTAEYFASTSRSASAHYVCDVSATVQCLSEETIGYHAPPNSHSIGIEICADGGSRASFEKASHAYTREQWLSPQVWPAVERAAILARGICHRHHIPVRKLTTAQVKSGMSGICGHDNVSDAFHQSDHDDPGPYFPWNEFIAAIQGKNTNKGELSGGEVRTPGQQDTKPSVPTPSLTEIGDQDMNGCYYNLNSKTRTYLIFDSRSGFYHEFSQGNGNGPMSPDYVNPIAKGWDTGSWPAISPGHAKVLKAALDKVRKGI

SEQ ID NO: 265 - protein, 297 aa, Artificial Sequence
MTFIQAAHHSSGSNLPPTRVVIHATCPELGFPRASAKGRAVSTARYFQSAISGGSAHYVVDVGETVQCLAEDVIAWHAPPNSRSLGIEICADGGSATSFKNPNVRYSRAQWLSPQVWPAVLRAAALTRQMCQKYGIPVTKLSASDLKAGKKGICGHVDVSNAWHQSDHDDPGPDFPWAEFMAAVKGGATNPDELELTGGPGQQDTKPSVPTPSLTEIGDQDMNGCYYNLNSKTRTYLIFDSRSGFYHEFSQGNGNGPMSPDYVNPIAKGWDTGSWPAISPGHAKVLKAALDKVRKGI

SEQ ID NO: 266 - protein, 304 aa, Artificial Sequence
MTFIQAAHHSSGSNLPPTRVVIHATCPEMGFPKASAKGRAVSTARYFQSASSGGSAHYVVDIGETVQCLGENVIAWHAPPNAHSLGIEICADGGSATSFSNPKVRYTRAQWLSPQVWPAVLRAAALTRKMCSKYGIPVVKLSASDLKAGKKGICGHVDVSNAFHQSDHDDPGPDFPWAEFMAAVKGGTTTQEDEDEMKEAGGEVRTPGQQDTKPSVPTPSLTEIGDQDMNGCYYNLNSKTRTYLIFDSRSGFYHEFSQGNGNGPMSPDYVNPIAKGWDTGSWPAISPGHAKVLKAALDKVRKGI

SEQ ID NO: 267 - protein, 290 aa, Artificial Sequence
MKYIPATHHGGHTNTPFTRIVIHATCPDLGFPHASAGGQAKATARYFQSEQSAGSAHYVCDIAETIQCLPDDVIAWHAPPNRRSIGIEICADGGSRSSFQHPEHAYTRSQWLSPQVWPAVARAAALTRDLCHRHNIPMQQLSVADVKAGKHGICGHNDVSEAFHKSDHDDPGPTFPWDQFIKEVRTGGEVRTPGQQDTKPSVPTPSLTEIGDQDMNGCYYNLNSKTRTYLIFDSRSGFYHEFSQGNGNGPMSPDYVNPIAKGWDTGSWPAISPGHAKVLKAALDKVRKGI

SEQ ID NO: 268 - protein, 317 aa, Artificial Sequence
MRYIPAAHHSAGSNKPVNRVVIHATCPDVGFPSASRKGRAVSTANYFASPSSGGSAHYVCDIGETVQCLSESTIGWHAPPNPHSLGIEICADGGSHASFRVPGHAYTREQWLDPRVWPAVERAAILCRQLCDKHGVPKRKLSVADLKAGKRGVCGHVDVTDAWHQSDHDDPGPWFPWDKFMAVVNGHGGGSSSEELSMADVQALHNQIKQLSAGGEVRTPGQQDTKPSVPTPSLTEIGDQDMNGCYYNLNSKTRTYLIFDSRSGFYHEFSQGNGNGPMSPDYVNPIAKGWDTGSWPAISPGHAKVLKAALDKVRKGI

SEQ ID NO: 269 - protein, 286 aa, Artificial Sequence
MKYIPATHHGGHTNTPFTRIVIHATCPDLGFPHASAGGQAKATARYFQSEQSAGSAHYVCDIAETIQCLPDDVIAWHAPPNRRSIGIEICADGGSRSSFQHPEHAYTRSQWLSPQVWPAVARAAALTRDLCHRHNIPMQQLSVADVKAGKHGICGHNDVSEAFHKSDHDDPGPTFPWDQFIKEVRTGGPGQQDTKPSVPTPSLTEIGDQDMNGCYYNLNSKTRTYLIFDSRSGFYHEFSQGNGNGPMSPDYVNPIAKGWDTGSWPAISPGHAKVLKAALDKVRKGI

SEQ ID NO: 270 - protein, 296 aa, Artificial Sequence
MTFIQARHHGGNSNAPITRLVIHATCPDVGYPSASKAGRAVSTANYFATTDRPASAHYVCDIATTVQCLSEETIGYHAPPNSHSIGIEICADGGSHASFEKASHAYTRDQWLSDDVWPAVERAAILARDICQRHRIPVRKLSTAQVKAGLSGICGHDNVSGAFHQSDHDDPGPYFPWDQFMALVQGKPATPGDLTMGGPGQQDTKPSVPTPSLTEIGDQDMNGCYYNLNSKTRTYLIFDSRSGFYHEFSQGNGNGPMSPDYVNPIAKGWDTGSWPAISPGHAKVLKAALDKVRKGI

SEQ ID NO: 271 - protein, 304 aa, Artificial Sequence
MTFIQAKHHGGHNNPPVTRLVIHATCPDVGYPSASRAGRAVSTAHYFQETTRPASAHYICDISTTVQCLSEETVGYHAPPNSHSIGIEICADGGSHASFSNPAHAYTREQWLSPQVWPAVERAAMLARGICQRHNIPIRRLSIADVKAGKRGICGHNEVSEAFHQSDHDDPGPYFPWDGFIALVNGHSAPSRQEELTVSDGGEVRTPGQQDTKPSVPTPSLTEIGDQDMNGCYYNLNSKTRTYLIFDSRSGFYHEFSQGNGNGPMSPDYVNPIAKGWDTGSWPAISPGHAKVLKAALDKVRKGI

SEQ ID NO: 272 - protein, 300 aa, Artificial Sequence
MTFIQAAHHSSGSNLPPTRVVIHATCPEMGFPKASAKGRAVSTARYFQSASSGGSAHYVVDIGETVQCLGENVIAWHAPPNAHSLGIEICADGGSATSFSNPKVRYTRAQWLSPQVWPAVLRAAALTRKMCSKYGIPVVKLSASDLKAGKKGICGHVDVSNAFHQSDHDDPGPDFPWAEFMAAVKGGTTTQEDEDEMKEAGGPGQQDTKPSVPTPSLTEIGDQDMNGCYYNLNSKTRTYLIFDSRSGFYHEFSQGNGNGPMSPDYVNPIAKGWDTGSWPAISPGHAKVLKAALDKVRKGI

SEQ ID NO: 273 - protein, 300 aa, Artificial Sequence
MTFIQAKHHGGHNNPPVTRLVIHATCPDVGYPSASRAGRAVSTAHYFQETTRPASAHYICDISTTVQCLSEETVGYHAPPNSHSIGIEICADGGSHASFSNPAHAYTREQWLSPQVWPAVERAAMLARGICQRHNIPIRRLSIADVKAGKRGICGHNEVSEAFHQSDHDDPGPYFPWDGFIALVNGHSAPSRQEELTVSDGGPGQQDTKPSVPTPSLTEIGDQDMNGCYYNLNSKTRTYLIFDSRSGFYHEFSQGNGNGPMSPDYVNPIAKGWDTGSWPAISPGHAKVLKAALDKVRKGI

SEQ ID NO: 274 - protein, 259 aa, Artificial Sequence
MTFIQAAHHSSGSNLPPTRVVIHATCPELGFPRASAKGRAVSTARYFQSAISGGSAHYVVDVGETVQCLAEDVIAWHAPPNSRSLGIEICADGGSATSFKNPNVRYSRAQWLSPQVWPAVLRAAALTRQMCQKYGIPVTKLSASDLKAGKKGICGHVDVSNAWHQSDHDDPGPDFPWAEFMAAVKGGVSQFSDLTKRLQGMQEQTHHDLGVVQTKLATMDTVKNPRTGAKWSLKDAIWSIWYYVLENRDRIAALEKKVK

SEQ ID NO: 275 - protein, 265 aa, Artificial Sequence
MTFIQAAHHSSGSNLPPTRVVIHATCPELGFPRASAKGRAVSTARYFQSAISGGSAHYVVDVGETVQCLAEDVIAWHAPPNSRSLGIEICADGGSATSFKNPNVRYSRAQWLSPQVWPAVLRAAALTRQMCQKYGIPVTKLSASDLKAGKKGICGHVDVSNAWHQSDHDDPGPDFPWAEFMAAVKGGDELELTVSQFSDLTKRLQGMQEQTHHDLGVVQTKLATMDTVKNPRTGAKWSLKDAIWSIWYYVLENRDRIAALEKKVK

SEQ ID NO: 276 - protein, 271 aa, Artificial Sequence
MTFIQAAHHSSGSNLPPTRVVIHATCPELGFPRASAKGRAVSTARYFQSAISGGSAHYVVDVGETVQCLAEDVIAWHAPPNSRSLGIEICADGGSATSFKNPNVRYSRAQWLSPQVWPAVLRAAALTRQMCQKYGIPVTKLSASDLKAGKKGICGHVDVSNAWHQSDHDDPGPDFPWAEFMAAVKGGGGATNPDELELTVSQFSDLTKRLQGMQEQTHHDLGVVQTKLATMDTVKNPRTGAKWSLKDAIWSIWYYVLENRDRIAALEKKVK

SEQ ID NO: 277 - protein, 265 aa, Artificial Sequence
MTFIQAAHHSSGSNLPPTRVVIHATCPELGFPRASAKGRAVSTARYFQSAISGGSAHYVVDVGETVQCLAEDVIAWHAPPNSRSLGIEICADGGSATSFKNPNVRYSRAQWLSPQVWPAVLRAAALTRQMCQKYGIPVTKLSASDLKAGKKGICGHVDVSNAWHQSDHDDPGPDFPWAEFMAAVKGGATNPGGVSQFSDLTKRLQGMQEQTHHDLGVVQTKLATMDTVKNPRTGAKWSLKDAIWSIWYYVLENRDRIAALEKKVK

SEQ ID NO: 278 - protein, 271 aa, Artificial Sequence
MTFIQAAHHSSGSNLPPTRVVIHATCPELGFPRASAKGRAVSTARYFQSAISGGSAHYVVDVGETVQCLAEDVIAWHAPPNSRSLGIEICADGGSATSFKNPNVRYSRAQWLSPQVWPAVLRAAALTRQMCQKYGIPVTKLSASDLKAGKKGICGHVDVSNAWHQSDHDDPGPDFPWAEFMAAVKGGATNPGGDELELTVSQFSDLTKRLQGMQEQTHHDLGVVQTKLATMDTVKNPRTGAKWSLKDAIWSIWYYVLENRDRIAALEKKVK

SEQ ID NO: 279 - protein, 277 aa, Artificial Sequence
MTFIQAAHHSSGSNLPPTRVVIHATCPELGFPRASAKGRAVSTARYFQSAISGGSAHYVVDVGETVQCLAEDVIAWHAPPNSRSLGIEICADGGSATSFKNPNVRYSRAQWLSPQVWPAVLRAAALTRQMCQKYGIPVTKLSASDLKAGKKGICGHVDVSNAWHQSDHDDPGPDFPWAEFMAAVKGGATNPGGGGATNPDELELTVSQFSDLTKRLQGMQEQTHHDLGVVQTKLATMDTVKNPRTGAKWSLKDAIWSIWYYVLENRDRIAALEKKVK

SEQ ID NO: 280 - protein, 271 aa, Artificial Sequence
MTFIQAAHHSSGSNLPPTRVVIHATCPELGFPRASAKGRAVSTARYFQSAISGGSAHYVVDVGETVQCLAEDVIAWHAPPNSRSLGIEICADGGSATSFKNPNVRYSRAQWLSPQVWPAVLRAAALTRQMCQKYGIPVTKLSASDLKAGKKGICGHVDVSNAWHQSDHDDPGPDFPWAEFMAAVKGGATNPDELELTGGVSQFSDLTKRLQGMQEQTHHDLGVVQTKLATMDTVKNPRTGAKWSLKDAIWSIWYYVLENRDRIAALEKKVK

SEQ ID NO: 281 - protein, 277 aa, Artificial Sequence
MTFIQAAHHSSGSNLPPTRVVIHATCPELGFPRASAKGRAVSTARYFQSAISGGSAHYVVDVGETVQCLAEDVIAWHAPPNSRSLGIEICADGGSATSFKNPNVRYSRAQWLSPQVWPAVLRAAALTRQMCQKYGIPVTKLSASDLKAGKKGICGHVDVSNAWHQSDHDDPGPDFPWAEFMAAVKGGATNPDELELTGGDELELTVSQFSDLTKRLQGMQEQTHHDLGVVQTKLATMDTVKNPRTGAKWSLKDAIWSIWYYVLENRDRIAALEKKVK

SEQ ID NO: 282 - protein, 283 aa, Artificial Sequence
MTFIQAAHHSSGSNLPPTRVVIHATCPELGFPRASAKGRAVSTARYFQSAISGGSAHYVVDVGETVQCLAEDVIAWHAPPNSRSLGIEICADGGSATSFKNPNVRYSRAQWLSPQVWPAVLRAAALTRQMCQKYGIPVTKLSASDLKAGKKGICGHVDVSNAWHQSDHDDPGPDFPWAEFMAAVKGGATNPDELELTGGGGATNPDELELTVSQFSDLTKRLQGMQEQTHHDLGVVQTKLATMDTVKNPRTGAKWSLKDAIWSIWYYVLENRDRIAALEKKVK

SEQ ID NO: 284 - DNA, 933 bp, Artificial Sequence
atgacgttcattcaggccgcgcatcacagcagcggctccaatctgccgcccacgagggtggtgatccacgcgacatgccccgaactcggcttcccgagggccagtgcgaagggccgagctgtctcgacagcccgctacttccagtctgcgatctcgggcggctcggcgcactatgttgtcgatgtcggcgaaaccgtgcagtgtctggcagaggatgtgatcgcctggcacgccccgcccaacagccgcagcctggggatcgagatctgcgctgacggcggctcggcgaccagcttcaagaaccccaacgtgcgctacagccgcgcccagtggctcagcccgcaggtctggcccgccgtgctccgtgccgcagcactcacccggcagatgtgccagaagtacggcataccggtcaccaagctcagcgcgtcggacctcaaggccgggaagaagggcatctgcggacacgtcgatgtcagcaatgcgtggcatcagtccgaccacgacgaccccggcccggacttcccctgggccgaattcatggcagccgtcaaaggcggcgccaccaaccccgatgaactggagctcacaggcggtacattcccgtgggaccaattcatcaaagaggttagaacaccaggacaacaagatacgaaaccttccgtaccaacaccatcactcacagaaataggagatcaggacatgaacgggtgctactacaacctcaattcgaaaacacggacgtaccttatcttcgatagccgttccggattttaccacgaattctcccaaggcaatgggaacggccccatgagcccagactatgtaaatccgatcgccaaaggatgggacaccggatcatggccggcaatctccccaggccacgcgaaagtgctcaaggccgccctcgataaagtccggaaaggaatctga

SEQ ID NO: 284 - DNA, 924 bp, Artificial Sequence
atgacgttcattcaggccgcgcatcacagcagcggctccaatctgccgcccacgagggtggtgatccacgcgacatgccccgaactcggcttcccgagggccagtgcgaagggccgagctgtctcgacagcccgctacttccagtctgcgatctcgggcggctcggcgcactatgttgtcgatgtcggcgaaaccgtgcagtgtctggcagaggatgtgatcgcctggcacgccccgcccaacagccgcagcctggggatcgagatctgcgctgacggcggctcggcgaccagcttcaagaaccccaacgtgcgctacagccgcgcccagtggctcagcccgcaggtctggcccgccgtgctccgtgccgcagcactcacccggcagatgtgccagaagtacggcataccggtcaccaagctcagcgcgtcggacctcaaggccgggaagaagggcatctgcggacacgtcgatgtcagcaatgcgtggcatcagtccgaccacgacgaccccggcccggacttcccctgggccgaattcatggcagccgtcaaaggcggcgccaccaaccccgatgaactggagctcacaggcggttacttcccgtgggaccagttcatggcactcgtccaaggaaaacccgccacaccaggagatctcaccatggcagacatcagcaaactcaccgacgcgatcaaggcatccaaccggcagctgcaccacgacatcggcgtagtacagacccaaaacggaaaattacgtgagcagatcgaaaggatcacctgggtcaaaaatccggtgacaggaaagaagtggcgcatcaccgacgcgctgtggtcgatctggcactacgtgctggaatgccgcacccgcatccagcggctcgacgcccgtctgtctgaggtcgagaagaaggtgaagtga

SEQ ID NO: 285 - DNA, 942 bp, Artificial Sequence
atgacgttcattcaggccgcgcatcacagcagcggctccaatctgccacccacgagggtggtgatccatgcgacatgccccgagatgggattcccgaaggccagtgcgaagggcagggctgtctcgacggcccgatacttccagtctgcgagctcgggcggtagcgcccactatgttgtcgacatcggcgagacggtgcagtgtctcggtgagaacgtgatcgcgtggcacgccccgcccaatgcccacagtctcggcatcgagatctgcgcggacgggggatcggccacctccttctccaatcccaaggtgcgctacacgcgggcgcagtggctgagcccgcaggtgtggcccgccgtgctccgtgccgcagcactcacccggaagatgtgcagcaagtacggcatccccgtcgtcaagctgtccgcgtcggacctcaaggccggaaagaagggcatctgcggccacgtggatgtcagcaatgctttccaccagtccgaccacgacgaccccggccccgacttcccgtgggccgaattcatggcagccgtcaaaggcggcaccaccacacaggaagatgaggatgaaatgaaggaagctggcggtacattcccgtgggaccaattcatcaaagaggttagaacaccaggacaacaagatacgaaaccttccgtaccaacaccatcactcacagaaataggagatcaggacatgaacgggtgctactacaacctcaattcgaaaacacggacgtaccttatcttcgatagccgttccggattttaccacgaattctcccaaggcaatgggaacggccccatgagcccagactatgtaaatccgatcgccaaaggatgggacaccggatcatggccggcaatctccccaggccacgcgaaagtgctcaaggccgccctcgataaagtccggaaaggaatctga

SEQ ID NO: 286 - DNA, 897 bp, Artificial Sequence
atgacgttcattcaggccgcgcatcacagcagcggctccaatctgccgcccacgagggtggtgatccacgcgacatgccccgaactcggcttcccgagggccagtgcgaagggccgagctgtctcgacagcccgctacttccagtctgcgatctcgggcggctcggcgcactatgttgtcgatgtcggcgaaaccgtgcagtgtctggcagaggatgtgatcgcctggcacgccccgcccaacagccgcagcctggggatcgagatctgcgctgacggcggctcggcgaccagcttcaagaaccccaacgtgcgctacagccgcgcccagtggctcagcccgcaggtctggcccgccgtgctccgtgccgcagcactcacccggcagatgtgccagaagtacggcataccggtcaccaagctcagcgcgtcggacctcaaggccgggaagaagggcatctgcggacacgtcgatgtcagcaatgcgtggcatcagtccgaccacgacgaccccggcccggacttcccctgggccgaattcatggcagccgtcaaaggcggcgccaccaaccccgatgaactggagctcacaggcggtggcagtggagagagtggagagttgagtatggctgatgtgaaagccttgcatgatcagattaaacagttgtcggggcaggtggcccagtcggtgaataagctgcatcacgatgtgggtgtggttcaggttcagaatgggaatcttaaaaagcaggttgattccctgtctatggtgaagaatcctgtgacggggaagctgtggcgtaccagggatgcgatctggtcgatctggtattacgtgttggagtgtcgtagccgtatcggcaagttggaggccgaggtggcccggttgaagaagtga

SEQ ID NO: 287 - DNA, 885 bp, Artificial Sequence
atgacgttcattcaggccgcgcatcacagcagcggctccaatctgccgcccacgagggtggtgatccacgcgacatgccccgaactcggcttcccgagggccagtgcgaagggccgagctgtctcgacagcccgctacttccagtctgcgatctcgggcggctcggcgcactatgttgtcgatgtcggcgaaaccgtgcagtgtctggcagaggatgtgatcgcctggcacgccccgcccaacagccgcagcctggggatcgagatctgcgctgacggcggctcggcgaccagcttcaagaaccccaacgtgcgctacagccgcgcccagtggctcagcccgcaggtctggcccgccgtgctccgtgccgcagcactcacccggcagatgtgccagaagtacggcataccggtcaccaagctcagcgcgtcggacctcaaggccgggaagaagggcatctgcggacacgtcgatgtcagcaatgcgtggcatcagtccgaccacgacgaccccggcccggacttcccctgggccgaattcatggcagccgtcaaaggcggcgccaccaaccccgatgaactggagctcacaggcggtaaaaacaccaacaagggagaactcagcatgtccgacgtcaacaccctgaccaagctcatcaaggccagcaacaatcagctccaccacgacattggcgtcgtccagacacagaacggcaccctcaaaagcaagatcgacaacttgtcgtgggtgaagaatcccgtcaccggcaagaagtggtccaccaaggatgcgctgtggtctgtctggtactacgtgctggaatgccgcaaccgcatccaggctatcgaaaaccgcctctctgacatcgaaaagaaggtgaagtga

SEQ ID NO: 288 - DNA, 927 bp, Artificial Sequence
atgacattcatccaggcccgccatcacggcggcaactccaacacgccgatcacccggctggtcatccacgccacctgccccgacgtgggctacccgtcggcgtcgaaggccggtagggcagtctccacggcggagtatttcgcgtccacgtcgcggtctgcctcggctcactacgtctgtgacgtatcggcaacggtgcagtgcctctccgaggaaaccatcggctaccacgcgccgcccaacagtcattccatcggcattgagatttgcgccgacggcgggtcccgcgcctcatttgagaaggcttctcacgcatacacccgcgagcaatggctctcgcctcaagtgtggcccgccgtggagcgcgccgccattctcgcccgcggcatctgccaccgccaccacatcccggttcgcaaactcaccaccgcacaggtcaaatcggggatgtcgggtatttgcggacacgacaacgtatccgatgcattccaccaatccgaccacgacgaccctggcccctacttcccgtggaacgaatttatcgccgccatccaaggaaaaaacaccaacaagggagaactcagcggcggtacattcccgtgggaccaattcatcaaagaggttagaacaccaggacaacaagatacgaaaccttccgtaccaacaccatcactcacagaaataggagatcaggacatgaacgggtgctactacaacctcaattcgaaaacacggacgtaccttatcttcgatagccgttccggattttaccacgaattctcccaaggcaatgggaacggccccatgagcccagactatgtaaatccgatcgccaaaggatgggacaccggatcatggccggcaatctccccaggccacgcgaaagtgctcaaggccgccctcgataaagtccggaaaggaatctga

SEQ ID NO: 289 - DNA, 930 bp, Artificial Sequence
atgacattcatccaggcccgccaccacggcggcaactccaacgcgccgatcacccggctggtcatccacgccacctgccccgacgtgggctacccgtcggcatcgaaggccggtagggcagtctcgaccgcgaactacttcgccacgactgatcggcccgcctcggcacattacgtatgtgacatcgccactacagtgcagtgcctctccgaggaaaccatcggctaccacgcgccgccgaactcgcattccatcggcattgaaatttgcgccgatggcgggtcgcacgcctcatttgagaaggcttctcacgcatacacccgcgaccaatggttgagcgatgacgtgtggcccgccgtagagcgcgccgccattcttgcccgcgatatttgccaacgacaccgcatcccggttcgtaaactctccaccgcacaggtgaaagccggactgtcgggaatttgcggacacgacaatgtatccggcgcattccatcagtccgaccacgacgacccgggcccctacttcccgtgggaccagttcatggcactcgtccaaggaaaacccgccacaccaggagatctcaccatgggcggtacattcccgtgggaccaattcatcaaagaggttagaacaccaggacaacaagatacgaaaccttccgtaccaacaccatcactcacagaaataggagatcaggacatgaacgggtgctactacaacctcaattcgaaaacacggacgtaccttatcttcgatagccgttccggattttaccacgaattctcccaaggcaatgggaacggccccatgagcccagactatgtaaatccgatcgccaaaggatgggacaccggatcatggccggcaatctccccaggccacgcgaaagtgctcaaggccgccctcgataaagtccggaaaggaatctga

SEQ ID NO: 290 - DNA, 942 bp, Artificial Sequence
atgacattcattcaggccaagcatcacggcggccacaacaaccctcccgtgactcgtcttgtcattcacgccacatgcccggatgtgggctatccgtctgcgtcgcgcgctggccgtgcggtgtcgacggcccactattttcaggaaacgacccggccagcatccgcccactacatttgtgacatatcgaccacggtgcagtgtctgtctgaggagacggtgggctatcacgccccgccgaactcacactccatcggtattgagatatgcgctgacggtgggtcgcatgcctcgttttcgaaccctgcccacgcctacacccgcgagcagtggttgagccctcaggtgtggcctgctgtggagcgtgccgcgatgctggcgcgcggtatctgtcaacgccacaacatcccgatccgccgcctctcgatcgctgacgtcaaggccgggaagcgcggcatctgcggccacaacgaggtgtccgaggccttccaccaatccgaccatgacgaccccggtccttatttcccgtgggacgggtttatcgcgcttgttaatggccattccgcaccatcacgccaggaggaactaactgtgtcagatggcggtacattcccgtgggaccaattcatcaaagaggttagaacaccaggacaacaagatacgaaaccttccgtaccaacaccatcactcacagaaataggagatcaggacatgaacgggtgctactacaacctcaattcgaaaacacggacgtaccttatcttcgatagccgttccggattttaccacgaattctcccaaggcaatgggaacggccccatgagcccagactatgtaaatccgatcgccaaaggatgggacaccggatcatggccggcaatctccccaggccacgcgaaagtgctcaaggccgccctcgataaagtccggaaaggaatctga

SEQ ID NO: 291 - DNA, 951 bp, Artificial Sequence
atgacgttcattcaggccgcgcatcacagcagcggctccaatctgccacccacgagggtggtgatccatgcgacatgccccgagatgggattcccgaaggccagtgcgaagggcagggctgtctcgacggcccgatacttccagtctgcgagctcgggcggtagcgcccactatgttgtcgacatcggcgagacggtgcagtgtctcggtgagaacgtgatcgcgtggcacgccccgcccaatgcccacagtctcggcatcgagatctgcgcggacgggggatcggccacctccttctccaatcccaaggtgcgctacacgcgggcgcagtggctgagcccgcaggtgtggcccgccgtgctccgtgccgcagcactcacccggaagatgtgcagcaagtacggcatccccgtcgtcaagctgtccgcgtcggacctcaaggccggaaagaagggcatctgcggccacgtggatgtcagcaatgctttccaccagtccgaccacgacgaccccggccccgacttcccgtgggccgaattcatggcagccgtcaaaggcggcaccaccacacaggaagatgaggatgaaatgaaggaagctggcggttggtttccgtgggacaaatttatggctgtggtgaatggccacggcggcggttcaagtagtgaggagttgagtatggctgatgtacaagcgttacataatcagattaaacagttgtcggcacaggtggcccagtcggtgaataagctgcatcacgatgttggtgtggttcaggttcagaatggtgatttgggtaaacgtgttgatgccttgtcgtgggtgaagaatccggtgacggggaagctgtggcgcagcaaggatgctttgtggagtgtctggtattacgtgttggagtgtcgtagccgtcttgacaggctcgagtctgctgtcaacgatttgaaaaagtga

SEQ ID NO: 292 - DNA, 939 bp, Artificial Sequence
atgacgttcattcaggccgcgcatcacagcagcggctccaatctgccacccacgagggtggtgatccatgcgacatgccccgagatgggattcccgaaggccagtgcgaagggcagggctgtctcgacggcccgatacttccagtctgcgagctcgggcggtagcgcccactatgttgtcgacatcggcgagacggtgcagtgtctcggtgagaacgtgatcgcgtggcacgccccgcccaatgcccacagtctcggcatcgagatctgcgcggacgggggatcggccacctccttctccaatcccaaggtgcgctacacgcgggcgcagtggctgagcccgcaggtgtggcccgccgtgctccgtgccgcagcactcacccggaagatgtgcagcaagtacggcatccccgtcgtcaagctgtccgcgtcggacctcaaggccggaaagaagggcatctgcggccacgtggatgtcagcaatgctttccaccagtccgaccacgacgaccccggccccgacttcccgtgggccgaattcatggcagccgtcaaaggcggcaccaccacacaggaagatgaggatgaaatgaaggaagctggcggttatttcccgtgggacgggtttatcgcgcttgttaatggccattccgcaccatcacgccaggaggaactaactgtgtcagatgtcaatatgctcaaaggtcttattcagcaatcgaacaagcagctgcaccacgatatcggtgttgtgcagacgcaggcgggtaacctccgccgccagctggaatccctgtcatgggtgaagaacccggtcagcggcaagctgtggcgcaccaaggacgccttgtggtcgatctggtactacgtgctggactgccgatctcgtctcggcaaactcgaggcccgcctgtcgacgctggaaaagaaggtgaagtga

SEQ ID NO: 293 - DNA, 942 bp, Artificial Sequence
atgacgttcattcaggccgcgcatcacagcagcggctccaatctgccgcccacgagggtggtgatccacgcgacatgccccgaactcggcttcccgagggccagtgcgaagggccgagctgtctcgacagcccgctacttccagtctgcgatctcgggcggctcggcgcactatgttgtcgatgtcggcgaaaccgtgcagtgtctggcagaggatgtgatcgcctggcacgccccgcccaacagccgcagcctggggatcgagatctgcgctgacggcggctcggcgaccagcttcaagaaccccaacgtgcgctacagccgcgcccagtggctcagcccgcaggtctggcccgccgtgctccgtgccgcagcactcacccggcagatgtgccagaagtacggcataccggtcaccaagctcagcgcgtcggacctcaaggccgggaagaagggcatctgcggacacgtcgatgtcagcaatgcgtggcatcagtccgaccacgacgaccccggcccggacttcccctgggccgaattcatggcagccgtcaaaggcggcgccaccaaccccgatgaactggagctcacaggcggttggtttccgtgggacaaatttatggctgtggtgaatggccacggcggcggttcaagtagtgaggagttgagtatggctgatgtacaagcgttacataatcagattaaacagttgtcggcacaggtggcccagtcggtgaataagctgcatcacgatgttggtgtggttcaggttcagaatggtgatttgggtaaacgtgttgatgccttgtcgtgggtgaagaatccggtgacggggaagctgtggcgcagcaaggatgctttgtggagtgtctggtattacgtgttggagtgtcgtagccgtcttgacaggctcgagtctgctgtcaacgatttgaaaaagtga

SEQ ID NO: 294 - DNA, 927 bp, Artificial Sequence
atgagatacattcctgcggcgcatcactcggccggctctaatagtccggtgaacagggttgtgattcatgcaacatgcccggatgtggggtttccgtccgcttcccgtaaaggacgggcggtgtccacggcaaactatttcgcgtccccatcggcgggcggttctgcccattatgtgtgtgatgttggggagacggtgcagtgcttgtcggagtctacgattggttggcatgccccgccgaatccgcatagtttgggtatagagatttgcgcggatgggggttcgcacgcctcgttccgtgtgccggggcatgcttacactcgtgagcagtggcttgatccgagggtgtggcctgcggtggagaaggcggctgtgctgtgtagacagttgtgtgacaaatataatgttccgaagaggaaactgtctgtatccgatttgaaggctggcaggcggggtgtgtgcggccatacggatgtgacggatgcgtggcatcagtcggatcatgatgatccggggccgtggtttccgtgggacaggtttatggccgtcgtcaacggcggcagtggagagagtggagagttgagtggcggtacattcccgtgggaccaattcatcaaagaggttagaacaccaggacaacaagatacgaaaccttccgtaccaacaccatcactcacagaaataggagatcaggacatgaacgggtgctactacaacctcaattcgaaaacacggacgtaccttatcttcgatagccgttccggattttaccacgaattctcccaaggcaatgggaacggccccatgagcccagactatgtaaatccgatcgccaaaggatgggacaccggatcatggccggcaatctccccaggccacgcgaaagtgctcaaggccgccctcgataaagtccggaaaggaatctga

SEQ ID NO: 295 - DNA, 921 bp, Artificial Sequence
atgacattcatccaggccgcccaccgtggcggcacttccaacacgccgatcacccggctggtcatccacgccacctgccccgatgtcggcttcccgtcggcatcgcgggcaggacgagcagtatccacagcggaatatttcgcgtccacgtcgaggtcagcctcggcgcactacgtatgcgacatctctaccacggtgcagtgcctgtccgaggcaacgatcggctatcacgcgccaccaaacgcccactccatcggcattgaaatctgcgccgacggaggctcgcgcgcttcatttgagaaggcttctcacgcatacacccgcgagcaatggctcagcccgcaggtatggcccgccgtggagcgcgccgcgattctcgcccgcgacatctgccaccgacaccacatccccatccgccgcctctccgtcgcgcaggtgcgggcaggtgagcgcggaatctgcggccacaacgaggtgagcgaggcgttccaccaatccgaccacgacgaccccggcccctatttcccttggaatgaatttattgccgccgtccaaggaaaaaccaccacaccagagggaggcggtacattcccgtgggaccaattcatcaaagaggttagaacaccaggacaacaagatacgaaaccttccgtaccaacaccatcactcacagaaataggagatcaggacatgaacgggtgctactacaacctcaattcgaaaacacggacgtaccttatcttcgatagccgttccggattttaccacgaattctcccaaggcaatgggaacggccccatgagcccagactatgtaaatccgatcgccaaaggatgggacaccggatcatggccggcaatctccccaggccacgcgaaagtgctcaaggccgccctcgataaagtccggaaaggaatctga

SEQ ID NO: 296 - DNA, 873 bp, Artificial Sequence
atgacattcatccaggccgcccaccgtggcggcacttccaacacgccgatcacccggctggtcatccacgccacctgccccgatgtcggcttcccgtcggcatcgcgggcaggacgagcagtatccacagcggaatatttcgcgtccacgtcgaggtcagcctcggcgcactacgtatgcgacatctctaccacggtgcagtgcctgtccgaggcaacgatcggctatcacgcgccaccaaacgcccactccatcggcattgaaatctgcgccgacggaggctcgcgcgcttcatttgagaaggcttctcacgcatacacccgcgagcaatggctcagcccgcaggtatggcccgccgtggagcgcgccgcgattctcgcccgcgacatctgccaccgacaccacatccccatccgccgcctctccgtcgcgcaggtgcgggcaggtgagcgcggaatctgcggccacaacgaggtgagcgaggcgttccaccaatccgaccacgacgaccccggcccctatttcccttggaatgaatttattgccgccgtccaaggaaaaaccaccacaccagagggaggcggtaaaaacaccaacaagggagaactcagcatgtccgacgtcaacaccctgaccaagctcatcaaggccagcaacaatcagctccaccacgacattggcgtcgtccagacacagaacggcaccctcaaaagcaagatcgacaacttgtcgtgggtgaagaatcccgtcaccggcaagaagtggtccaccaaggatgcgctgtggtctgtctggtactacgtgctggaatgccgcaaccgcatccaggctatcgaaaaccgcctctctgacatcgaaaagaaggtgaagtga

SEQ ID NO: 297 - DNA, 933 bp, Artificial Sequence
atgagatacattcctgcggcgcatcattctgccggatcaaataagccggtgaaccgggttgtgattcatgcaacatgcccggatgtggggtttccgtctgcttcgcgtaagggtcgggcggtgtctacagcaaactattttgcttccccatcgtctggtggttcggcgcattatgtgtgtgatattggggagacggtgcagtgcttgtcggagtctacgattggttggcatgccccgccgaatccgcatagtttgggtatagagatttgcgcggatgggggttcgcacgcctcattccgtgttccagggcatgcctatacgcgggagcagtggcttgaccctcgggtgtggcccgcggtggagagggccgccatcctgtgtcggcagttgtgtgataagcatggtgttccgaagaggaaactgtctgtggctgatttgaaggccggtaaacggggtgtttgcgggcatgtggatgttacggatgcgtggcatcagtcggatcatgacgatccggggccgtggtttccgtgggacaaatttatggctgtggtgaatggccacggcggcggttcaagtagtgaggagttgagtatggctgatgtacaagcgttacataatcagattaaacagttgtcggcaggcggtaaaaacaccaacaagggagaactcagcatgtccgacgtcaacaccctgaccaagctcatcaaggccagcaacaatcagctccaccacgacattggcgtcgtccagacacagaacggcaccctcaaaagcaagatcgacaacttgtcgtgggtgaagaatcccgtcaccggcaagaagtggtccaccaaggatgcgctgtggtctgtctggtactacgtgctggaatgccgcaaccgcatccaggctatcgaaaaccgcctctctgacatcgaaaagaaggtgaagtga

SEQ ID NO: 298 - DNA, 882 bp, Artificial Sequence
atgacattcatccaggcccgccaccacggcggcaactccaacgcgccgatcacccggctggtcatccacgccacctgccccgacgtgggctacccgtcggcatcgaaggccggtagggcagtctcgaccgcgaactacttcgccacgactgatcggcccgcctcggcacattacgtatgtgacatcgccactacagtgcagtgcctctccgaggaaaccatcggctaccacgcgccgccgaactcgcattccatcggcattgaaatttgcgccgatggcgggtcgcacgcctcatttgagaaggcttctcacgcatacacccgcgaccaatggttgagcgatgacgtgtggcccgccgtagagcgcgccgccattcttgcccgcgatatttgccaacgacaccgcatcccggttcgtaaactctccaccgcacaggtgaaagccggactgtcgggaatttgcggacacgacaatgtatccggcgcattccatcagtccgaccacgacgacccgggcccctacttcccgtgggaccagttcatggcactcgtccaaggaaaacccgccacaccaggagatctcaccatgggcggtaaaaacaccaacaagggagaactcagcatgtccgacgtcaacaccctgaccaagctcatcaaggccagcaacaatcagctccaccacgacattggcgtcgtccagacacagaacggcaccctcaaaagcaagatcgacaacttgtcgtgggtgaagaatcccgtcaccggcaagaagtggtccaccaaggatgcgctgtggtctgtctggtactacgtgctggaatgccgcaaccgcatccaggctatcgaaaaccgcctctctgacatcgaaaagaaggtgaagtga

SEQ ID NO: 299 - DNA, 870 bp, Artificial Sequence
atggcctatccctatatcggggcattgaagcatggcggcaagcagggcaagatccagcggatcgtcatccatgccacggtttcgccctgtgtgcggggcggtgcccggaacgtcgcgaagtactttcagagttcagccgccggaggcagcgcccactacgtggtggatcccggtgagatcatccagtgtgtcaaggacgacgtggtggcctaccacgcgccgcccaacaccggaacgctcgggatcgagctgtgcgacccgcaggccggatcgccgaagcggtggagcaacgaggcccaccaggcgatgctcgtgctcgccgcgaagctcgtcagggaactcgcggcgaagcacgacgtgccgctcgtccgggtgaccgccgcgcagctcagggcgggcaagcgcggcatctgctcgcatgtcgcggtcagcgacgcgttcgggcagtccgaccacggcgatcccgaggtcgccgggccgttcccctgggcgaagttcatgcagctcatcaaggaggaggacgacatgggcggtacattcccgtgggaccaattcatcaaagaggttagaacaccaggacaacaagatacgaaaccttccgtaccaacaccatcactcacagaaataggagatcaggacatgaacgggtgctactacaacctcaattcgaaaacacggacgtaccttatcttcgatagccgttccggattttaccacgaattctcccaaggcaatgggaacggccccatgagcccagactatgtaaatccgatcgccaaaggatgggacaccggatcatggccggcaatctccccaggccacgcgaaagtgctcaaggccgccctcgataaagtccggaaaggaatctga

SEQ ID NO: 300 - DNA, 936 bp, Artificial Sequence
atgacgttcattcaggccgcgcatcacagcagcggctccaatctgccacccacgagggtggtgatccatgcgacatgccccgagatgggattcccgaaggccagtgcgaagggcagggctgtctcgacggcccgatacttccagtctgcgagctcgggcggtagcgcccactatgttgtcgacatcggcgagacggtgcagtgtctcggtgagaacgtgatcgcgtggcacgccccgcccaatgcccacagtctcggcatcgagatctgcgcggacgggggatcggccacctccttctccaatcccaaggtgcgctacacgcgggcgcagtggctgagcccgcaggtgtggcccgccgtgctccgtgccgcagcactcacccggaagatgtgcagcaagtacggcatccccgtcgtcaagctgtccgcgtcggacctcaaggccggaaagaagggcatctgcggccacgtggatgtcagcaatgctttccaccagtccgaccacgacgaccccggccccgacttcccgtgggccgaattcatggcagccgtcaaaggcggcaccaccacacaggaagatgaggatgaaatgaaggaagctggcggttatttcccttggaatgaatttattgccgccgtccaaggaaaaaccaccacaccagagggagaactcagcatgtcagacgtaaacaccctgaccaagctcatcaaggccagcaacgaccagcttcactacgatattggcgtcgtccagacgcaaaacgggaacatcaagaagaagatcgacaatctgtcgtgggtgaagaaccccgtcaccggcaagaagtggtccactaaggatgccctgtggtccgtctggtattacgtgctggaatgccgcaaccgcatccaggctatcgagaaccgtatttacgaccttgagaagaaggtgaagtga

SEQ ID NO: 301 - DNA, 933 bp, Artificial Sequence
atgacgttcattcaggccgcgcatcacagcagcggctccaatctgccacccacgagggtggtgatccatgcgacatgccccgagatgggattcccgaaggccagtgcgaagggcagggctgtctcgacggcccgatacttccagtctgcgagctcgggcggtagcgcccactatgttgtcgacatcggcgagacggtgcagtgtctcggtgagaacgtgatcgcgtggcacgccccgcccaatgcccacagtctcggcatcgagatctgcgcggacgggggatcggccacctccttctccaatcccaaggtgcgctacacgcgggcgcagtggctgagcccgcaggtgtggcccgccgtgctccgtgccgcagcactcacccggaagatgtgcagcaagtacggcatccccgtcgtcaagctgtccgcgtcggacctcaaggccggaaagaagggcatctgcggccacgtggatgtcagcaatgctttccaccagtccgaccacgacgaccccggccccgacttcccgtgggccgaattcatggcagccgtcaaaggcggcaccaccacacaggaagatgaggatgaaatgaaggaagctggcggttacttcccgtgggaccagttcatggcactcgtccaaggaaaacccgccacaccaggagatctcaccatggcagacatcagcaaactcaccgacgcgatcaaggcatccaaccggcagctgcaccacgacatcggcgtagtacagacccaaaacggaaaattacgtgagcagatcgaaaggatcacctgggtcaaaaatccggtgacaggaaagaagtggcgcatcaccgacgcgctgtggtcgatctggcactacgtgctggaatgccgcacccgcatccagcggctcgacgcccgtctgtctgaggtcgagaagaaggtgaagtga

SEQ ID NO: 302 - DNA, 981 bp, Artificial Sequence
atgagatacattcctgcggcgcatcattctgccggatcaaataagccggtgaaccgggttgtgattcatgcaacatgcccggatgtggggtttccgtctgcttcgcgtaagggtcgggcggtgtctacagcaaactattttgcttccccatcgtctggtggttcggcgcattatgtgtgtgatattggggagacggtgcagtgcttgtcggagtctacgattggttggcatgccccgccgaatccgcatagtttgggtatagagatttgcgcggatgggggttcgcacgcctcattccgtgttccagggcatgcctatacgcgggagcagtggcttgaccctcgggtgtggcccgcggtggagagggccgccatcctgtgtcggcagttgtgtgataagcatggtgttccgaagaggaaactgtctgtggctgatttgaaggccggtaaacggggtgtttgcgggcatgtggatgttacggatgcgtggcatcagtcggatcatgacgatccggggccgtggtttccgtgggacaaatttatggctgtggtgaatggccacggcggcggttcaagtagtgaggagttgagtatggctgatgtacaagcgttacataatcagattaaacagttgtcggcaggcggtacattcccgtgggaccaattcatcaaagaggttagaacaccaggacaacaagatacgaaaccttccgtaccaacaccatcactcacagaaataggagatcaggacatgaacgggtgctactacaacctcaattcgaaaacacggacgtaccttatcttcgatagccgttccggattttaccacgaattctcccaaggcaatgggaacggccccatgagcccagactatgtaaatccgatcgccaaaggatgggacaccggatcatggccggcaatctccccaggccacgcgaaagtgctcaaggccgccctcgataaagtccggaaaggaatctga

SEQ ID NO: 303 - DNA, 909 bp, Artificial Sequence
atgaaatacattcccgcgacacatcacggaggccacacgaacacccccttcacccggatcgtgatccacgccacctgccccgaccttggcttcccccacgcatcagctggtggacaggcaaaagccaccgcacgctatttccaatcagagcagtctgccggatcagcacactatgtgtgcgacatcgccgagactatccaatgcctgcccgatgacgtgatcgcctggcacgccccaccaaacagaaggtcgatcggaatcgaaatatgtgccgacggcggctcccgctcctcattccagcaccccgagcacgcctacaccagatcccaatggctcagcccccaagtgtggcccgccgtcgcccgtgccgccgcgctcacccgcgacctctgccaccgccacaacattccgatgcaacaactctccgttgctgatgtgaaagccgggaagcacggaatctgcggccacaacgacgtatccgaggcattccacaagtccgaccatgacgaccccggccccacattcccgtgggaccaattcatcaaagaggttagaacaggcggttggtttccgtgggacaaatttatggctgtggtgaatggccacggcggcggttcaagtagtgaggagttgagtatggctgatgtacaagcgttacataatcagattaaacagttgtcggcacaggtggcccagtcggtgaataagctgcatcacgatgttggtgtggttcaggttcagaatggtgatttgggtaaacgtgttgatgccttgtcgtgggtgaagaatccggtgacggggaagctgtggcgcagcaaggatgctttgtggagtgtctggtattacgtgttggagtgtcgtagccgtcttgacaggctcgagtctgctgtcaacgatttgaaaaagtga

SEQ ID NO: 304 - DNA, 912 bp, Artificial Sequence
atgacgttcattcaggccgcgcatcacagcagcggctccaatctgccacccacgagggtggtgatccatgcgacatgccccgagatgggattcccgaaggccagtgcgaagggcagggctgtctcgacggcccgatacttccagtctgcgagctcgggcggtagcgcccactatgttgtcgacatcggcgagacggtgcagtgtctcggtgagaacgtgatcgcgtggcacgccccgcccaatgcccacagtctcggcatcgagatctgcgcggacgggggatcggccacctccttctccaatcccaaggtgcgctacacgcgggcgcagtggctgagcccgcaggtgtggcccgccgtgctccgtgccgcagcactcacccggaagatgtgcagcaagtacggcatccccgtcgtcaagctgtccgcgtcggacctcaaggccggaaagaagggcatctgcggccacgtggatgtcagcaatgctttccaccagtccgaccacgacgaccccggccccgacttcccgtgggccgaattcatggcagccgtcaaaggcggcaccaccacacaggaagatgaggatgaaatgaaggaagctggcggtaacggcggtagtggagatagtggggagttaactgtggctgatgtgaaagccttgcatgatcagattaaacaattgtctgctcagcttactggttcggtgaataagctgcaccatgatgttggtgtggtacaggtacagaatggtgatttgggtaaacgtgttgatgccttgtcgtgggtgaagaatccggtgacggggaagctgtggcgcaccaaagacgctttgtggagtgtctggtattacgtgctggagtgtcgcagccgcatagacaggctcgagtctgctgttaacggtttgaaaaagtga

SEQ ID NO: 305 - DNA, 927 bp, Artificial Sequence
atgacgttcattcaggccgcgcatcacagcagcggctccaatctgccgcccacgagggtggtgatccacgcgacatgccccgaactcggcttcccgagggccagtgcgaagggccgagctgtctcgacagcccgctacttccagtctgcgatctcgggcggctcggcgcactatgttgtcgatgtcggcgaaaccgtgcagtgtctggcagaggatgtgatcgcctggcacgccccgcccaacagccgcagcctggggatcgagatctgcgctgacggcggctcggcgaccagcttcaagaaccccaacgtgcgctacagccgcgcccagtggctcagcccgcaggtctggcccgccgtgctccgtgccgcagcactcacccggcagatgtgccagaagtacggcataccggtcaccaagctcagcgcgtcggacctcaaggccgggaagaagggcatctgcggacacgtcgatgtcagcaatgcgtggcatcagtccgaccacgacgaccccggcccggacttcccctgggccgaattcatggcagccgtcaaaggcggcgccaccaaccccgatgaactggagctcacaggcggttatttcccttggaatgaatttattgccgccgtccaaggaaaaaccaccacaccagagggagaactcagcatgtcagacgtaaacaccctgaccaagctcatcaaggccagcaacgaccagcttcactacgatattggcgtcgtccagacgcaaaacgggaacatcaagaagaagatcgacaatctgtcgtgggtgaagaaccccgtcaccggcaagaagtggtccactaaggatgccctgtggtccgtctggtattacgtgctggaatgccgcaaccgcatccaggctatcgagaaccgtatttacgaccttgagaagaaggtgaagtga

SEQ ID NO: 306 - DNA, 921 bp, Artificial Sequence
atgacattcatccaggcccgccatcacggcggcaactccaacacgccgatcacccggctggtcatccacgccacctgccccgacgtgggctacccgtcggcgtcgaaggccggtagggcagtctccacggcggagtatttcgcgtccacgtcgcggtctgcctcggctcactacgtctgtgacgtatcggcaacggtgcagtgcctctccgaggaaaccatcggctaccacgcgccgcccaacagtcattccatcggcattgagatttgcgccgacggcgggtcccgcgcctcatttgagaaggcttctcacgcatacacccgcgagcaatggctctcgcctcaagtgtggcccgccgtggagcgcgccgccattctcgcccgcggcatctgccaccgccaccacatcccggttcgcaaactcaccaccgcacaggtcaaatcggggatgtcgggtatttgcggacacgacaacgtatccgatgcattccaccaatccgaccacgacgaccctggcccctacttcccgtggaacgaatttatcgccgccatccaaggaaaaaacaccaacaagggagaactcagcggcggttatttcccttggaatgaatttattgccgccgtccaaggaaaaaccaccacaccagagggagaactcagcatgtcagacgtaaacaccctgaccaagctcatcaaggccagcaacgaccagcttcactacgatattggcgtcgtccagacgcaaaacgggaacatcaagaagaagatcgacaatctgtcgtgggtgaagaaccccgtcaccggcaagaagtggtccactaaggatgccctgtggtccgtctggtattacgtgctggaatgccgcaaccgcatccaggctatcgagaaccgtatttacgaccttgagaagaaggtgaagtga

SEQ ID NO: 307 - DNA, 894 bp, Artificial Sequence
atgacattcattcaggccaagcatcacggcggccacaacaaccctcccgtgactcgtcttgtcattcacgccacatgcccggatgtgggctatccgtctgcgtcgcgcgctggccgtgcggtgtcgacggcccactattttcaggaaacgacccggccagcatccgcccactacatttgtgacatatcgaccacggtgcagtgtctgtctgaggagacggtgggctatcacgccccgccgaactcacactccatcggtattgagatatgcgctgacggtgggtcgcatgcctcgttttcgaaccctgcccacgcctacacccgcgagcagtggttgagccctcaggtgtggcctgctgtggagcgtgccgcgatgctggcgcgcggtatctgtcaacgccacaacatcccgatccgccgcctctcgatcgctgacgtcaaggccgggaagcgcggcatctgcggccacaacgaggtgtccgaggccttccaccaatccgaccatgacgaccccggtccttatttcccgtgggacgggtttatcgcgcttgttaatggccattccgcaccatcacgccaggaggaactaactgtgtcagatggcggtaaaaacaccaacaagggagaactcagcatgtccgacgtcaacaccctgaccaagctcatcaaggccagcaacaatcagctccaccacgacattggcgtcgtccagacacagaacggcaccctcaaaagcaagatcgacaacttgtcgtgggtgaagaatcccgtcaccggcaagaagtggtccaccaaggatgcgctgtggtctgtctggtactacgtgctggaatgccgcaaccgcatccaggctatcgaaaaccgcctctctgacatcgaaaagaaggtgaagtga

SEQ ID NO: 308 - DNA, 894 bp, Artificial Sequence
atgacgttcattcaggccgcgcatcacagcagcggctccaatctgccacccacgagggtggtgatccatgcgacatgccccgagatgggattcccgaaggccagtgcgaagggcagggctgtctcgacggcccgatacttccagtctgcgagctcgggcggtagcgcccactatgttgtcgacatcggcgagacggtgcagtgtctcggtgagaacgtgatcgcgtggcacgccccgcccaatgcccacagtctcggcatcgagatctgcgcggacgggggatcggccacctccttctccaatcccaaggtgcgctacacgcgggcgcagtggctgagcccgcaggtgtggcccgccgtgctccgtgccgcagcactcacccggaagatgtgcagcaagtacggcatccccgtcgtcaagctgtccgcgtcggacctcaaggccggaaagaagggcatctgcggccacgtggatgtcagcaatgctttccaccagtccgaccacgacgaccccggccccgacttcccgtgggccgaattcatggcagccgtcaaaggcggcaccaccacacaggaagatgaggatgaaatgaaggaagctggcggtaaaaacaccaacaagggagaactcagcatgtccgacgtcaacaccctgaccaagctcatcaaggccagcaacaatcagctccaccacgacattggcgtcgtccagacacagaacggcaccctcaaaagcaagatcgacaacttgtcgtgggtgaagaatcccgtcaccggcaagaagtggtccaccaaggatgcgctgtggtctgtctggtactacgtgctggaatgccgcaaccgcatccaggctatcgaaaaccgcctctctgacatcgaaaagaaggtgaagtga

SEQ ID NO: 309 - DNA, 873 bp, Artificial Sequence
atgacattcatccaggcccgccatcacggcggcaactccaacacgccgatcacccggctggtcatccacgccacctgccccgacgtgggctacccgtcggcgtcgaaggccggtagggcagtctccacggcggagtatttcgcgtccacgtcgcggtctgcctcggctcactacgtctgtgacgtatcggcaacggtgcagtgcctctccgaggaaaccatcggctaccacgcgccgcccaacagtcattccatcggcattgagatttgcgccgacggcgggtcccgcgcctcatttgagaaggcttctcacgcatacacccgcgagcaatggctctcgcctcaagtgtggcccgccgtggagcgcgccgccattctcgcccgcggcatctgccaccgccaccacatcccggttcgcaaactcaccaccgcacaggtcaaatcggggatgtcgggtatttgcggacacgacaacgtatccgatgcattccaccaatccgaccacgacgaccctggcccctacttcccgtggaacgaatttatcgccgccatccaaggaggcggtgaggttagaacaccaggacaacaagatacgaaaccttccgtaccaacaccatcactcacagaaataggagatcaggacatgaacgggtgctactacaacctcaattcgaaaacacggacgtaccttatcttcgatagccgttccggattttaccacgaattctcccaaggcaatgggaacggccccatgagcccagactatgtaaatccgatcgccaaaggatgggacaccggatcatggccggcaatctccccaggccacgcgaaagtgctcaaggccgccctcgataaagtccggaaaggaatctga

SEQ ID NO: 310 - DNA, 861 bp, Artificial Sequence
atgacattcatccaggcccgccatcacggcggcaactccaacacgccgatcacccggctggtcatccacgccacctgccccgacgtgggctacccgtcggcgtcgaaggccggtagggcagtctccacggcggagtatttcgcgtccacgtcgcggtctgcctcggctcactacgtctgtgacgtatcggcaacggtgcagtgcctctccgaggaaaccatcggctaccacgcgccgcccaacagtcattccatcggcattgagatttgcgccgacggcgggtcccgcgcctcatttgagaaggcttctcacgcatacacccgcgagcaatggctctcgcctcaagtgtggcccgccgtggagcgcgccgccattctcgcccgcggcatctgccaccgccaccacatcccggttcgcaaactcaccaccgcacaggtcaaatcggggatgtcgggtatttgcggacacgacaacgtatccgatgcattccaccaatccgaccacgacgaccctggcccctacttcccgtggaacgaatttatcgccgccatccaaggaggcggtccaggacaacaagatacgaaaccttccgtaccaacaccatcactcacagaaataggagatcaggacatgaacgggtgctactacaacctcaattcgaaaacacggacgtaccttatcttcgatagccgttccggattttaccacgaattctcccaaggcaatgggaacggccccatgagcccagactatgtaaatccgatcgccaaaggatgggacaccggatcatggccggcaatctccccaggccacgcgaaagtgctcaaggccgccctcgataaagtccggaaaggaatctga

SEQ ID NO: 311 - DNA, 870 bp, Artificial Sequence
atgacgttcattcaggccgcgcatcacagcagcggctccaatctgccgcccacgagggtggtgatccacgcgacatgccccgaactcggcttcccgagggccagtgcgaagggccgagctgtctcgacagcccgctacttccagtctgcgatctcgggcggctcggcgcactatgttgtcgatgtcggcgaaaccgtgcagtgtctggcagaggatgtgatcgcctggcacgccccgcccaacagccgcagcctggggatcgagatctgcgctgacggcggctcggcgaccagcttcaagaaccccaacgtgcgctacagccgcgcccagtggctcagcccgcaggtctggcccgccgtgctccgtgccgcagcactcacccggcagatgtgccagaagtacggcataccggtcaccaagctcagcgcgtcggacctcaaggccgggaagaagggcatctgcggacacgtcgatgtcagcaatgcgtggcatcagtccgaccacgacgaccccggcccggacttcccctgggccgaattcatggcagccgtcaaaggcggtgaggttagaacaccaggacaacaagatacgaaaccttccgtaccaacaccatcactcacagaaataggagatcaggacatgaacgggtgctactacaacctcaattcgaaaacacggacgtaccttatcttcgatagccgttccggattttaccacgaattctcccaaggcaatgggaacggccccatgagcccagactatgtaaatccgatcgccaaaggatgggacaccggatcatggccggcaatctccccaggccacgcgaaagtgctcaaggccgccctcgataaagtccggaaaggaatctga

SEQ ID NO: 312 - DNA, 852 bp, Artificial Sequence
atgacattcatccaggcccgccatcacggcggcaactccaacacgccgatcacccggctggtcatccacgccacctgccccgacgtgggctacccgtcggcgtcgaaggccggtagggcagtctccacggcggagtatttcgcgtccacgtcgcggtctgcctcggctcactacgtctgtgacgtatcggcaacggtgcagtgcctctccgaggaaaccatcggctaccacgcgccgcccaacagtcattccatcggcattgagatttgcgccgacggcgggtcccgcgcctcatttgagaaggcttctcacgcatacacccgcgagcaatggctctcgcctcaagtgtggcccgccgtggagcgcgccgccattctcgcccgcggcatctgccaccgccaccacatcccggttcgcaaactcaccaccgcacaggtcaaatcggggatgtcgggtatttgcggacacgacaacgtatccgatgcattccaccaatccgaccacgacgaccctggcccctacttcccgtggaacgaatttatcgccgccatccaaggaggcggtaaaaacaccaacaagggagaactcagcatgtccgacgtcaacaccctgaccaagctcatcaaggccagcaacaatcagctccaccacgacattggcgtcgtccagacacagaacggcaccctcaaaagcaagatcgacaacttgtcgtgggtgaagaatcccgtcaccggcaagaagtggtccaccaaggatgcgctgtggtctgtctggtactacgtgctggaatgccgcaaccgcatccaggctatcgaaaaccgcctctctgacatcgaaaagaaggtgaagtga

SEQ ID NO: 313 - DNA, 897 bp, Artificial Sequence
atgacgttcattcaggccgcgcatcacagcagcggctccaatctgccgcccacgagggtggtgatccacgcgacatgccccgaactcggcttcccgagggccagtgcgaagggccgagctgtctcgacagcccgctacttccagtctgcgatctcgggcggctcggcgcactatgttgtcgatgtcggcgaaaccgtgcagtgtctggcagaggatgtgatcgcctggcacgccccgcccaacagccgcagcctggggatcgagatctgcgctgacggcggctcggcgaccagcttcaagaaccccaacgtgcgctacagccgcgcccagtggctcagcccgcaggtctggcccgccgtgctccgtgccgcagcactcacccggcagatgtgccagaagtacggcataccggtcaccaagctcagcgcgtcggacctcaaggccgggaagaagggcatctgcggacacgtcgatgtcagcaatgcgtggcatcagtccgaccacgacgaccccggcccggacttcccctgggccgaattcatggcagccgtcaaaggcggtacattcccgtgggaccaattcatcaaagaggttagaacaccaggacaacaagatacgaaaccttccgtaccaacaccatcactcacagaaataggagatcaggacatgaacgggtgctactacaacctcaattcgaaaacacggacgtaccttatcttcgatagccgttccggattttaccacgaattctcccaaggcaatgggaacggccccatgagcccagactatgtaaatccgatcgccaaaggatgggacaccggatcatggccggcaatctccccaggccacgcgaaagtgctcaaggccgccctcgataaagtccggaaaggaatctga

SEQ ID NO: 314 - DNA, 900 bp, Artificial Sequence
atgacattcatccaggcccgccatcacggcggcaactccaacacgccgatcacccggctggtcatccacgccacctgccccgacgtgggctacccgtcggcgtcgaaggccggtagggcagtctccacggcggagtatttcgcgtccacgtcgcggtctgcctcggctcactacgtctgtgacgtatcggcaacggtgcagtgcctctccgaggaaaccatcggctaccacgcgccgcccaacagtcattccatcggcattgagatttgcgccgacggcgggtcccgcgcctcatttgagaaggcttctcacgcatacacccgcgagcaatggctctcgcctcaagtgtggcccgccgtggagcgcgccgccattctcgcccgcggcatctgccaccgccaccacatcccggttcgcaaactcaccaccgcacaggtcaaatcggggatgtcgggtatttgcggacacgacaacgtatccgatgcattccaccaatccgaccacgacgaccctggcccctacttcccgtggaacgaatttatcgccgccatccaaggaggcggtacattcccgtgggaccaattcatcaaagaggttagaacaccaggacaacaagatacgaaaccttccgtaccaacaccatcactcacagaaataggagatcaggacatgaacgggtgctactacaacctcaattcgaaaacacggacgtaccttatcttcgatagccgttccggattttaccacgaattctcccaaggcaatgggaacggccccatgagcccagactatgtaaatccgatcgccaaaggatgggacaccggatcatggccggcaatctccccaggccacgcgaaagtgctcaaggccgccctcgataaagtccggaaaggaatctga

SEQ ID NO: 315 - DNA, 870 bp, Artificial Sequence
atgacgttcattcaggccgcgcatcacagcagcggctccaatctgccacccacgagggtggtgatccatgcgacatgccccgagatgggattcccgaaggccagtgcgaagggcagggctgtctcgacggcccgatacttccagtctgcgagctcgggcggtagcgcccactatgttgtcgacatcggcgagacggtgcagtgtctcggtgagaacgtgatcgcgtggcacgccccgcccaatgcccacagtctcggcatcgagatctgcgcggacgggggatcggccacctccttctccaatcccaaggtgcgctacacgcgggcgcagtggctgagcccgcaggtgtggcccgccgtgctccgtgccgcagcactcacccggaagatgtgcagcaagtacggcatccccgtcgtcaagctgtccgcgtcggacctcaaggccggaaagaagggcatctgcggccacgtggatgtcagcaatgctttccaccagtccgaccacgacgaccccggccccgacttcccgtgggccgaattcatggcagccgtcaaaggcggtgaggttagaacaccaggacaacaagatacgaaaccttccgtaccaacaccatcactcacagaaataggagatcaggacatgaacgggtgctactacaacctcaattcgaaaacacggacgtaccttatcttcgatagccgttccggattttaccacgaattctcccaaggcaatgggaacggccccatgagcccagactatgtaaatccgatcgccaaaggatgggacaccggatcatggccggcaatctccccaggccacgcgaaagtgctcaaggccgccctcgataaagtccggaaaggaatctga

SEQ ID NO: 316 - DNA, 858 bp, Artificial Sequence
atgacgttcattcaggccgcgcatcacagcagcggctccaatctgccacccacgagggtggtgatccatgcgacatgccccgagatgggattcccgaaggccagtgcgaagggcagggctgtctcgacggcccgatacttccagtctgcgagctcgggcggtagcgcccactatgttgtcgacatcggcgagacggtgcagtgtctcggtgagaacgtgatcgcgtggcacgccccgcccaatgcccacagtctcggcatcgagatctgcgcggacgggggatcggccacctccttctccaatcccaaggtgcgctacacgcgggcgcagtggctgagcccgcaggtgtggcccgccgtgctccgtgccgcagcactcacccggaagatgtgcagcaagtacggcatccccgtcgtcaagctgtccgcgtcggacctcaaggccggaaagaagggcatctgcggccacgtggatgtcagcaatgctttccaccagtccgaccacgacgaccccggccccgacttcccgtgggccgaattcatggcagccgtcaaaggcggtccaggacaacaagatacgaaaccttccgtaccaacaccatcactcacagaaataggagatcaggacatgaacgggtgctactacaacctcaattcgaaaacacggacgtaccttatcttcgatagccgttccggattttaccacgaattctcccaaggcaatgggaacggccccatgagcccagactatgtaaatccgatcgccaaaggatgggacaccggatcatggccggcaatctccccaggccacgcgaaagtgctcaaggccgccctcgataaagtccggaaaggaatctga

SEQ ID NO: 317 - DNA, 888 bp, Artificial Sequence
atgacgttcattcaggccgcgcatcacagcagcggctccaatctgccgcccacgagggtggtgatccacgcgacatgccccgaactcggcttcccgagggccagtgcgaagggccgagctgtctcgacagcccgctacttccagtctgcgatctcgggcggctcggcgcactatgttgtcgatgtcggcgaaaccgtgcagtgtctggcagaggatgtgatcgcctggcacgccccgcccaacagccgcagcctggggatcgagatctgcgctgacggcggctcggcgaccagcttcaagaaccccaacgtgcgctacagccgcgcccagtggctcagcccgcaggtctggcccgccgtgctccgtgccgcagcactcacccggcagatgtgccagaagtacggcataccggtcaccaagctcagcgcgtcggacctcaaggccgggaagaagggcatctgcggacacgtcgatgtcagcaatgcgtggcatcagtccgaccacgacgaccccggcccggacttcccctgggccgaattcatggcagccgtcaaaggcggcgccaccaaccccggcggtgaggttagaacaccaggacaacaagatacgaaaccttccgtaccaacaccatcactcacagaaataggagatcaggacatgaacgggtgctactacaacctcaattcgaaaacacggacgtaccttatcttcgatagccgttccggattttaccacgaattctcccaaggcaatgggaacggccccatgagcccagactatgtaaatccgatcgccaaaggatgggacaccggatcatggccggcaatctccccaggccacgcgaaagtgctcaaggccgccctcgataaagtccggaaaggaatctga

SEQ ID NO: 318 - DNA, 876 bp, Artificial Sequence
atgacgttcattcaggccgcgcatcacagcagcggctccaatctgccgcccacgagggtggtgatccacgcgacatgccccgaactcggcttcccgagggccagtgcgaagggccgagctgtctcgacagcccgctacttccagtctgcgatctcgggcggctcggcgcactatgttgtcgatgtcggcgaaaccgtgcagtgtctggcagaggatgtgatcgcctggcacgccccgcccaacagccgcagcctggggatcgagatctgcgctgacggcggctcggcgaccagcttcaagaaccccaacgtgcgctacagccgcgcccagtggctcagcccgcaggtctggcccgccgtgctccgtgccgcagcactcacccggcagatgtgccagaagtacggcataccggtcaccaagctcagcgcgtcggacctcaaggccgggaagaagggcatctgcggacacgtcgatgtcagcaatgcgtggcatcagtccgaccacgacgaccccggcccggacttcccctgggccgaattcatggcagccgtcaaaggcggcgccaccaaccccggcggtccaggacaacaagatacgaaaccttccgtaccaacaccatcactcacagaaataggagatcaggacatgaacgggtgctactacaacctcaattcgaaaacacggacgtaccttatcttcgatagccgttccggattttaccacgaattctcccaaggcaatgggaacggccccatgagcccagactatgtaaatccgatcgccaaaggatgggacaccggatcatggccggcaatctccccaggccacgcgaaagtgctcaaggccgccctcgataaagtccggaaaggaatctga

SEQ ID NO: 319 - DNA, 867 bp, Artificial Sequence
atgacgttcattcaggccgcgcatcacagcagcggctccaatctgccacccacgagggtggtgatccatgcgacatgccccgagatgggattcccgaaggccagtgcgaagggcagggctgtctcgacggcccgatacttccagtctgcgagctcgggcggtagcgcccactatgttgtcgacatcggcgagacggtgcagtgtctcggtgagaacgtgatcgcgtggcacgccccgcccaatgcccacagtctcggcatcgagatctgcgcggacgggggatcggccacctccttctccaatcccaaggtgcgctacacgcgggcgcagtggctgagcccgcaggtgtggcccgccgtgctccgtgccgcagcactcacccggaagatgtgcagcaagtacggcatccccgtcgtcaagctgtccgcgtcggacctcaaggccggaaagaagggcatctgcggccacgtggatgtcagcaatgctttccaccagtccgaccacgacgaccccggccccgacttcccgtgggccgaattcatggcagccgtcaaaggcggtaacggcggtagtggagatagtggggagttaactgtggctgatgtgaaagccttgcatgatcagattaaacaattgtctgctcagcttactggttcggtgaataagctgcaccatgatgttggtgtggtacaggtacagaatggtgatttgggtaaacgtgttgatgccttgtcgtgggtgaagaatccggtgacggggaagctgtggcgcaccaaagacgctttgtggagtgtctggtattacgtgctggagtgtcgcagccgcatagacaggctcgagtctgctgttaacggtttgaaaaagtga

SEQ ID NO: 320 - DNA, 897 bp, Artificial Sequence
atgacgttcattcaggccgcgcatcacagcagcggctccaatctgccacccacgagggtggtgatccatgcgacatgccccgagatgggattcccgaaggccagtgcgaagggcagggctgtctcgacggcccgatacttccagtctgcgagctcgggcggtagcgcccactatgttgtcgacatcggcgagacggtgcagtgtctcggtgagaacgtgatcgcgtggcacgccccgcccaatgcccacagtctcggcatcgagatctgcgcggacgggggatcggccacctccttctccaatcccaaggtgcgctacacgcgggcgcagtggctgagcccgcaggtgtggcccgccgtgctccgtgccgcagcactcacccggaagatgtgcagcaagtacggcatccccgtcgtcaagctgtccgcgtcggacctcaaggccggaaagaagggcatctgcggccacgtggatgtcagcaatgctttccaccagtccgaccacgacgaccccggccccgacttcccgtgggccgaattcatggcagccgtcaaaggcggtacattcccgtgggaccaattcatcaaagaggttagaacaccaggacaacaagatacgaaaccttccgtaccaacaccatcactcacagaaataggagatcaggacatgaacgggtgctactacaacctcaattcgaaaacacggacgtaccttatcttcgatagccgttccggattttaccacgaattctcccaaggcaatgggaacggccccatgagcccagactatgtaaatccgatcgccaaaggatgggacaccggatcatggccggcaatctccccaggccacgcgaaagtgctcaaggccgccctcgataaagtccggaaaggaatctga

SEQ ID NO: 321 - DNA, 906 bp, Artificial Sequence
atgacgttcattcaggccgcgcatcacagcagcggctccaatctgccgcccacgagggtggtgatccacgcgacatgccccgaactcggcttcccgagggccagtgcgaagggccgagctgtctcgacagcccgctacttccagtctgcgatctcgggcggctcggcgcactatgttgtcgatgtcggcgaaaccgtgcagtgtctggcagaggatgtgatcgcctggcacgccccgcccaacagccgcagcctggggatcgagatctgcgctgacggcggctcggcgaccagcttcaagaaccccaacgtgcgctacagccgcgcccagtggctcagcccgcaggtctggcccgccgtgctccgtgccgcagcactcacccggcagatgtgccagaagtacggcataccggtcaccaagctcagcgcgtcggacctcaaggccgggaagaagggcatctgcggacacgtcgatgtcagcaatgcgtggcatcagtccgaccacgacgaccccggcccggacttcccctgggccgaattcatggcagccgtcaaaggcggcgccaccaaccccgatgaactggagctcacaggcggtgaggttagaacaccaggacaacaagatacgaaaccttccgtaccaacaccatcactcacagaaataggagatcaggacatgaacgggtgctactacaacctcaattcgaaaacacggacgtaccttatcttcgatagccgttccggattttaccacgaattctcccaaggcaatgggaacggccccatgagcccagactatgtaaatccgatcgccaaaggatgggacaccggatcatggccggcaatctccccaggccacgcgaaagtgctcaaggccgccctcgataaagtccggaaaggaatctga

SEQ ID NO: 322 - DNA, 900 bp, Artificial Sequence
atgacattcatccaggcccgccatcacggcggcaactccaacacgccgatcacccggctggtcatccacgccacctgccccgacgtgggctacccgtcggcgtcgaaggccggtagggcagtctccacggcggagtatttcgcgtccacgtcgcggtctgcctcggctcactacgtctgtgacgtatcggcaacggtgcagtgcctctccgaggaaaccatcggctaccacgcgccgcccaacagtcattccatcggcattgagatttgcgccgacggcgggtcccgcgcctcatttgagaaggcttctcacgcatacacccgcgagcaatggctctcgcctcaagtgtggcccgccgtggagcgcgccgccattctcgcccgcggcatctgccaccgccaccacatcccggttcgcaaactcaccaccgcacaggtcaaatcggggatgtcgggtatttgcggacacgacaacgtatccgatgcattccaccaatccgaccacgacgaccctggcccctacttcccgtggaacgaatttatcgccgccatccaaggaaaaaacaccaacaagggagaactcagcggcggtgaggttagaacaccaggacaacaagatacgaaaccttccgtaccaacaccatcactcacagaaataggagatcaggacatgaacgggtgctactacaacctcaattcgaaaacacggacgtaccttatcttcgatagccgttccggattttaccacgaattctcccaaggcaatgggaacggccccatgagcccagactatgtaaatccgatcgccaaaggatgggacaccggatcatggccggcaatctccccaggccacgcgaaagtgctcaaggccgccctcgataaagtccggaaaggaatctga

SEQ ID NO: 323 - DNA, 894 bp, Artificial Sequence
atgacgttcattcaggccgcgcatcacagcagcggctccaatctgccgcccacgagggtggtgatccacgcgacatgccccgaactcggcttcccgagggccagtgcgaagggccgagctgtctcgacagcccgctacttccagtctgcgatctcgggcggctcggcgcactatgttgtcgatgtcggcgaaaccgtgcagtgtctggcagaggatgtgatcgcctggcacgccccgcccaacagccgcagcctggggatcgagatctgcgctgacggcggctcggcgaccagcttcaagaaccccaacgtgcgctacagccgcgcccagtggctcagcccgcaggtctggcccgccgtgctccgtgccgcagcactcacccggcagatgtgccagaagtacggcataccggtcaccaagctcagcgcgtcggacctcaaggccgggaagaagggcatctgcggacacgtcgatgtcagcaatgcgtggcatcagtccgaccacgacgaccccggcccggacttcccctgggccgaattcatggcagccgtcaaaggcggcgccaccaaccccgatgaactggagctcacaggcggtccaggacaacaagatacgaaaccttccgtaccaacaccatcactcacagaaataggagatcaggacatgaacgggtgctactacaacctcaattcgaaaacacggacgtaccttatcttcgatagccgttccggattttaccacgaattctcccaaggcaatgggaacggccccatgagcccagactatgtaaatccgatcgccaaaggatgggacaccggatcatggccggcaatctccccaggccacgcgaaagtgctcaaggccgccctcgataaagtccggaaaggaatctga

SEQ ID NO: 324 - DNA, 915 bp, Artificial Sequence
atgacgttcattcaggccgcgcatcacagcagcggctccaatctgccacccacgagggtggtgatccatgcgacatgccccgagatgggattcccgaaggccagtgcgaagggcagggctgtctcgacggcccgatacttccagtctgcgagctcgggcggtagcgcccactatgttgtcgacatcggcgagacggtgcagtgtctcggtgagaacgtgatcgcgtggcacgccccgcccaatgcccacagtctcggcatcgagatctgcgcggacgggggatcggccacctccttctccaatcccaaggtgcgctacacgcgggcgcagtggctgagcccgcaggtgtggcccgccgtgctccgtgccgcagcactcacccggaagatgtgcagcaagtacggcatccccgtcgtcaagctgtccgcgtcggacctcaaggccggaaagaagggcatctgcggccacgtggatgtcagcaatgctttccaccagtccgaccacgacgaccccggccccgacttcccgtgggccgaattcatggcagccgtcaaaggcggcaccaccacacaggaagatgaggatgaaatgaaggaagctggcggtgaggttagaacaccaggacaacaagatacgaaaccttccgtaccaacaccatcactcacagaaataggagatcaggacatgaacgggtgctactacaacctcaattcgaaaacacggacgtaccttatcttcgatagccgttccggattttaccacgaattctcccaaggcaatgggaacggccccatgagcccagactatgtaaatccgatcgccaaaggatgggacaccggatcatggccggcaatctccccaggccacgcgaaagtgctcaaggccgccctcgataaagtccggaaaggaatctga

SEQ ID NO: 325 - DNA, 873 bp, Artificial Sequence
atgaaatacattcccgcgacacatcacggaggccacacgaacacccccttcacccggatcgtgatccacgccacctgccccgaccttggcttcccccacgcatcagctggtggacaggcaaaagccaccgcacgctatttccaatcagagcagtctgccggatcagcacactatgtgtgcgacatcgccgagactatccaatgcctgcccgatgacgtgatcgcctggcacgccccaccaaacagaaggtcgatcggaatcgaaatatgtgccgacggcggctcccgctcctcattccagcaccccgagcacgcctacaccagatcccaatggctcagcccccaagtgtggcccgccgtcgcccgtgccgccgcgctcacccgcgacctctgccaccgccacaacattccgatgcaacaactctccgttgctgatgtgaaagccgggaagcacggaatctgcggccacaacgacgtatccgaggcattccacaagtccgaccatgacgaccccggccccacattcccgtgggaccaattcatcaaagaggttagaacaggcggtgaggttagaacaccaggacaacaagatacgaaaccttccgtaccaacaccatcactcacagaaataggagatcaggacatgaacgggtgctactacaacctcaattcgaaaacacggacgtaccttatcttcgatagccgttccggattttaccacgaattctcccaaggcaatgggaacggccccatgagcccagactatgtaaatccgatcgccaaaggatgggacaccggatcatggccggcaatctccccaggccacgcgaaagtgctcaaggccgccctcgataaagtccggaaaggaatctga

SEQ ID NO: 326 - DNA, 954 bp, Artificial Sequence
atgagatacattcctgcggcgcatcattctgccggatcaaataagccggtgaaccgggttgtgattcatgcaacatgcccggatgtggggtttccgtctgcttcgcgtaagggtcgggcggtgtctacagcaaactattttgcttccccatcgtctggtggttcggcgcattatgtgtgtgatattggggagacggtgcagtgcttgtcggagtctacgattggttggcatgccccgccgaatccgcatagtttgggtatagagatttgcgcggatgggggttcgcacgcctcattccgtgttccagggcatgcctatacgcgggagcagtggcttgaccctcgggtgtggcccgcggtggagagggccgccatcctgtgtcggcagttgtgtgataagcatggtgttccgaagaggaaactgtctgtggctgatttgaaggccggtaaacggggtgtttgcgggcatgtggatgttacggatgcgtggcatcagtcggatcatgacgatccggggccgtggtttccgtgggacaaatttatggctgtggtgaatggccacggcggcggttcaagtagtgaggagttgagtatggctgatgtacaagcgttacataatcagattaaacagttgtcggcaggcggtgaggttagaacaccaggacaacaagatacgaaaccttccgtaccaacaccatcactcacagaaataggagatcaggacatgaacgggtgctactacaacctcaattcgaaaacacggacgtaccttatcttcgatagccgttccggattttaccacgaattctcccaaggcaatgggaacggccccatgagcccagactatgtaaatccgatcgccaaaggatgggacaccggatcatggccggcaatctccccaggccacgcgaaagtgctcaaggccgccctcgataaagtccggaaaggaatctga

SEQ ID NO: 327 - DNA, 861 bp, Artificial Sequence
atgaaatacattcccgcgacacatcacggaggccacacgaacacccccttcacccggatcgtgatccacgccacctgccccgaccttggcttcccccacgcatcagctggtggacaggcaaaagccaccgcacgctatttccaatcagagcagtctgccggatcagcacactatgtgtgcgacatcgccgagactatccaatgcctgcccgatgacgtgatcgcctggcacgccccaccaaacagaaggtcgatcggaatcgaaatatgtgccgacggcggctcccgctcctcattccagcaccccgagcacgcctacaccagatcccaatggctcagcccccaagtgtggcccgccgtcgcccgtgccgccgcgctcacccgcgacctctgccaccgccacaacattccgatgcaacaactctccgttgctgatgtgaaagccgggaagcacggaatctgcggccacaacgacgtatccgaggcattccacaagtccgaccatgacgaccccggccccacattcccgtgggaccaattcatcaaagaggttagaacaggcggtccaggacaacaagatacgaaaccttccgtaccaacaccatcactcacagaaataggagatcaggacatgaacgggtgctactacaacctcaattcgaaaacacggacgtaccttatcttcgatagccgttccggattttaccacgaattctcccaaggcaatgggaacggccccatgagcccagactatgtaaatccgatcgccaaaggatgggacaccggatcatggccggcaatctccccaggccacgcgaaagtgctcaaggccgccctcgataaagtccggaaaggaatctga

SEQ ID NO: 328 - DNA, 891 bp, Artificial Sequence
atgacattcatccaggcccgccaccacggcggcaactccaacgcgccgatcacccggctggtcatccacgccacctgccccgacgtgggctacccgtcggcatcgaaggccggtagggcagtctcgaccgcgaactacttcgccacgactgatcggcccgcctcggcacattacgtatgtgacatcgccactacagtgcagtgcctctccgaggaaaccatcggctaccacgcgccgccgaactcgcattccatcggcattgaaatttgcgccgatggcgggtcgcacgcctcatttgagaaggcttctcacgcatacacccgcgaccaatggttgagcgatgacgtgtggcccgccgtagagcgcgccgccattcttgcccgcgatatttgccaacgacaccgcatcccggttcgtaaactctccaccgcacaggtgaaagccggactgtcgggaatttgcggacacgacaatgtatccggcgcattccatcagtccgaccacgacgacccgggcccctacttcccgtgggaccagttcatggcactcgtccaaggaaaacccgccacaccaggagatctcaccatgggcggtccaggacaacaagatacgaaaccttccgtaccaacaccatcactcacagaaataggagatcaggacatgaacgggtgctactacaacctcaattcgaaaacacggacgtaccttatcttcgatagccgttccggattttaccacgaattctcccaaggcaatgggaacggccccatgagcccagactatgtaaatccgatcgccaaaggatgggacaccggatcatggccggcaatctccccaggccacgcgaaagtgctcaaggccgccctcgataaagtccggaaaggaatctga

SEQ ID NO: 329 - DNA, 915 bp, Artificial Sequence
atgacattcattcaggccaagcatcacggcggccacaacaaccctcccgtgactcgtcttgtcattcacgccacatgcccggatgtgggctatccgtctgcgtcgcgcgctggccgtgcggtgtcgacggcccactattttcaggaaacgacccggccagcatccgcccactacatttgtgacatatcgaccacggtgcagtgtctgtctgaggagacggtgggctatcacgccccgccgaactcacactccatcggtattgagatatgcgctgacggtgggtcgcatgcctcgttttcgaaccctgcccacgcctacacccgcgagcagtggttgagccctcaggtgtggcctgctgtggagcgtgccgcgatgctggcgcgcggtatctgtcaacgccacaacatcccgatccgccgcctctcgatcgctgacgtcaaggccgggaagcgcggcatctgcggccacaacgaggtgtccgaggccttccaccaatccgaccatgacgaccccggtccttatttcccgtgggacgggtttatcgcgcttgttaatggccattccgcaccatcacgccaggaggaactaactgtgtcagatggcggtgaggttagaacaccaggacaacaagatacgaaaccttccgtaccaacaccatcactcacagaaataggagatcaggacatgaacgggtgctactacaacctcaattcgaaaacacggacgtaccttatcttcgatagccgttccggattttaccacgaattctcccaaggcaatgggaacggccccatgagcccagactatgtaaatccgatcgccaaaggatgggacaccggatcatggccggcaatctccccaggccacgcgaaagtgctcaaggccgccctcgataaagtccggaaaggaatctga

SEQ ID NO: 330 - DNA, 903 bp, Artificial Sequence
atgacgttcattcaggccgcgcatcacagcagcggctccaatctgccacccacgagggtggtgatccatgcgacatgccccgagatgggattcccgaaggccagtgcgaagggcagggctgtctcgacggcccgatacttccagtctgcgagctcgggcggtagcgcccactatgttgtcgacatcggcgagacggtgcagtgtctcggtgagaacgtgatcgcgtggcacgccccgcccaatgcccacagtctcggcatcgagatctgcgcggacgggggatcggccacctccttctccaatcccaaggtgcgctacacgcgggcgcagtggctgagcccgcaggtgtggcccgccgtgctccgtgccgcagcactcacccggaagatgtgcagcaagtacggcatccccgtcgtcaagctgtccgcgtcggacctcaaggccggaaagaagggcatctgcggccacgtggatgtcagcaatgctttccaccagtccgaccacgacgaccccggccccgacttcccgtgggccgaattcatggcagccgtcaaaggcggcaccaccacacaggaagatgaggatgaaatgaaggaagctggcggtccaggacaacaagatacgaaaccttccgtaccaacaccatcactcacagaaataggagatcaggacatgaacgggtgctactacaacctcaattcgaaaacacggacgtaccttatcttcgatagccgttccggattttaccacgaattctcccaaggcaatgggaacggccccatgagcccagactatgtaaatccgatcgccaaaggatgggacaccggatcatggccggcaatctccccaggccacgcgaaagtgctcaaggccgccctcgataaagtccggaaaggaatctga

SEQ ID NO: 331 - DNA, 903 bp, Artificial Sequence
atgacattcattcaggccaagcatcacggcggccacaacaaccctcccgtgactcgtcttgtcattcacgccacatgcccggatgtgggctatccgtctgcgtcgcgcgctggccgtgcggtgtcgacggcccactattttcaggaaacgacccggccagcatccgcccactacatttgtgacatatcgaccacggtgcagtgtctgtctgaggagacggtgggctatcacgccccgccgaactcacactccatcggtattgagatatgcgctgacggtgggtcgcatgcctcgttttcgaaccctgcccacgcctacacccgcgagcagtggttgagccctcaggtgtggcctgctgtggagcgtgccgcgatgctggcgcgcggtatctgtcaacgccacaacatcccgatccgccgcctctcgatcgctgacgtcaaggccgggaagcgcggcatctgcggccacaacgaggtgtccgaggccttccaccaatccgaccatgacgaccccggtccttatttcccgtgggacgggtttatcgcgcttgttaatggccattccgcaccatcacgccaggaggaactaactgtgtcagatggcggtccaggacaacaagatacgaaaccttccgtaccaacaccatcactcacagaaataggagatcaggacatgaacgggtgctactacaacctcaattcgaaaacacggacgtaccttatcttcgatagccgttccggattttaccacgaattctcccaaggcaatgggaacggccccatgagcccagactatgtaaatccgatcgccaaaggatgggacaccggatcatggccggcaatctccccaggccacgcgaaagtgctcaaggccgccctcgataaagtccggaaaggaatctga

SEQ ID NO: 332 - DNA, 780 bp, Artificial Sequence
atgacgttcattcaggccgcgcatcacagcagcggctccaatctgccgcccacgagggtggtgatccacgcgacatgccccgaactcggcttcccgagggccagtgcgaagggccgagctgtctcgacagcccgctacttccagtctgcgatctcgggcggctcggcgcactatgttgtcgatgtcggcgaaaccgtgcagtgtctggcagaggatgtgatcgcctggcacgccccgcccaacagccgcagcctggggatcgagatctgcgctgacggcggctcggcgaccagcttcaagaaccccaacgtgcgctacagccgcgcccagtggctcagcccgcaggtctggcccgccgtgctccgtgccgcagcactcacccggcagatgtgccagaagtacggcataccggtcaccaagctcagcgcgtcggacctcaaggccgggaagaagggcatctgcggacacgtcgatgtcagcaatgcgtggcatcagtccgaccacgacgaccccggcccggacttcccctgggccgaattcatggcagccgtcaaaggcggtgtgtctcaattcagtgacctgaccaagcgcctgcagggcatgcaggagcagacccaccacgacctcggcgtcgtccagaccaagctggccaccatggacaccgtcaagaacccccgcaccggcgccaagtggagcctcaaggacgccatctggtcgatctggtactacgtgctggagaacagggaccggatcgccgccctcgagaagaaggtgaagtga

SEQ ID NO: 333 - DNA, 798 bp, Artificial Sequence
atgacgttcattcaggccgcgcatcacagcagcggctccaatctgccgcccacgagggtggtgatccacgcgacatgccccgaactcggcttcccgagggccagtgcgaagggccgagctgtctcgacagcccgctacttccagtctgcgatctcgggcggctcggcgcactatgttgtcgatgtcggcgaaaccgtgcagtgtctggcagaggatgtgatcgcctggcacgccccgcccaacagccgcagcctggggatcgagatctgcgctgacggcggctcggcgaccagcttcaagaaccccaacgtgcgctacagccgcgcccagtggctcagcccgcaggtctggcccgccgtgctccgtgccgcagcactcacccggcagatgtgccagaagtacggcataccggtcaccaagctcagcgcgtcggacctcaaggccgggaagaagggcatctgcggacacgtcgatgtcagcaatgcgtggcatcagtccgaccacgacgaccccggcccggacttcccctgggccgaattcatggcagccgtcaaaggcggtgatgaactggagctcacagtgtctcaattcagtgacctgaccaagcgcctgcagggcatgcaggagcagacccaccacgacctcggcgtcgtccagaccaagctggccaccatggacaccgtcaagaacccccgcaccggcgccaagtggagcctcaaggacgccatctggtcgatctggtactacgtgctggagaacagggaccggatcgccgccctcgagaagaaggtgaagtga

SEQ ID NO: 334 - DNA, 816 bp, Artificial Sequence
atgacgttcattcaggccgcgcatcacagcagcggctccaatctgccgcccacgagggtggtgatccacgcgacatgccccgaactcggcttcccgagggccagtgcgaagggccgagctgtctcgacagcccgctacttccagtctgcgatctcgggcggctcggcgcactatgttgtcgatgtcggcgaaaccgtgcagtgtctggcagaggatgtgatcgcctggcacgccccgcccaacagccgcagcctggggatcgagatctgcgctgacggcggctcggcgaccagcttcaagaaccccaacgtgcgctacagccgcgcccagtggctcagcccgcaggtctggcccgccgtgctccgtgccgcagcactcacccggcagatgtgccagaagtacggcataccggtcaccaagctcagcgcgtcggacctcaaggccgggaagaagggcatctgcggacacgtcgatgtcagcaatgcgtggcatcagtccgaccacgacgaccccggcccggacttcccctgggccgaattcatggcagccgtcaaaggcggtggcggcgccaccaaccccgatgaactggagctcacagtgtctcaattcagtgacctgaccaagcgcctgcagggcatgcaggagcagacccaccacgacctcggcgtcgtccagaccaagctggccaccatggacaccgtcaagaacccccgcaccggcgccaagtggagcctcaaggacgccatctggtcgatctggtactacgtgctggagaacagggaccggatcgccgccctcgagaagaaggtgaagtga

SEQ ID NO: 335 - DNA, 798 bp, Artificial Sequence
atgacgttcattcaggccgcgcatcacagcagcggctccaatctgccgcccacgagggtggtgatccacgcgacatgccccgaactcggcttcccgagggccagtgcgaagggccgagctgtctcgacagcccgctacttccagtctgcgatctcgggcggctcggcgcactatgttgtcgatgtcggcgaaaccgtgcagtgtctggcagaggatgtgatcgcctggcacgccccgcccaacagccgcagcctggggatcgagatctgcgctgacggcggctcggcgaccagcttcaagaaccccaacgtgcgctacagccgcgcccagtggctcagcccgcaggtctggcccgccgtgctccgtgccgcagcactcacccggcagatgtgccagaagtacggcataccggtcaccaagctcagcgcgtcggacctcaaggccgggaagaagggcatctgcggacacgtcgatgtcagcaatgcgtggcatcagtccgaccacgacgaccccggcccggacttcccctgggccgaattcatggcagccgtcaaaggcggcgccaccaaccccggcggtgtgtctcaattcagtgacctgaccaagcgcctgcagggcatgcaggagcagacccaccacgacctcggcgtcgtccagaccaagctggccaccatggacaccgtcaagaacccccgcaccggcgccaagtggagcctcaaggacgccatctggtcgatctggtactacgtgctggagaacagggaccggatcgccgccctcgagaagaaggtgaagtga

SEQ ID NO: 336 - DNA, 816 bp, Artificial Sequence
atgacgttcattcaggccgcgcatcacagcagcggctccaatctgccgcccacgagggtggtgatccacgcgacatgccccgaactcggcttcccgagggccagtgcgaagggccgagctgtctcgacagcccgctacttccagtctgcgatctcgggcggctcggcgcactatgttgtcgatgtcggcgaaaccgtgcagtgtctggcagaggatgtgatcgcctggcacgccccgcccaacagccgcagcctggggatcgagatctgcgctgacggcggctcggcgaccagcttcaagaaccccaacgtgcgctacagccgcgcccagtggctcagcccgcaggtctggcccgccgtgctccgtgccgcagcactcacccggcagatgtgccagaagtacggcataccggtcaccaagctcagcgcgtcggacctcaaggccgggaagaagggcatctgcggacacgtcgatgtcagcaatgcgtggcatcagtccgaccacgacgaccccggcccggacttcccctgggccgaattcatggcagccgtcaaaggcggcgccaccaaccccggcggtgatgaactggagctcacagtgtctcaattcagtgacctgaccaagcgcctgcagggcatgcaggagcagacccaccacgacctcggcgtcgtccagaccaagctggccaccatggacaccgtcaagaacccccgcaccggcgccaagtggagcctcaaggacgccatctggtcgatctggtactacgtgctggagaacagggaccggatcgccgccctcgagaagaaggtgaagtga

SEQ ID NO: 337 - DNA, 834 bp, Artificial Sequence
atgacgttcattcaggccgcgcatcacagcagcggctccaatctgccgcccacgagggtggtgatccacgcgacatgccccgaactcggcttcccgagggccagtgcgaagggccgagctgtctcgacagcccgctacttccagtctgcgatctcgggcggctcggcgcactatgttgtcgatgtcggcgaaaccgtgcagtgtctggcagaggatgtgatcgcctggcacgccccgcccaacagccgcagcctggggatcgagatctgcgctgacggcggctcggcgaccagcttcaagaaccccaacgtgcgctacagccgcgcccagtggctcagcccgcaggtctggcccgccgtgctccgtgccgcagcactcacccggcagatgtgccagaagtacggcataccggtcaccaagctcagcgcgtcggacctcaaggccgggaagaagggcatctgcggacacgtcgatgtcagcaatgcgtggcatcagtccgaccacgacgaccccggcccggacttcccctgggccgaattcatggcagccgtcaaaggcggcgccaccaaccccggcggtggcggcgccaccaaccccgatgaactggagctcacagtgtctcaattcagtgacctgaccaagcgcctgcagggcatgcaggagcagacccaccacgacctcggcgtcgtccagaccaagctggccaccatggacaccgtcaagaacccccgcaccggcgccaagtggagcctcaaggacgccatctggtcgatctggtactacgtgctggagaacagggaccggatcgccgccctcgagaagaaggtgaagtga

SEQ ID NO: 338 - DNA, 816 bp, Artificial Sequence
atgacgttcattcaggccgcgcatcacagcagcggctccaatctgccgcccacgagggtggtgatccacgcgacatgccccgaactcggcttcccgagggccagtgcgaagggccgagctgtctcgacagcccgctacttccagtctgcgatctcgggcggctcggcgcactatgttgtcgatgtcggcgaaaccgtgcagtgtctggcagaggatgtgatcgcctggcacgccccgcccaacagccgcagcctggggatcgagatctgcgctgacggcggctcggcgaccagcttcaagaaccccaacgtgcgctacagccgcgcccagtggctcagcccgcaggtctggcccgccgtgctccgtgccgcagcactcacccggcagatgtgccagaagtacggcataccggtcaccaagctcagcgcgtcggacctcaaggccgggaagaagggcatctgcggacacgtcgatgtcagcaatgcgtggcatcagtccgaccacgacgaccccggcccggacttcccctgggccgaattcatggcagccgtcaaaggcggcgccaccaaccccgatgaactggagctcacaggcggtgtgtctcaattcagtgacctgaccaagcgcctgcagggcatgcaggagcagacccaccacgacctcggcgtcgtccagaccaagctggccaccatggacaccgtcaagaacccccgcaccggcgccaagtggagcctcaaggacgccatctggtcgatctggtactacgtgctggagaacagggaccggatcgccgccctcgagaagaaggtgaagtga

SEQ ID NO: 339 - DNA, 834 bp, Artificial Sequence
atgacgttcattcaggccgcgcatcacagcagcggctccaatctgccgcccacgagggtggtgatccacgcgacatgccccgaactcggcttcccgagggccagtgcgaagggccgagctgtctcgacagcccgctacttccagtctgcgatctcgggcggctcggcgcactatgttgtcgatgtcggcgaaaccgtgcagtgtctggcagaggatgtgatcgcctggcacgccccgcccaacagccgcagcctggggatcgagatctgcgctgacggcggctcggcgaccagcttcaagaaccccaacgtgcgctacagccgcgcccagtggctcagcccgcaggtctggcccgccgtgctccgtgccgcagcactcacccggcagatgtgccagaagtacggcataccggtcaccaagctcagcgcgtcggacctcaaggccgggaagaagggcatctgcggacacgtcgatgtcagcaatgcgtggcatcagtccgaccacgacgaccccggcccggacttcccctgggccgaattcatggcagccgtcaaaggcggcgccaccaaccccgatgaactggagctcacaggcggtgatgaactggagctcacagtgtctcaattcagtgacctgaccaagcgcctgcagggcatgcaggagcagacccaccacgacctcggcgtcgtccagaccaagctggccaccatggacaccgtcaagaacccccgcaccggcgccaagtggagcctcaaggacgccatctggtcgatctggtactacgtgctggagaacagggaccggatcgccgccctcgagaagaaggtgaagtga

SEQ ID NO: 340 - DNA, 852 bp, Artificial Sequence
atgacgttcattcaggccgcgcatcacagcagcggctccaatctgccgcccacgagggtggtgatccacgcgacatgccccgaactcggcttcccgagggccagtgcgaagggccgagctgtctcgacagcccgctacttccagtctgcgatctcgggcggctcggcgcactatgttgtcgatgtcggcgaaaccgtgcagtgtctggcagaggatgtgatcgcctggcacgccccgcccaacagccgcagcctggggatcgagatctgcgctgacggcggctcggcgaccagcttcaagaaccccaacgtgcgctacagccgcgcccagtggctcagcccgcaggtctggcccgccgtgctccgtgccgcagcactcacccggcagatgtgccagaagtacggcataccggtcaccaagctcagcgcgtcggacctcaaggccgggaagaagggcatctgcggacacgtcgatgtcagcaatgcgtggcatcagtccgaccacgacgaccccggcccggacttcccctgggccgaattcatggcagccgtcaaaggcggcgccaccaaccccgatgaactggagctcacaggcggtggcggcgccaccaaccccgatgaactggagctcacagtgtctcaattcagtgacctgaccaagcgcctgcagggcatgcaggagcagacccaccacgacctcggcgtcgtccagaccaagctggccaccatggacaccgtcaagaacccccgcaccggcgccaagtggagcctcaaggacgccatctggtcgatctggtactacgtgctggagaacagggaccggatcgccgccctcgagaagaaggtgaagtga

SEQ ID NO: 342 - DNA, 879 bp, Artificial Sequence
atgacattcatccaggcccgccatcacggcggcaactccaacacgccgatcacccggctggtcatccacgccacctgccccgacgtgggctacccgtcggcgtcgaaggccggtagggcagtctccacggcggagtatttcgcgtccacgtcgcggtctgcctcggctcactacgtctgtgacgtatcggcaacggtgcagtgcctctccgaggaaaccatcggctaccacgcgccgcccaacagtcattccatcggcattgagatttgcgccgacggcgggtcccgcgcctcatttgagaaggcttctcacgcatacacccgcgagcaatggctctcgcctcaagtgtggcccgccgtggagcgcgccgccattctcgcccgcggcatctgccaccgccaccacatcccggttcgcaaactcaccaccgcacaggtcaaatcggggatgtcgggtatttgcggacacgacaacgtatccgatgcattccaccaatccgaccacgacgaccctggcccctacttcccgtggaacgaatttatcgccgccatccaaggaaaaaacaccaacaagggagaactcagcggcggtaaaaacaccaacaagggagaactcagcatgtccgacgtcaacaccctgaccaagctcatcaaggccagcaacaatcagctccaccacgacattggcgtcgtccagacacagaacggcaccctcaaaagcaagatcgacaacttgtcgtgggtgaagaatcccgtcaccggcaagaagtggtccaccaaggatgcgctgtggtctgtctggtactacgtgctggaatgccgcaaccgcatccaggctatcgaaaaccgcctctctgacatcgaaaagaaggtgaagtga

SEQ ID NO: 342 - DNA, 900 bp, Artificial Sequence
atgaaatacattcccgcgacacatcacggaggccacacgaacacccccttcacccggatcgtgatccacgccacctgccccgaccttggcttcccccacgcatcagctggtggacaggcaaaagccaccgcacgctatttccaatcagagcagtctgccggatcagcacactatgtgtgcgacatcgccgagactatccaatgcctgcccgatgacgtgatcgcctggcacgccccaccaaacagaaggtcgatcggaatcgaaatatgtgccgacggcggctcccgctcctcattccagcaccccgagcacgcctacaccagatcccaatggctcagcccccaagtgtggcccgccgtcgcccgtgccgccgcgctcacccgcgacctctgccaccgccacaacattccgatgcaacaactctccgttgctgatgtgaaagccgggaagcacggaatctgcggccacaacgacgtatccgaggcattccacaagtccgaccatgacgaccccggccccacattcccgtgggaccaattcatcaaagaggttagaacaggcggtacattcccgtgggaccaattcatcaaagaggttagaacaccaggacaacaagatacgaaaccttccgtaccaacaccatcactcacagaaataggagatcaggacatgaacgggtgctactacaacctcaattcgaaaacacggacgtaccttatcttcgatagccgttccggattttaccacgaattctcccaaggcaatgggaacggccccatgagcccagactatgtaaatccgatcgccaaaggatgggacaccggatcatggccggcaatctccccaggccacgcgaaagtgctcaaggccgccctcgataaagtccggaaaggaatctga

SEQ ID NO: 343 - protein, 38 aa, Artificial Sequence
DRILPSASETGTQTSKTTAAEKVLDYKRDWVKQDTYYN

SEQ ID NO: 344 - protein, 6 aa, Artificial Sequence
IPQEGL

SEQ ID NO: 345 - protein, 21 aa, Artificial Sequence
GFEKGPLGYPTRRHATVNGVG

SEQ ID NO: 346 - protein, 24 aa, Artificial Sequence
GADWPGDAPSNSSAKPETGKVKNI

SEQ ID NO: 347 - protein, 12 aa, Artificial Sequence
HGDTPEIEEEFD

SEQ ID NO: 348 - protein, 17 aa, Artificial Sequence
IDLLTPNDDGRATKPRN

SEQ ID NO: 349 - protein, 35 aa, Artificial Sequence
PKPTPAPPSDPAPRPIPPKETLVPTTLDTVLPSLV

SEQ ID NO: 350 - protein, 9 aa, Artificial Sequence
GSGESGELS

SEQ ID NO: 351 - protein, 20 aa, Artificial Sequence
NGGSGDSGELTVADVKALHD

SEQ ID NO: 352 - protein, 9 aa, Artificial Sequence
KNTNKGELS

SEQ ID NO: 353 - protein, 12 aa, Artificial Sequence
GGATNPDELELT

SEQ ID NO: 354 - protein, 71 aa, Artificial Sequence
ASLAENQRADYMARAQAYFDGAPVTGRSSVPAPAPAPAGIHVDLPAWTLPAGNFYGSIDGGEDSHGGYYEG

SEQ ID NO: 355 - protein, 14 aa, Artificial Sequence
LTDDLQGGDDMPLS

SEQ ID NO: 356 - protein, 71 aa, Artificial Sequence
ASLARDQLGDYMGRAQAYFDGAPVAAVHQSVPAPAPAPSRHVDLPAWNLPEGNFYGLVSGGNDSHGGFYPA

SEQ ID NO: 357 - protein, 28 aa, Artificial Sequence
AIAKQMVGATTTGRLSNDCVTGTANETG

SEQ ID NO: 358 - protein, 32 aa, Artificial Sequence
RAQAYYDGTSVAAAPAAPSAPAGIHVDLPSWT

SEQ ID NO: 359 - protein, 47 aa, Artificial Sequence
RAQAYYDGAPVAAVHQSAPAPAPASSRHVDLPAWNLPEGNFYGLASG

SEQ ID NO: 360 - protein, 68 aa, Artificial Sequence
GAYAYSGESYTGTNTEGSYGSSYDTSAQDASYDGSYSYDNSYSYDNSAGYDSSSAYSGGYQATREATG

SEQ ID NO: 361 - protein, 52 aa, Artificial Sequence
VTAAQLRAGKRGICSHVAVSDAFGQSDHGDPEVAGPFPWAKFMQLIKEEDDM

SEQ ID NO: 362 - protein, 20 aa, Artificial Sequence
YFPWNEFIAAVQGKTTTPEG

SEQ ID NO: 363 - protein, 40 aa, Artificial Sequence
WFPWDKFMAVVNGHGGGSSSEELSMADVQALHNQIKQLSA

SEQ ID NO: 364 - protein, 23 aa, Artificial Sequence
YFPWDQFMALVQGKPATPGDLTM

SEQ ID NO: 365 - protein, 27 aa, Artificial Sequence
YFPWDGFIALVNGHSAPSRQEELTVSD

SEQ ID NO: 366 - protein, 27 aa, Artificial Sequence
DFPWAEFMAAVKGGTTTQEDEDEMKEA

SEQ ID NO: 367 - protein, 13 aa, Artificial Sequence
TFPWDQFIKEVRT

SEQ ID NO: 369 - DNA, 114 bp, Artificial Sequence
gaccgaatccttccttcagcctctgagacaggcacacagacatcgaaaacgacggctgcggagaaggtcctggattataagcgagactgggtgaagcaggacacctactataac

SEQ ID NO: 369 - DNA, 18 bp, Artificial Sequence
attcctcaggaaggacta

SEQ ID NO: 370 - DNA, 63 bp, Artificial Sequence
ggattcgagaagggaccgctcggctacccgacgcgccgtcacgccacggtcaacggtgtcggc

SEQ ID NO: 371 - DNA, 72 bp, Artificial Sequence
ggtgcagactggccgggtgatgcgccctcaaattcgagcgcgaaaccggaaacggggaaggtcaaaaacatc

SEQ ID NO: 372 - DNA, 36 bp, Artificial Sequence
catggggacaccccagaaatagaggaggagttcgat

SEQ ID NO: 373 - DNA, 51 bp, Artificial Sequence
atcgacctgctgacccccaacgacgatggccgggcgacgaagccccgcaac

SEQ ID NO: 374 - DNA, 105 bp, Artificial Sequence
ccgaagccgacgcccgccccgccgtcggatccggcgccccgtccgattcccccgaaggagactctggtgcccaccacgctcgacaccgtcctgccgtcgctcgtc

SEQ ID NO: 375 - DNA, 27 bp, Artificial Sequence
ggcagtggagagagtggagagttgagt

SEQ ID NO: 377 - DNA, 60 bp, Artificial Sequence
aacggcggtagtggagatagtggggagttaactgtggctgatgtgaaagccttgcatgat

SEQ ID NO: 378 - DNA, 27 bp, Artificial Sequence
aaaaacaccaacaagggagaactcagc

SEQ ID NO: 378 - DNA, 36 bp, Artificial Sequence
ggcggcgccaccaaccccgatgaactggagctcaca

SEQ ID NO: 379 - DNA, 213 bp, Artificial Sequence
gcctcgcttgccgagaatcagcgcgcggattacatggcgcgcgctcaggcctatttcgatggcgctcccgtcacaggccgttcttcggtccctgcaccggctccggcgcctgccgggatccatgtggacctgcctgcctggactctccccgcaggcaacttttacgggtcgatcgatggcggcgaggactcgcatggcggctactacgagggt

SEQ ID NO: 380 - DNA, 42 bp, Artificial Sequence
ctcaccgacgatctccaaggaggagacgacatgcccctgtca

SEQ ID NO: 381 - DNA, 213 bp, Artificial Sequence
gcgtcgctggcccgggaccagctcggcgactacatggggcgcgcacaagcctacttcgatggcgcgccggtggctgcggtccatcagtcggtccctgcccccgccccagcgcccagccgtcatgtggacctgcccgcgtggaatctccccgagggcaacttctacggcctcgtcagcggcggaaacgactcccacggcggcttctatcccgcc

SEQ ID NO: 382 - DNA, 84 bp, Artificial Sequence
gccatcgccaaacagatggtgggagccaccaccacagggcgcctgtccaacgactgtgtcaccgggaccgctaacgaaaccggc

SEQ ID NO: 383 - DNA, 96 bp, Artificial Sequence
cgggctcaggcctactacgacggcacttcagtggctgccgcacctgctgccccgtcggcacctgccgggatccacgtcgatcttccgagctggacc

SEQ ID NO: 384 - DNA, 141 bp, Artificial Sequence
cgggctcaggcctactacgacggcgcgccggtggctgcggtccatcagtcggcacctgcccccgccccagcgtccagccgtcacgtggacctgcccgcgtggaatctccccgagggcaacttctacggcctggcgagcggt

SEQ ID NO: 385 - DNA, 204 bp, Artificial Sequence
ggcgcgtacgcctactccggtgaaagctacaccggcaccaacaccgagggttcctacggctcttcgtacgacacgtcggcccaggacgcctcctacgacggctcgtactcgtatgacaactcgtactcgtacgacaacagcgccgggtacgactcgtcctccgcctactccggcggctaccaggccactcgtgaggccactggc

SEQ ID NO: 386 - DNA, 156 bp, Artificial Sequence
gtgaccgccgcgcagctcagggcgggcaagcgcggcatctgctcgcatgtcgcggtcagcgacgcgttcgggcagtccgaccacggcgatcccgaggtcgccgggccgttcccctgggcgaagttcatgcagctcatcaaggaggaggacgacatg

SEQ ID NO: 387 - DNA, 60 bp, Artificial Sequence
tatttcccttggaatgaatttattgccgccgtccaaggaaaaaccaccacaccagaggga

SEQ ID NO: 388 - DNA, 120 bp, Artificial Sequence
tggtttccgtgggacaaatttatggctgtggtgaatggccacggcggcggttcaagtagtgaggagttgagtatggctgatgtacaagcgttacataatcagattaaacagttgtcggca

SEQ ID NO: 389 - DNA, 69 bp, Artificial Sequence
tacttcccgtgggaccagttcatggcactcgtccaaggaaaacccgccacaccaggagatctcaccatg

SEQ ID NO: 390 - DNA, 81 bp, Artificial Sequence
tatttcccgtgggacgggtttatcgcgcttgttaatggccattccgcaccatcacgccaggaggaactaactgtgtcagat

SEQ ID NO: 391 - DNA, 81 bp, Artificial Sequence
gacttcccgtgggccgaattcatggcagccgtcaaaggcggcaccaccacacaggaagatgaggatgaaatgaaggaagct

SEQ ID NO: 392 - DNA, 39 bp, Artificial Sequence
acattcccgtgggaccaattcatcaaagaggttagaaca

SEQ ID NO: 394 - protein, 5 aa, Artificial Sequence
PAPAP

SEQ ID NO: 394 - protein, 12 aa, Artificial Sequence
AEAAAKEAAAKA

SEQ ID NO: 395 - protein, 17 aa, Artificial Sequence
VSQTSKLTRAETVFPDV

SEQ ID NO: 396 - protein, 6 aa, Artificial Sequence
PLGLWA

SEQ ID NO: 397 - protein, 6 aa, Artificial Sequence
RVLAEA

SEQ ID NO: 398 - protein, 10 aa, Artificial Sequence
EDVVCCSMSY

SEQ ID NO: 399 - protein, 8 aa, Artificial Sequence
GGIEGRGS

SEQ ID NO: 400 - protein, 10 aa, Artificial Sequence
TRHRQPRGWE

SEQ ID NO: 401 - protein, 10 aa, Artificial Sequence
AGNRVRRSVG

SEQ ID NO: 402 - protein, 9 aa, Artificial Sequence
RRRRRRRRR

SEQ ID NO: 403 - protein, 4 aa, Artificial Sequence
GFLG

SEQ ID NO: 404 - protein, 18 aa, Artificial Sequence
KESGSVSSEQLAQFRSLD

SEQ ID NO: 405 - protein, 14 aa, Artificial Sequence
EGKSSGSGSESKST

SEQ ID NO: 406 - protein, 12 aa, Artificial Sequence
GSAGSAAGSGEF